European Patent Application EP 4 265 270 A1, published October 25, 2023. Title: Agent for activating a neuronal cell. Applicant: Kyoto University. The sequence listing filed with the application follows.

SEQUENCE LISTING (122 sequences)

SEQ ID NO: 1 - protein, 148 aa, Mus musculus
MKTLLTLGLLLLSVTAQAKVYERCEFARTLKRNGMAGYYGVSLADWVCLAQHESNYNTRATNYNRGDQSTDYGIFQINSRYWCNDGKTPRAVNACGINCSALLQDDITAAIQCAKRVVRDPQGIRAWVAWRAHCQNRDLSQYIRNCGV

SEQ ID NO: 2 - protein, 148 aa, Homo sapiens
MKALIVLGLVLLSVTVQGKVFERCELARTLKRLGMDGYRGISLANWMCLAKWESGYNTRATNYNAGDRSTDYGIFQINSRYWCNDGKTPGAVNACHLSCSALLQDNIADAVACAKRVVRDPQGIRAWVAWRNRCQNRDVRQYVQGCGV

SEQ ID NO: 3 - protein, 74 aa, Mus musculus
MKSFLLFLTIILLVVIQIQTGSLGQATTAASGTNKNSTSTKKTPLKSGASSIIDAGACSFLFFANTLMCLFYLS

SEQ ID NO: 4 - protein, 61 aa, Homo sapiens
MKRFLFLLLTISLLVMVQIQTGLSGQNDTSQTSSPSASSNISGGIFLFFVANAIIHLFCFS

SEQ ID NO: 5 - protein, 713 aa, Mus musculus
MNSFMALVLIWMIIACAEADKPLGETGTTGFQICKNALKLPVLEVLPGGGWDNLRNVDMGRVMDLTYTNCKTTEDGQYIIPDEVYTIPQKESNLEMNSEVLESWMNYQSTTSLSINTELALFSRVNGKFSTEFQRMKTLQVKDQAVTTRVQVRNRIYTVKTTPTSELSLGFTKALMDICDQLEKNQTKMATYLAELLILNYGTHVITSVDAGAALVQEDHVRSSFLLDNQNSQNTVTASAGIAFLNIVNFKVETDYISQTSLTKDYLSNRTNSRVQSFGGVPFYPGITLETWQKGITNHLVAIDRAGLPLHFFIKPDKLPGLPGPLVKKLSKTVETAVRHYYTFNTHPGCTNVDSPNFNFQANMDDDSCDAKVTNFTFGGVYQECTELSGDVLCQNLEQKNLLTGDFSCPPGYTPVHLLSQTHEEGYSRLECKKKCTLKIFCKTVCEDVFRVAKAEFRAYWCVAAGQVPDNSGLLFGGVFTDKTINPMTNAQSCPAGYIPLNLFESLKVCVSLDYELGFKFSVPFGGFFSCIMGNPLVNSDTAKDVRAPSLKKCPGGFSQHLAVISDGCQVSYCVKAGIFTGGSLLPVRLPPYTKPPLMSQVATNTVIVTNSETARSWIKDPQTNQWKLGEPLELRRAMTVIHGDSNGMSGGEAAGITLGVTIALGVVITLAIYGTRKYKKKEYQEIEEQESLVGSLATDATVLNGEEDPSPA

SEQ ID NO: 6 - protein, 713 aa, Mus musculus; identical to SEQ ID NO: 5

SEQ ID NO: 7 - protein, 716 aa, Homo sapiens
MNNFRATILFWAAAAWAKSGKPSGEMDEVGVQKCKNALKLPVLEVLPGGGWDNLRNVDMGRVMELTYSNCRTTEDGQYIIPDEIFTIPQKQSNLEMNSEILESWANYQSSTSYSINTELSLFSKVNGKFSTEFQRMKTLQVKDQAITTRVQVRNLVYTVKINPTLELSSGFRKELLDISDRLENNQTRMATYLAELLVLNYGTHVTTSVDAGAALIQEDHLRASFLQDSQSSRSAVTASAGLAFQNTVNFKFEENYTSQNVLTKSYLSNRTNSRVQSIGGVPFYPGITLQAWQQGITNHLVAIDRSGLPLHFFINPNMLPDLPGPLVKKVSKTVETAVKRYYTFNTYPGCTDLNSPNFNFQANTDDGSCEGKMTNFSFGGVYQECTQLSGNRDVLLCQKLEQKNPLTGDFSCPSGYSPVHLLSQIHEEGYNHLECHRKCTLLVFCKTVCEDVFQVAKAEFRAFWCVASSQVPENSGLLFGGLFSSKSINPMTNAQSCPAGYFPLRLFENLKVCVSQDYELGSRFAVPFGGFFSCTVGNPLVDPAISRDLGAPSLKKCPGGFSQHPALISDGCQVSYCVKSGLFTGGSLPPARLPPFTRPPLMSQAATNTVIVTNSENARSWIKDSQTHQWRLGEPIELRRAMNVIHGDGGGLSGGAAAGVTVGVTTILAVVITLAIYGTRKFKKKAYQAIEERQSLVPGTAATGDTTYQEQGQSPA

SEQ ID NO: 8 - protein, 104 aa, Mus musculus
MKISTLLCLLLIATTISPQVLAGPDAVSTPVTCCYNVVKQKIHVRKLKSYRRITSSQCPREAVIFRTILDKEICADPKEKWVKNSINHLDKTSQTFILEPSCLG

SEQ ID NO: 9 - protein, 99 aa, Homo sapiens
MKVSAALLCLLLIAATFIPQGLAQPDAINAPVTCCYNFTNRKISVQRLASYRRITSSKCPKEAVIFKTIVAKEICADPKQKWVQDSMDHLDKQTQTPKT

SEQ ID NO: 10 - protein, 144 aa, Mus musculus
MWLAILLALCCLTSDTHGARPPDFCSKDLISSVKPGFPKTIETNNPGVLKAARHSVEKFNNCTNDIFLFKESHVSKALVQVVKGLKYMLEVKIGRTTCRKTMHHQLDNCDFQTNPALKRTLYCYSEVWVIPWLHSFEVPVLLCQ

SEQ ID NO: 11 - protein, 145 aa, Homo sapiens
MRAAGTLLAFCCLVLSTTGGPSPDTCSQDLNSRVKPGFPKTIKTNDPGVLQAARYSVEKFNNCTNDMFLFKESRITRALVQIVKGLKYMLEVEIGRTTCKKNQHLRLDDCDFQTNHTLKQTLSCYSEVWVVPWLQHFEVPVLRCH

SEQ ID NO: 12 - protein, 192 aa, Mus musculus
MQAIKCVVVGDGAVGKTCLLISYTTNAFPGEYIPTVFDNYSANVMVDSKPVNLGLWDTAGQEDYDRLRPLSYPQTDVFLICFSLVSPASYENVRAKWFPEVRHHCPSTPIILVGTKLDLRDDKDTIEKLKEKKLAPITYPQGLALAKDIDSVKYLECSALTQRGLKTVFDEAIRAVLCPQPTRQQKRPCSLL

SEQ ID NO: 13 - protein, 192 aa, Homo sapiens
MQAIKCVVVGDGAVGKTCLLISYTTNAFPGEYIPTVFDNYSANVMVDSKPVNLGLWDTAGQEDYDRLRPLSYPQTDVFLICFSLVSPASYENVRAKWFPEVRHHCPSTPIILVGTKLDLRDDKDTIEKLKEKKLAPITYPQGLALAKEIDSVKYLECSALTQRGLKTVFDEAIRAVLCPQPTRQQKRACSLL

SEQ ID NO: 14 - protein, 418 aa, Mus musculus
MAFIAALGLLMAGICPAVLCFPDGTLGMDAAVQEDHDNGTQLDSLTLASINTDFAFSLYKELVLKNPDKNIVFSPLSISAALAVMSLGAKGNTLEEILEGLKFNLTETSEADIHQGFGHLLQRLNQPKDQVQISTGSALFIEKRQQILTEFQEKARALYQAEAFTADFQQPRQAKKLINDYVRKQTQGMIKELVSDLDKRTLMVLVNYIYFKAKWKVPFDPLDTFKSEFYAGKRRPVIVPMMSMEDLTTPYFRDEELFCTVVELKYTGNASAMFILPDQGKMQQVEASLQPETLRKWKNSLKPRMIDELHLPKFSISTDYSLEDVLSKLGIREVFSTQADLSAITGTKDLRVSQVVHKAVLDVAETGTEAAAATGVKFVPMSAKLYPLTVYFNRPFLIMIFDTETEIAPFIAKIANPK

SEQ ID NO: 15 - protein, 423 aa, Homo sapiens
MERMLPLLALGLLAAGFCPAVLCHPNSPLDEENLTQENQDRGTHVDLGLASANVDFAFSLYKQLVLKAPDKNVIFSPLSISTALAFLSLGAHNTTLTEILKGLKFNLTETSEAEIHQSFQHLLRTLNQSSDELQLSMGNAMFVKEQLSLLDRFTEDAKRLYGSEAFATDFQDSAAAKKLINDYVKNGTRGKITDLIKDLDSQTMMVLVNYIFFKAKWEMPFDPQDTHQSRFYLSKKKWVMVPMMSLHHLTIPYFRDEELSCTVVELKYTGNASALFILPDQDKMEEVEAMLLPETLKRWRDSLEFREIGELYLPKFSISRDYNLNDILLQLGIEEAFTSKADLSGITGARNLAVSQVVHKAVLDVFEEGTEASAATAVKITLLSALVETRTIVRFNRPFLMIIVPTDTQNIFFMSKVTNPKQA

SEQ ID NO: 16 - protein, 76 aa, Mus musculus
MKTATVLFLVALITVGMNTTYVVSCPKEFEKPGACPKPSPESVGICVDQCSGDGSCPGNMKCCSNSCGHVCKTPVF

SEQ ID NO: 17 - protein, 680 aa, Homo sapiens
MVPGVPGAVLTLCLWLAASSGCLAAGPGAAAARRLDESLSAGSVQRARCASRCLSLQITRISAFFQHFQNNGSLVWCQNHKQCSKCLEPCKESGDLRKHQCQSFCEPLFPKKSYECLTSCEFLKYILLVKQGDCPAPEKASGFAAACVESCEVDNECSGVKKCCSNGCGHTCQVPKTLYKGVPLKPRKELRFTELQSGQLEVKWSSKFNISIEPVIYVVQRRWNYGIHPSEDDATHWQTVAQTTDERVQLTDIRPSRWYQFRVAAVNVHGTRGFTAPSKHFRSSKDPSAPPAPANLRLANSTVNSDGSVTVTIVWDLPEEPDIPVHHYKVFWSWMVSSKSLVPTKKKRRKTTDGFQNSVILEKLQPDCDYVVELQAITYWGQTRLKSAKVSLHFTSTHATNNKEQLVKTRKGGIQTQLPFQRRRPTRPLEVGAPFYQDGQLQVKVYWKKTEDPTVNRYHVRWFPEACAHNRTTGSEASSGMTHENYIILQDLSFSCKYKVTVQPIRPKSHSKAEAVFFTTPPCSALKGKSHKPVGCLGEAGHVLSKVLAKPENLSASFIVQDVNITGHFSWKMAKANLYQPMTGFQVTWAEVTTESRQNSLPNSIISQSQILPSDHYVLTVPNLRPSTLYRLEVQVLTPGGEGPATIKTFRTPELPPSSAHRSHLKHRHPHHYKPSPERY

SEQ ID NO: 18 - protein, 253 aa, Mus musculus
MPMKMLTMKMLALCLVLAKSAWSEEQEKVVHGGPCLKDSHPFQAALYTSGHLLCGGVLIDPQWVLTAAHCKKPNLQVILGKHNLRQTETFQRQISVDRTIVHPRYNPETHDNDIMMVHLKNPVKFSKKIQPLPLKNDCSEENPNCQILGWGKMENGDFPDTIQCADVHLVPREQCERAYPGKITQSMVCAGDMKEGNDSCQGDSGGPLVCGGRLRGLVSWGDMPCGSKEKPGVYTDVCTHIRWIQNILRNKWL

SEQ ID NO: 19 - protein, 244 aa, Homo sapiens
MKKLMVVLSLIAAAWAEEQNKLVHGGPCDKTSHPYQAALYTSGHLLCGGVLIHPLWVLTAAHCKKPNLQVFLGKHNLRQRESSQEQSSVVRAVIHPDYDAASHDQDIMLLRLARPAKLSELIQPLPLERDCSANTTSCHILGWGKTADGDFPDTIQCAYIHLVSREECEHAYPGQITQNMLCAGDEKYGKDSCQGDSGGPLVCGDHLRGLVSWGNIPCGSKEKPGVYTNVCRYTNWIQKTIQAK

SEQ ID NO: 20 - protein, 137 aa, Homo sapiens
MLLRLARPAKLSELIQPLPLERDCSANTTSCHILGWGKTADGDFPDTIQCAYIHLVSREECEHAYPGQITQNMLCAGDEKYGKDSCQGDSGGPLVCGDHLRGLVSWGNIPCGSKEKPGVYTNVCRYTNWIQKTIQAK

SEQ ID NO: 21 - protein, 137 aa, Homo sapiens; identical to SEQ ID NO: 20

SEQ ID NO: 22 - protein, 137 aa, Homo sapiens; identical to SEQ ID NO: 20

SEQ ID NO: 23 - protein, 244 aa, Homo sapiens; identical to SEQ ID NO: 19

SEQ ID NO: 24 - protein, 1474 aa, Mus musculus
MGKRWLPSLALLPLPPPLLLLLLLLLPTNASAPQKPIYMVMVPSLLHAGTPEKGCLLFNHLNETVTVKVSMESVRGNQSLFTDLVVDKDLFHCASFIVPQSSSNEVMFLTVQVKGPTHEFRRRSTVLIKTKESLVFAQTDKPIYKPGQMVRFRVVSLDENFHPLNELIPLLYIQDSKKNRIAQWQNFRLEGGLKQLSFPLSSEPTQGSYKVVIRTESGRTVEHPFSVKEFVLPKFEVKVAVPETITILEEEMNVSVCGIYTYGKPVPGHVTVNICRKYSNPSSCFGEESLAFCEKFSQQLDGRGCFSQLVKTKSFQLKRQEYEMQLDVNAKIQEEGTGVEETGKGLTKITRTITKLSFVNVDTHFRQGIPFVGQVLLVDGRGTPIPYEMIFIGADEANQNINTTTDKNGLARFSINTDDIMGTSLTVRAKYKDSNVCYGFRWLTEENVEAWHTANAVFSPSRSFVHLESLPYKLRCEQTLAVQAHYILNDEAVLERKELVFYYLMMAKGGIVRAGTHVLPVTQGHKKGHFSILISMETDLAPVARLVLYTILPNGEVVGDTVKYEIEKCLANKVDLVFHPNIGLPATRAFLSVMASPQSLCGLRAVDQSVLLTKPEAELSASLVYDLLPVKDLTGFPKGVNQQEEDTNGCLKQNDTYINGILYSPVQNTNEEDMYGFLKDMGLKVFTNLNIRKPKVCERLGVNKIPAAYHLVSQGHMDAFLESSESPTETTRSYFPETWIWDLVIVDSTGVAEMEVTVPDTITEWKAGAFCLSNDTGLGLSPVIDFQAFQPFFVDLTMPYSVIRGEAFTLKATVLNYLQTCIRVGVQLEASPDFLATPEEKEQKSHCICMNERHTMSWAVIPKSLGNVNFTVSAEALDSKELCRNEVPVVPERGKKDTIIKSLLVEPEGLENEVTFNSLLCPTGAEVSEQISLKLPSDVVEESARASVTVLGDILGSAMQNTQDLLKMPYGCGEQNMVLFAPNIYVLDYLNETEQLTQEIKTKAITYLNTGYQRQLNYKHRDGSYSTFGDKPGRSHANTWLTAFVLKSFAQARRYIFIDESHITQALTWLSQQQKDNGCFRSSGSLLNNAMKGGVEDEVTLSAYITIALLEMSLPVTHPVVRNALFCLDTAWKSARRGASGNHVYTKALLAYAFALAGNQDTKKEILKSLDEEAVKEDNSVHWTRAQKPRVPADLWYQPQAPSAEVEMTAYVLLAYLTTELVPTREDLTAAMLIVKWLTKQQNSHGGFSSTQDTVVALHALSKYGAATFTRAKKAAHVTIQSSGAFYTKFQVNNDNQLLLQRVTLPTVPGDYTAKVAGEGCVYLQTSLKYSVLPREKEFPFALVVQTLPGTCEDLKAHTTFQISLNISYIGSRSDSNMAIADVKMVSGFIPLKPTVKMLERSVHVSRTEVSNNHVLIYLDKVSNQMLTLFFMVQQDIPVRDLKPAIVKVYDYYEKDEFAVAKYSAPCSAGYGNA

SEQ ID NO: 25 - protein, 1474 aa, Homo sapiens
MGKNKLLHPSLVLLLLVLLPTDASVSGKPQYMVLVPSLLHTETTEKGCVLLSYLNETVTVSASLESVRGNRSLFTDLEAENDVLHCVAFAVPKSSSNEEVMFLTVQVKGPTQEFKKRTTVMVKNEDSLVFVQTDKSIYKPGQTVKFRVVSMDENFHPLNELIPLVYIQDPKGNRIAQWQSFQLEGGLKQFSFPLSSEPFQGSYKVVVQKKSGGRTEHPFTVEEFVLPKFEVQVTVPKIITILEEEMNVSVCGLYTYGKPVPGHVTVSICRKYSDASDCHGEDSQAFCEKFSGQLNSHGCFYQQVKTKVFQLKRKEYEMKLHTEAQIQEEGTVVELTGRQSSEITRTITKLSFVKVDSHFRQGIPFFGQVRLVDGKGVPIPNKVIFIRGNEANYYSNATTDEHGLVQFSINTTNVMGTSLTVRVNYKDRSPCYGYQWVSEEHEEAHHTAYLVFSPSKSFVHLEPMSHELPCGHTQTVQAHYILNGGTLLGLKKLSFYYLIMAKGGIVRTGTHGLLVKQEDMKGHFSISIPVKSDIAPVARLLIYAVLPTGDVIGDSAKYDVENCLANKVDLSFSPSQSLPASHAHLRVTAAPQSVCALRAVDQSVLLMKPDAELSASSVYNLLPEKDLTGFPGPLNDQDNEDCINRHNVYINGITYTPVSSTNEKDMYSFLEDMGLKAFTNSKIRKPKMCPQLQQYEMHGPEGLRVGFYESDVMGRGHARLVHVEEPHTETVRKYFPETWIWDLVVVNSAGVAEVGVTVPDTITEWKAGAFCLSEDAGLGISSTASLRAFQPFFVELTMPYSVIRGEAFTLKATVLNYLPKCIRVSVQLEASPAFLAVPVEKEQAPHCICANGRQTVSWAVTPKSLGNVNFTVSAEALESQELCGTEVPSVPEHGRKDTVIKPLLVEPEGLEKETTFNSLLCPSGGEVSEELSLKLPPNVVEESARASVSVLGDILGSAMQNTQNLLQMPYGCGEQNMVLFAPNIYVLDYLNETQQLTPEIKSKAIGYLNTGYQRQLNYKHYDGSYSTFGERYGRNQGNTWLTAFVLKTFAQARAYIFIDEAHITQALIWLSQRQKDNGCFRSSGSLLNNAIKGGVEDEVTLSAYITIALLEIPLTVTHPVVRNALFCLESAWKTAQEGDHGSHVYTKALLAYAFALAGNQDKRKEVLKSLNEEAVKKDNSVHWERPQKPKAPVGHFYEPQAPSAEVEMTSYVLLAYLTAQPAPTSEDLTSATNIVKWITKQQNAQGGFSSTQDTVVALHALSKYGAATFTRTGKAAQVTIQSSGTFSSKFQVDNNNRLLLQQVSLPELPGEYSMKVTGEGCVYLQTSLKYNILPEKEEFPFALGVQTLPQTCDEPKAHTSFQISLSVSYTGSRSASNMAIVDVKMVSGFIPLKPTVKMLERSNHVSRTEVSSNHVLIYLDKVSNQTLSLFFTVLQDVPVRDLKPAIVKVYDYYETDEFAIAEYNAPCSKDLGNA

SEQ ID NO: 26 - protein, 1474 aa, Homo sapiens; identical to SEQ ID NO: 25

SEQ ID NO: 27 - protein, 1374 aa, Homo sapiens
MFLTVQVKGPTQEFKKRTTVMVKNEDSLVFVQTDKSIYKPGQTVKFRVVSMDENFHPLNELIPLVYIQDPKGNRIAQWQSFQLEGGLKQFSFPLSSEPFQGSYKVVVQKKSGGRTEHPFTVEEFVLPKFEVQVTVPKIITILEEEMNVSVCGLYTYGKPVPGHVTVSICRKYSDASDCHGEDSQAFCEKFSGQLNSHGCFYQQVKTKVFQLKRKEYEMKLHTEAQIQEEGTVVELTGRQSSEITRTITKLSFVKVDSHFRQGIPFFGQVRLVDGKGVPIPNKVIFIRGNEANYYSNATTDEHGLVQFSINTTNVMGTSLTVRVNYKDRSPCYGYQWVSEEHEEAHHTAYLVFSPSKSFVHLEPMSHELPCGHTQTVQAHYILNGGTLLGLKKLSFYYLIMAKGGIVRTGTHGLLVKQEDMKGHFSISIPVKSDIAPVARLLIYAVLPTGDVIGDSAKYDVENCLANKVDLSFSPSQSLPASHAHLRVTAAPQSVCALRAVDQSVLLMKPDAELSASSVYNLLPEKDLTGFPGPLNDQDNEDCINRHNVYINGITYTPVSSTNEKDMYSFLEDMGLKAFTNSKIRKPKMCPQLQQYEMHGPEGLRVGFYESDVMGRGHARLVHVEEPHTETVRKYFPETWIWDLVVVNSAGVAEVGVTVPDTITEWKAGAFCLSEDAGLGISSTASLRAFQPFFVELTMPYSVIRGEAFTLKATVLNYLPKCIRVSVQLEASPAFLAVPVEKEQAPHCICANGRQTVSWAVTPKSLGNVNFTVSAEALESQELCGTEVPSVPEHGRKDTVIKPLLVEPEGLEKETTFNSLLCPSGGEVSEELSLKLPPNVVEESARASVSVLGDILGSAMQNTQNLLQMPYGCGEQNMVLFAPNIYVLDYLNETQQLTPEIKSKAIGYLNTGYQRQLNYKHYDGSYSTFGERYGRNQGNTWLTAFVLKTFAQARAYIFIDEAHITQALIWLSQRQKDNGCFRSSGSLLNNAIKGGVEDEVTLSAYITIALLEIPLTVTHPVVRNALFCLESAWKTAQEGDHGSHVYTKALLAYAFALAGNQDKRKEVLKSLNEEAVKKDNSVHWERPQKPKAPVGHFYEPQAPSAEVEMTSYVLLAYLTAQPAPTSEDLTSATNIVKWITKQQNAQGGFSSTQDTVVALHALSKYGAATFTRTGKAAQVTIQSSGTFSSKFQVDNNNRLLLQQVSLPELPGEYSMKVTGEGCVYLQTSLKYNILPEKEEFPFALGVQTLPQTCDEPKAHTSFQISLSVSYTGSRSASNMAIVDVKMVSGFIPLKPTVKMLERSNHVSRTEVSSNHVLIYLDKVSNQTLSLFFTVLQDVPVRDLKPAIVKVYDYYETDEFAIAEYNAPCSKDLGNA

SEQ ID NO: 28 - protein, 1324 aa, Homo sapiens
MDENFHPLNELIPLVYIQDPKGNRIAQWQSFQLEGGLKQFSFPLSSEPFQGSYKVVVQKKSGGRTEHPFTVEEFVLPKFEVQVTVPKIITILEEEMNVSVCGLYTYGKPVPGHVTVSICRKYSDASDCHGEDSQAFCEKFSGQLNSHGCFYQQVKTKVFQLKRKEYEMKLHTEAQIQEEGTVVELTGRQSSEITRTITKLSFVKVDSHFRQGIPFFGQVRLVDGKGVPIPNKVIFIRGNEANYYSNATTDEHGLVQFSINTTNVMGTSLTVRVNYKDRSPCYGYQWVSEEHEEAHHTAYLVFSPSKSFVHLEPMSHELPCGHTQTVQAHYILNGGTLLGLKKLSFYYLIMAKGGIVRTGTHGLLVKQEDMKGHFSISIPVKSDIAPVARLLIYAVLPTGDVIGDSAKYDVENCLANKVDLSFSPSQSLPASHAHLRVTAAPQSVCALRAVDQSVLLMKPDAELSASSVYNLLPEKDLTGFPGPLNDQDNEDCINRHNVYINGITYTPVSSTNEKDMYSFLEDMGLKAFTNSKIRKPKMCPQLQQYEMHGPEGLRVGFYESDVMGRGHARLVHVEEPHTETVRKYFPETWIWDLVVVNSAGVAEVGVTVPDTITEWKAGAFCLSEDAGLGISSTASLRAFQPFFVELTMPYSVIRGEAFTLKATVLNYLPKCIRVSVQLEASPAFLAVPVEKEQAPHCICANGRQTVSWAVTPKSLGNVNFTVSAEALESQELCGTEVPSVPEHGRKDTVIKPLLVEPEGLEKETTFNSLLCPSGGEVSEELSLKLPPNVVEESARASVSVLGDILGSAMQNTQNLLQMPYGCGEQNMVLFAPNIYVLDYLNETQQLTPEIKSKAIGYLNTGYQRQLNYKHYDGSYSTFGERYGRNQGNTWLTAFVLKTFAQARAYIFIDEAHITQALIWLSQRQKDNGCFRSSGSLLNNAIKGGVEDEVTLSAYITIALLEIPLTVTHPVVRNALFCLESAWKTAQEGDHGSHVYTKALLAYAFALAGNQDKRKEVLKSLNEEAVKKDNSVHWERPQKPKAPVGHFYEPQAPSAEVEMTSYVLLAYLTAQPAPTSEDLTSATNIVKWITKQQNAQGGFSSTQDTVVALHALSKYGAATFTRTGKAAQVTIQSSGTFSSKFQVDNNNRLLLQQVSLPELPGEYSMKVTGEGCVYLQTSLKYNILPEKEEFPFALGVQTLPQTCDEPKAHTSFQISLSVSYTGSRSASNMAIVDVKMVSGFIPLKPTVKMLERSNHVSRTEVSSNHVLIYLDKVSNQTLSLFFTVLQDVPVRDLKPAIVKVYDYYETDEFAIAEYNAPCSKDLGNA

SEQ ID NO: 29 - protein, 64 aa, Mus musculus
MDLVTYDDVQVNFTQDEWALLDPSQKSLYKGVMLETYRNLTAIGYIWEEHTIEDHFQTSRSHGR

SEQ ID NO: 30 - protein, 311 aa, Mus musculus
MRLQFSWLNSEGLTTTMRLAVICFCLFGIASSLPVKVTDSGSSEEKKLYSLHPDPIATWLVPDPSQKQNLLAPQNAVSSEEKDDFKQETLPSNSNESHDHMDDDDDDDDDDGDHAESEDSVDSDESDESHHSDESDETVTASTQADTFTPIVPTVDVPNGRGDSLAYGLRSKSRSFQVSDEQYPDATDEDLTSHMKSGESKESLDVIPVAQLLSMPSDQDNNGKGSHESSQLDEPSLETHRLEHSKESQESADQSDVIDSQASSKASLEHQSHKFHSHKDKLVLDPKSKEDDRYLKFRISHELESSSSEVN

SEQ ID NO: 31 - protein, 310 aa, Mus musculus
MRLQFSWLNSEGLTTTMRLAVICFCLFGIASSLPVKVTDSGSSEEKLYSLHPDPIATWLVPDPSQKQNLLAPQNAVSSEEKDDFKQETLPSNSNESHDHMDDDDDDDDDDGDHAESEDSVDSDESDESHHSDESDETVTASTQADTFTPIVPTVDVPNGRGDSLAYGLRSKSRSFQVSDEQYPDATDEDLTSHMKSGESKESLDVIPVAQLLSMPSDQDNNGKGSHESSQLDEPSLETHRLEHSKESQESADQSDVIDSQASSKASLEHQSHKFHSHKDKLVLDPKSKEDDRYLKFRISHELESSSSEVN

SEQ ID NO: 32 - protein, 295 aa, Mus musculus
MRLAVICFCLFGIASSLPVKVTDSGSSEEKKLYSLHPDPIATWLVPDPSQKQNLLAPQNAVSSEEKDDFKQETLPSNSNESHDHMDDDDDDDDDDGDHAESEDSVDSDESDESHHSDESDETVTASTQADTFTPIVPTVDVPNGRGDSLAYGLRSKSRSFQVSDEQYPDATDEDLTSHMKSGESKESLDVIPVAQLLSMPSDQDNNGKGSHESSQLDEPSLETHRLEHSKESQESADQSDVIDSQASSKASLEHQSHKFHSHKDKLVLDPKSKEDDRYLKFRISHELESSSSEVN

SEQ ID NO: 33 - protein, 294 aa, Mus musculus
MRLAVICFCLFGIASSLPVKVTDSGSSEEKLYSLHPDPIATWLVPDPSQKQNLLAPQNAVSSEEKDDFKQETLPSNSNESHDHMDDDDDDDDDDGDHAESEDSVDSDESDESHHSDESDETVTASTQADTFTPIVPTVDVPNGRGDSLAYGLRSKSRSFQVSDEQYPDATDEDLTSHMKSGESKESLDVIPVAQLLSMPSDQDNNGKGSHESSQLDEPSLETHRLEHSKESQESADQSDVIDSQASSKASLEHQSHKFHSHKDKLVLDPKSKEDDRYLKFRISHELESSSSEVN

SEQ ID NO: 34 - protein, 294 aa, Mus musculus; identical to SEQ ID NO: 33

SEQ ID NO: 35 - protein, 300 aa, Homo sapiens
MRIAVICFCLLGITCAIPVKQADSGSSEEKQLYNKYPDAVATWLNPDPSQKQNLLAPQTLPSKSNESHDHMDDMDDEDDDDHVDSQDSIDSNDSDDVDDTDDSHQSDESHHSDESDELVTDFPTDLPATEVFTPVVPTVDTYDGRGDSVVYGLRSKSKKFRRPDIQYPDATDEDITSHMESEELNGAYKAIPVAQDLNAPSDWDSRGKDSYETSQLDDQSAETHSHKQSRLYKRKANDESNEHSDVIDSQELSKVSREFHSHEFHSHEDMLVVDPKSKEEDKHLKFRISHELDSASSEVN

SEQ ID NO: 36 - protein, 314 aa, Homo sapiens
MRIAVICFCLLGITCAIPVKQADSGSSEEKQLYNKYPDAVATWLNPDPSQKQNLLAPQNAVSSEETNDFKQETLPSKSNESHDHMDDMDDEDDDDHVDSQDSIDSNDSDDVDDTDDSHQSDESHHSDESDELVTDFPTDLPATEVFTPVVPTVDTYDGRGDSVVYGLRSKSKKFRRPDIQYPDATDEDITSHMESEELNGAYKAIPVAQDLNAPSDWDSRGKDSYETSQLDDQSAETHSHKQSRLYKRKANDESNEHSDVIDSQELSKVSREFHSHEFHSHEDMLVVDPKSKEEDKHLKFRISHELDSASSEVN

SEQ ID NO: 37 - protein, 577 aa, Mus musculus
MALLWLLSVFLLVPGTQGTEDGDMRLVNGASANEGRVEIFYRGRWGTVCDNLWNLLDAHVVCRALGYENATQALGRAAFGPGKGPIMLDEVECTGTESSLASCRSLGWMVSRCGHEKDAGVVCSNDTTGLHILDLSGELSDALGQIFDSQQGCDLFIQVTGQGYEDLSLCAHTLILRTNPEAQALWQVVGSSVIMRVDAECMPVVRDFLRYFYSRRIEVSMSSVKCLHKLASAYGATELQDYCGRLFATLLPQDPTFHTPLDLYAYARATGDSMLEDLCVQFLAWNFEPLTQSESWSAVPTTLIQALLPKSELAVSSELDLLKAVDQWSTETIASHEDIERLVEQVRFPMMLPQELFELQFNLSLYQDHQALFQRKTMQALEFHTVPVEVLAKYKGLNLTEDTYKPRLYTSSTWSSLVMASTWRAQRYEYNRYNQLYTYGYGSVARYNSYQSFQTPQHPSFLFKDKQISWSATYLPTMQSCWNYGFSCTSNELPVLGLTTSSYSNPTIGYENRVLILCGGYSVVDVTSFEGSKAPIPTALDTNSSKTPSLFPCASGAFSSFRVVIRPFYLTNSTDMV

SEQ ID NO: 38 - protein, 585 aa, Homo sapiens
MTPPRLFWVWLLVAGTQGVNDGDMRLADGGATNQGRVEIFYRGQWGTVCDNLWDLTDASVVCRALGFENATQALGRAAFGQGSGPIMLDEVQCTGTEASLADCKSLGWLKSNCRHERDAGVVCTNETRSTHTLDLSRELSEALGQIFDSQRGCDLSISVNVQGEDALGFCGHTVILTANLEAQALWKEPGSNVTMSVDAECVPMVRDLLRYFYSRRIDITLSSVKCFHKLASAYGARQLQGYCASLFAILLPQDPSFQMPLDLYAYAVATGDALLEKLCLQFLAWNFEALTQAEAWPSVPTDLLQLLLPRSDLAVPSELALLKAVDTWSWGERASHEEVEGLVEKIRFPMMLPEELFELQFNLSLYWSHEALFQKKTLQALEFHTVPFQLLARYKGLNLTEDTYKPRIYTSPTWSAFVTDSSWSARKSQLVYQSRRGPLVKYSSDYFQAPSDYRYYPYQSFQTPQHPSFLFQDKRVSWSLVYLPTIQSCWNYGFSCSSDELPVLGLTKSGGSDRTIAYENKALMLCEGLFVADVTDFEGWKAAIPSALDTNSSKSTSSFPCPAGHFNGFRTVIRPFYLTNSSGVD

SEQ ID NO: 39 - protein, 88 aa, Mus musculus
MRLFIALPVLIVVVAMTLEGPAPAQAAPDLSGTLESIPDKLKEFGNTLEDKARAAIEHIKQKEILTKTRAWFSEAFGKVKEKLKTTFS

SEQ ID NO: 40 - protein, 88 aa, Mus musculus; identical to SEQ ID NO: 39

SEQ ID NO: 41 - protein, 83 aa, Homo sapiens
MRLFLSLPVLVVVLSIVLEGPAPAQGTPDVSSALDKLKEFGNTLEDKARELISRIKQSELSAKMREWFSETFQKVKEKLKIDS

SEQ ID NO: 42 - protein, 83 aa, Homo sapiens; identical to SEQ ID NO: 41

SEQ ID NO: 43 - protein, 129 aa, Homo sapiens
MRLFLSLPVLVVVLSIVLEGPAPAQGTPDVSSALDKLKEFGNTLEDKARELISRIKQSELSAKMRLEPFPGHGRAGVCFWVEPWQMVQDEQIEKKTSPGEADNIPLVTQLDLKGVVFRDISESEGETQD

SEQ ID NO: 44 - protein, 83 aa, Homo sapiens; identical to SEQ ID NO: 41

SEQ ID NO: 45 - DNA, 1057 bp, Mus musculus
agccagcagctgacccagcctccagtcaccatgaagactctcctgactctgggactcctcctgctttctgtcactgctcaggccaaggtctatgaacgttgtgagtttgccagaactctgaaaaggaatggaatggctggctactatggagtcagcctggccgactgggtgtgtttagctcagcacgagagcaattataacacacgagctacaaactacaaccgtggagaccaaagcactgactatgggatatttcagatcaatagccgatactggtgtaatgatggcaaaaccccaagagctgtgaatgcctgtgggatcaattgcagtgctctgctgcaggatgacatcactgcagccatacaatgtgcaaagagggtggtgagagatccccaaggcattcgagcatgggtggcatggcgagcacactgtcaaaaccgagatctgtcccagtatattcggaactgcggagtctgaccgcggtgtgcttctactgcagctcattcggtctctttctcactgtaggagtagatatgagagaggtcacattccctcgatttcccctctaagtcacaggacttcagcagaaacagggcaaaacagagacttcctcctcacaagcttcagctgatgctgtgttgtgcaaagtctcccttgtcagtcagcacagccctggacgctggtgacagtcagccaacacaatgatcaccacacagacacctctgtaggtcagttcttcagccaggaagtgattcacattgagttccattggaattcatcttaatcagacctgtgtgaataaaaatacaagaactgcttataggagaccagttgatcttgggaaacagcagtcgtgtgagctgcagggctttgtgcagtcccagcacccagttagaacagcctctgtggtgggccgggaaggtttctgagggcacaggagtctcagtggatgagaactgagattgtctgaactcagaaacttatcagggaacccgtgacctgtctttcttagagctgcccctttcatcttgcttaaaaaataaattctcagctcatg

SEQ ID NO: 46 - DNA, 1490 bp, Homo sapiens
agcctagcactctgacctagcagtcaacatgaaggctctcattgttctggggcttgtcctcctttctgttacggtccagggcaaggtctttgaaaggtgtgagttggccagaactctgaaaagattgggaatggatggctacaggggaatcagcctagcaaactggatgtgtttggccaaatgggagagtggttacaacacacgagctacaaactacaatgctggagacagaagcactgattatgggatatttcagatcaatagccgctactggtgtaatgatggcaaaaccccaggagcagttaatgcctgtcatttatcctgcagtgctttgctgcaagataacatcgctgatgctgtagcttgtgcaaagagggttgtccgtgatccacaaggcattagagcatgggtggcatggagaaatcgttgtcaaaacagagatgtccgtcagtatgttcaaggttgtggagtgtaactccagaattttccttcttcagctcattttgtctctctcacattaagggagtaggaattaagtgaaaggtcacactaccattatttccccttcaaacaaataatatttttacagaagcaggagcaaaatatggcctttcttctaagagatataatgttcactaatgtggttattttacattaagcctacaacatttttcagtttgcaaatagaactaatactggtgaaaatttacctaaaaccttggttatcaaatacatctccagtacattccgttctttttttttttgagacagtctcgctctgtcgcccaggctggagtgcagtggcgcaatctcggctcactgcaacctccacctcccgggttcacgccattctcctgcctcagcctcccgagtagctgggattacgggcgcccgccaccacgcccggctaattttttgtatttttagtagagacagggtttcaccgtgttagccaggatggtctcgatctcctgaccttgtgatccacccacctcggcctcccaaagtgctgggattacaggcgtgagccactgcgcccggccacattcagttcttatcaaagaaataacccagacttaatcttgaatgatacgattatgcccaatattaagtaaaaaatataagaaaaggttatcttaaatagatcttaggcaaaataccagctgatgaaggcatctgatgccttcatctgttcagtcatctccaaaaacagtaaaaataaccactttttgttgggcaatatgaaatttttaaaggagtagaataccaaatgatagaaacagactgcctgaattgagaattttgatttcttaaagtgtgtttctttctaaattgctgttccttaatttgattaatttaattcatgtattatgattaaatctgaggcagatgagcttacaagtattgaaataattactaattaatcacaaatgtgaagttatgcatgatgtaaaaaatacaaacattctaattaaaggctttgcaacaca

SEQ ID NO: 47 - DNA, 531 bp, Mus musculus
tgcagaaaaagcagccaggttcaaagtggcctgcagactgtcctgaactcatctctcaaagctgctacagagcccaggaagatttcaggatgaagagcttcctcctcttcctcactatcattcttctggttgtgattcagatacaaacaggatccttgggacaagccactacggccgcttctggtactaacaaaaacagcacctccaccaaaaaaacccccttaaagagtggggcctcatccatcatcgatgcgggtgcctgcagtttcctcttctttgccaataccttaatgtgcctcttctacctcagctgaggtgaaggcgcagcttctgaagccccgtgctccacccactgctgccaccatcagtagcgagagacatcccaacccacgggaagggttgatagcagatatccaaggaggctaaagttgacagccaatggccggaatgggagcggggccgtgacacccagctagggcacaataaagttatacttatgcttaaaaaaaaaaaaaaaaaaaaaaaaaaaaa

SEQ ID NO: 48 - DNA, 467 bp, Homo sapiens
agacagccctgagatcacctaaaaagctgctaccaagacagccacgaagatcctaccaaaatgaagcgcttcctcttcctcctactcaccatcagcctcctggttatggtacagatacaaactggactctcaggacaaaacgacaccagccaaaccagcagcccctcagcatccagcaacataagcggaggcattttccttttcttcgtggccaatgccataatccacctcttctgcttcagttgaggtgacacgtctcagccttagccctgtgccccctgaaacagctgccaccatcactcgcaagagaatcccctccatctttgggaggggttgatgccagacatcaccaggttgtagaagttgacaggcagtgccatgggggcaacagccaaaataggggggtaatgatgtaggggccaagcagtgcccagctgggggtcaataaagttacccttgtacttgca

SEQ ID NO: 49 - DNA, 4222 bp, Mus musculus
aaactaatactgtgatttcacaaaagaagagaaaggcaggttttgaagtcaaagagagtgaaacaaaagccagacagagccttctgacagagtcttgttggtgaatgcttagggctggtatatggccaaaaccatctgcgccatgaacagcttcatggccttggtcctcatctggatgataatagcgtgtgctgaagcagacaagcctcttggagaaacgggtaccactggatttcaaatatgcaagaatgccctgaaactacctgtcttggaggtcctaccaggaggaggctgggataatctgagaaatgtagacatgggacgggtgatggacttgacatacaccaactgtaagaccacagaagatgggcagtacatcatccccgatgaagtgtatactattcctcagaaagagagcaacctggagatgaactcagaagtcctggagtcctggatgaattaccagagtaccacctcactttctatcaacacagaactcgcccttttctccagagtcaacggcaagttctctactgagttccaaaggatgaagacccttcaagtaaaggaccaagctgtgactaccagggttcaggtaagaaaccggatctacacagtgaaaaccaccccaacttcagagctcagcttggggtttacgaaggcacttatggacatctgtgaccaactagagaaaaaccagacgaagatggccacctacctggcagagctcttgatcctcaactatggcacacacgtaatcactagtgtggatgctggggctgcactggttcaggaggatcacgtaaggtcctccttccttctggacaaccagaatagccagaacaccgtgaccgcttctgcagggattgccttcttaaacattgtgaacttcaaagttgaaacagactacatttctcagaccagtttgacgaaggactacctgtcgaacaggaccaactccagggtgcagagttttggaggggttcccttctatccaggcatcaccttagaaacctggcagaagggcatcactaaccacctagtggcaatagaccgtgctggcttgcctctgcatttcttcattaaacctgacaagctacctggcttgccaggtcccttggtgaagaagctgtcgaagacagtggaaactgctgtgagacactattacacttttaacactcacccaggatgcacaaatgttgattcccccaactttaattttcaagccaatatggatgatgattcctgtgatgcgaaagtcaccaacttcacctttggtggagtttatcaggaatgcactgaactgtcaggtgatgttctttgccaaaacctggagcagaagaacctgctcacaggtgatttctcttgtccccctggctacacccctgtccatctgctctcccagacccatgaagagggttacagtcgtctggaatgtaaaaagaaatgcaccctcaagattttctgcaagacagtgtgtgaagatgtgttcagagtggccaaggctgaatttagggcttattggtgtgtggctgctggccaagtacctgacaactcaggacttctctttggaggagtcttcactgacaagaccatcaaccctatgacaaatgcacagtcatgcccagcaggctacatcccactgaacctgtttgaaagcctcaaggtatgtgtgtccctggattatgagttggggttcaagttttcagtcccctttggtgggttcttcagttgtataatggggaaccccttggttaattctgatacagctaaagacgtcagagcaccatctctgaaaaagtgtcccgggggcttcagccaacacctagctgttatcagtgatggatgccaagtgtcctactgtgtcaaggctggaatcttcacaggagggtccctgctccctgtcaggctcccaccttataccaaaccacctcttatgagccaggttgccaccaacactgtcatagtgaccaatagtgagactgccagatcctggattaaggatcctcagaccaaccagtggaagctgggagaacctctggagcttcgtagggccatgacagtcatccatggggacagtaatggaatgtcaggaggggaagctgctggaatcactttgggagtcaccatagcactaggagttgtcattaccttggccatctatggtactcggaagtacaagaagaaggaataccaggaaattgaggagcaggagagtttggttggaagcttagcaacagatgcaacagtccttaatggagaagaggatccaagtccagcttaattgtctccaaaggaaacagtttccagccacagcttcaagcacatcttttgctttgttttctctacttctgccttcctaagtgactgaagtgacagtcgccataggaagaaagcagctattacaaccctggcagtattttcttaggcctctgcaccaggaaattaaaggagccatttgaagtgaggtgtggggaggggtatgattcatttggaaaaagctggactgggactaagcctcggggtgtatgcgtccattctcatagttgtctgtacctgaatgcatgtgtgtggaacgaggggtgggggagaaattggatttggtgcatttagtctgaatttgaaaggctttccagtttgtaagctgaagaggtctgtgctttaagtacattacttcttttcttgtgttttcaaagaggccctcagggtttcagtaaacagtgccctgaaatgccacaggaggcctacatgccccctactctttagctttaaggacttggtgttgattgacagtgccctccccatgagtcacctcacaggcatttgaaggagaagcgggtggggtttatacaaattccatttcccaacttcctcacagctaatctaggtcagtcttgggcttctgaactgtgcaaacaagtcctgggggggggggggggaatataacataattttctgttaggggatgaaggatgaagaaacagtaaggaaatgagtaataaattaaggctaaaaaccggggttcgggagacaatgagagtattctaggaaactttgaattcttagatctgtcaattaacagggttataaatgaagaactaaacagagctctagtttggcagatcaagcagtatggtttcacgttcatgtgtcaaaaatgtaactccttcctctctctggacagtctttccccttgtcttcttaccacagctgagggtgcacaggaatacacacaaaccccttggactgtagcaagaagcttttatctgcctaggggtgaaaaatgcgcaagtcacagtgagcctgcacttacatagtacttcctccctaaaactaaagctattgggaaagcgctgtcttctgtctgttaggatttgccttttcgcgctgcttggaagaggggtggggtaatttaaaacaaaacaaaatttatgtcacagttagctgggaaaaggccatgatatgtatttcagttccaggatggcttccatgggttatctggaaggcctcgtgattgacaactggcaatagttggggtattgctcaattttcatatctgagaatttaattctctacaacacggaaattcctctacagctgtcttagaaattatgtatctattcaccacaacacatcagtgagctatcttctacgaaagatgatgtattcttgctttaacacttacaatcaagctcttgtgcacagagtaggccctcctgaagagctccaagtgtctcagccttcaggaacagggagagacttcctcattcgtttccatttgagatacagagaggaatgaatgactgaattggaattctgccctaccacctgcccagccaagagggctaattgcacaacctctccatcgaacctgcctcttgagcgttaaaatgttcttcttaacctctgtgtgctttgtgggtttgggctatattttaatgtttcattgaagccagccatctttctgaaaatactagttacaatcaagctcttgtgcacagagtaggccctcctgaagagctccaagtgtctcagccttcaggaacggggagagacttctttctgtaaattctctgaatctgcaaagcaaggcacatcagaagactcccagatctttaatgcagaaacttcctgttgaattttttaatatttgtcccataaacatgtaactctactaacaaaaatgagtataaatatgcattaaaatgtgtacttggcaaaa

SEQ ID NO: 50 - DNA, 4345 bp, Mus musculus
aaactaatactgtgatttcacaaaagaagagaaaggcaggttttgaagtcaaagagagtgaaacaaaagccagacagagccttctgacagagctttcacttctctgttttgcaattggagcagcataaagaggaactgatggttttaggagaactgtagaattttctgtttcaacaaccgctttcttttccatccttctgtttgccccagtcttgttggtgaatgcttagggctggtatatggccaaaaccatctgcgccatgaacagcttcatggccttggtcctcatctggatgataatagcgtgtgctgaagcagacaagcctcttggagaaacgggtaccactggatttcaaatatgcaagaatgccctgaaactacctgtcttggaggtcctaccaggaggaggctgggataatctgagaaatgtagacatgggacgggtgatggacttgacatacaccaactgtaagaccacagaagatgggcagtacatcatccccgatgaagtgtatactattcctcagaaagagagcaacctggagatgaactcagaagtcctggagtcctggatgaattaccagagtaccacctcactttctatcaacacagaactcgcccttttctccagagtcaacggcaagttctctactgagttccaaaggatgaagacccttcaagtaaaggaccaagctgtgactaccagggttcaggtaagaaaccggatctacacagtgaaaaccaccccaacttcagagctcagcttggggtttacgaaggcacttatggacatctgtgaccaactagagaaaaaccagacgaagatggccacctacctggcagagctcttgatcctcaactatggcacacacgtaatcactagtgtggatgctggggctgcactggttcaggaggatcacgtaaggtcctccttccttctggacaaccagaatagccagaacaccgtgaccgcttctgcagggattgccttcttaaacattgtgaacttcaaagttgaaacagactacatttctcagaccagtttgacgaaggactacctgtcgaacaggaccaactccagggtgcagagttttggaggggttcccttctatccaggcatcaccttagaaacctggcagaagggcatcactaaccacctagtggcaatagaccgtgctggcttgcctctgcatttcttcattaaacctgacaagctacctggcttgccaggtcccttggtgaagaagctgtcgaagacagtggaaactgctgtgagacactattacacttttaacactcacccaggatgcacaaatgttgattcccccaactttaattttcaagccaatatggatgatgattcctgtgatgcgaaagtcaccaacttcacctttggtggagtttatcaggaatgcactgaactgtcaggtgatgttctttgccaaaacctggagcagaagaacctgctcacaggtgatttctcttgtccccctggctacacccctgtccatctgctctcccagacccatgaagagggttacagtcgtctggaatgtaaaaagaaatgcaccctcaagattttctgcaagacagtgtgtgaagatgtgttcagagtggccaaggctgaatttagggcttattggtgtgtggctgctggccaagtacctgacaactcaggacttctctttggaggagtcttcactgacaagaccatcaaccctatgacaaatgcacagtcatgcccagcaggctacatcccactgaacctgtttgaaagcctcaaggtatgtgtgtccctggattatgagttggggttcaagttttcagtcccctttggtgggttcttcagttgtataatggggaaccccttggttaattctgatacagctaaagacgtcagagcaccatctctgaaaaagtgtcccgggggcttcagccaacacctagctgttatcagtgatggatgccaagtgtcctactgtgtcaaggctggaatcttcacaggagggtccctgctccctgtcaggctcccaccttataccaaaccacctcttatgagccaggttgccaccaacactgtcatagtgaccaatagtgagactgccagatcctggattaaggatcctcagaccaaccagtggaagctgggagaacctctggagcttcgtagggccatgacagtcatccatggggacagtaatggaatgtcaggaggggaagctgctggaatcactttgggagtcaccatagcactaggagttgtcattaccttggccatctatggtactcggaagtacaagaagaaggaataccaggaaattgaggagcaggagagtttggttggaagcttagcaacagatgcaacagtccttaatggagaagaggatccaagtccagcttaattgtctccaaaggaaacagtttccagccacagcttcaagcacatcttttgctttgttttctctacttctgccttcctaagtgactgaagtgacagtcgccataggaagaaagcagctattacaaccctggcagtattttcttaggcctctgcaccaggaaattaaaggagccatttgaagtgaggtgtggggaggggtatgattcatttggaaaaagctggactgggactaagcctcggggtgtatgcgtccattctcatagttgtctgtacctgaatgcatgtgtgtggaacgaggggtgggggagaaattggatttggtgcatttagtctgaatttgaaaggctttccagtttgtaagctgaagaggtctgtgctttaagtacattacttcttttcttgtgttttcaaagaggccctcagggtttcagtaaacagtgccctgaaatgccacaggaggcctacatgccccctactctttagctttaaggacttggtgttgattgacagtgccctccccatgagtcacctcacaggcatttgaaggagaagcgggtggggtttatacaaattccatttcccaacttcctcacagctaatctaggtcagtcttgggcttctgaactgtgcaaacaagtcctgggggggggggggggaatataacataattttctgttaggggatgaaggatgaagaaacagtaaggaaatgagtaataaattaaggctaaaaaccggggttcgggagacaatgagagtattctaggaaactttgaattcttagatctgtcaattaacagggttataaatgaagaactaaacagagctctagtttggcagatcaagcagtatggtttcacgttcatgtgtcaaaaatgtaactccttcctctctctggacagtctttccccttgtcttcttaccacagctgagggtgcacaggaatacacacaaaccccttggactgtagcaagaagcttttatctgcctaggggtgaaaaatgcgcaagtcacagtgagcctgcacttacatagtacttcctccctaaaactaaagctattgggaaagcgctgtcttctgtctgttaggatttgccttttcgcgctgcttggaagaggggtggggtaatttaaaacaaaacaaaatttatgtcacagttagctgggaaaaggccatgatatgtatttcagttccaggatggcttccatgggttatctggaaggcctcgtgattgacaactggcaatagttggggtattgctcaattttcatatctgagaatttaattctctacaacacggaaattcctctacagctgtcttagaaattatgtatctattcaccacaacacatcagtgagctatcttctacgaaagatgatgtattcttgctttaacacttacaatcaagctcttgtgcacagagtaggccctcctgaagagctccaagtgtctcagccttcaggaacagggagagacttcctcattcgtttccatttgagatacagagaggaatgaatgactgaattggaattctgccctaccacctgcccagccaagagggctaattgcacaacctctccatcgaacctgcctcttgagcgttaaaatgttcttcttaacctctgtgtgctttgtgggtttgggctatattttaatgtttcattgaagccagccatctttctgaaaatactagttacaatcaagctcttgtgcacagagtaggccctcctgaagagctccaagtgtctcagccttcaggaacggggagagacttctttctgtaaattctctgaatctgcaaagcaaggcacatcagaagactcccagatctttaatgcagaaacttcctgttgaattttttaatatttgtcccataaacatgtaactctactaacaaaaatgagtataaatatgcattaaaatgtgtacttggcaaaatttta

SEQ ID NO: 51 - DNA, 4418 bp, Homo sapiens
agtttgcccaaagcttgctggccgctgtgtagggctggtgagtggctggggctgtctgagccatgaacaacttcagggccaccatcctcttctgggcagcggcagcatgggctaaatcaggcaagccttcgggagagatggacgaagttggagttcaaaaatgcaagaatgccttgaaactacctgtcctggaagtcctacctggagggggctgggacaatctgcggaatgtggacatgggacgagttatggaattgacttactccaactgcaggacaacagaggatggacagtatatcatccctgatgaaatcttcaccattccccagaaacagagcaacctggagatgaactcagaaatcctggaatcctgggcaaattaccagagtagcacctcctactccatcaacacagaactctctcttttttccaaagtcaatggcaagttttccactgagttccagaggatgaagaccctccaagtgaaggaccaagctataactacccgagttcaggtaagaaacctcgtctacacagtcaaaatcaacccaactttagagctaagctcaggttttaggaaggaactccttgacatctctgaccgtctagagaacaaccagacgaggatggccacctacctggcagaactcctggtgctcaactatggcacccacgtcaccaccagtgtcgacgctggggctgctcttattcaggaggaccacctcagggcctccttcctccaagacagccagagcagtcgtagtgccgtgaccgcctctgctggacttgcctttcaaaacaccgtgaacttcaaatttgaggaaaactatacctcgcagaatgtcctcaccaagagctacctctcaaaccgaaccaactccagggtgcagagcattggaggggttcctttttacccaggcatcaccctccaggcctggcagcagggtatcaccaaccacctggtggccatcgaccgctctggcctgccgctgcatttcttcatcaaccccaacatgctacctgacttgccaggccccctggtgaagaaggtgtcaaagacagtggaaactgctgtgaagcgctattatacattcaacacctaccctggctgcacagatctcaattctcccaacttcaattttcaggccaacacggatgatggctcctgcgaggggaaaatgaccaacttctctttcggtggggtttatcaggaatgcactcagctctcagggaatagggatgtcctcctctgccaaaagttggagcagaagaatccactcactggtgatttctcctgcccctctggctactccccggtgcacctgttatcccagatccacgaggagggttacaaccacctggagtgtcatcgaaagtgcactctcctcgtcttctgcaagaccgtgtgtgaagatgtgttccaggtggcaaaagctgaatttagggctttttggtgtgtggccagcagccaagtacctgaaaactcaggactgctttttgggggcctcttcagcagcaagagcataaaccccatgacaaatgcacagtcatgcccagccggctactttccactgagactctttgaaaacctcaaggtatgtgtttctcaggactatgagttgggaagcaggtttgcggtcccctttggcgggttctttagctgcacagttgggaaccccctggtagatcctgctatatccagagatttaggggcaccgtctctgaaaaagtgccccgggggcttcagccagcacccagccctcatcagcgatggatgccaagtgtcctattgcgtcaaatccgggctcttcacaggagggtccctgccccctgccaggctcccacctttcacccggccacccctcatgagtcaggctgccaccaatactgtcatagtgaccaattctgagaatgcgagatcctggattaaagactcccagacccaccagtggaggctgggagaaccgatagagctgcggagggccatgaatgtcatccatggggatggtggtggtctgtcaggaggggctgcagctggggtcacagtgggggtcaccaccattctggctgttgttatcaccttggccatctacggcacccggaagttcaagaagaaagcatatcaggcaattgaggaaaggcagagtttggttccaggcactgcagcaactggagacaccacttaccaagagcaggggcagagtccagcttaaatctctccccgaaaatggtttctctcatctccagtgtggtcattgctgaccactctgttttcctaagcattgaaatggcaagtgcaaccaaaagtaggtatattcgtgacttcttgtttaggtctctgggccaggaaattcatactgttacatggataaggttgggattggggagagggaacagttgggactagaagcaaaagtgattctgggactaaaataggaagcagatgtcctttcccaatgtgtgttgctgtcttcacctgaatgcatttgtgtaaaaatagcggagggacaatgtgaacatttgtatttggaagctatgaatttactctgaagtttgcagttgtttccaatttgtgagctctaagagtttctgcctgtaagaactactctccttttattttgatttttaaaaacctgtctgaatttcacactcttagagcctggaagagccctgaaaagacacaagtcttgcctggctactgctttttaactttgagggctctatgttgacagactgttatctcctctgggtgacctcaaacatctgaaaagaaagatgttgcctgtgccaattccactttttccagctgccccttgatgaacactcccttataccagaccactcttggacttctgactggtgtcatcaagtcctcagaaaatattttaagttattttaagttattaaggaagggatgatttggagacaaggagtaatgaaagatgggtaaaaactggaaaagattctggtgctaagtactaccccttcatcttccatggatggtcattacctttcctgtcctcctgttatatgaacacacacacacacacacacacacacacacacacacacgcacacacataccacatttcaataagtcttcattgttctgggtccttacctttcctgtcctcctgttatatgaacacacacacacacacacacacacacacacacgcacaccacatttcaatgtctgcatggttctgggggtaacaaaggcaagaagttaaagtaagaccacatttgagtattacttactctgtagaatcaaaacagagtagttaacaccaattatgcaaactacttttttttccagcagaaagggagctgacatgatcaaatccatgttttcaaatgaactgaaaaaggcatccagcaccacttataacacatttatttcagttccaggctgacagccctggggcatctagcaggatgcataattgtcatctggtgagagttgggactttgctcaattttaataccaatctctcctgattgtaattacctccactactttcatgatccccctacaatatttttttaaatgatatatttattcactgaatcaaatgtcattaatgagttatcttctgtggaggatgactgttctctttgttaatgttcacaatcaagatcttgggctgagaagaggcccttcacccaaggagtttgaagtatcacagtgtgtgggaaggtgggaaccaggatacccattcatttccaaccgagacacagagaagtgagtcacagaatttgagcccgctctcttgactgcccagccagagacactgatttctgtaacctcttcacttgatcctgcctcttaagcattaaaacattctcctaaacctctgagtgttttgtgggttctgggtgttttgtacattttagccaagctaaccacttgtctgcaagtactgactttcctatgaattctttgaagattattgagtcagaaaggaaaaatatagccccaaattcccaggcttttaatgcattacattaactgcctattgaaatgagaagttcttcacaaacttgtatacccactaacaagattgcacataaacatgcattaaagtatatactaagaaaccctctgtccaacggctcatgcatatgaagtccgaacatgggagtttgccaattgcattcatcaagtcgttttgcggagtcagatccctgatggaagagctcacaggctctgccttccaagtcctgggttcctaactggtgaccttagcctggggtctgtggggagaccaaccctggcttccaagaaaaccacattccatggactatcagaaatagacacagatttgggtgacaaagctggctctgtatttgcattttatttttgtgttcttgtcagtttgggaatgattaatattaaacatttatttgagaaacaa

SEQ ID NO: 52 - DNA, 536 bp, Mus musculus
agagacactggttcctgactcctctagctttcatttcgaagtctttgacctcaacatgaagatttccacacttctatgcctcctgctcatagctaccaccatcagtcctcaggtattggctggaccagatgcggtgagcaccccagtcacgtgctgttataatgttgttaagcagaagattcacgtccggaagctgaagagctacaggagaatcacaagcagccagtgtccccgggaagctgtgatcttcaggaccatactggataaggagatctgtgctgaccccaaggagaagtgggttaagaattccataaaccacttggataagacgtctcaaaccttcatccttgaaccttcatgtctaggctgagagttccaaaaactcttacgtatttccccctgaagttccccacgggcagtgtgatatttattatgatatctaaaaagagatgtttttaataatttaaacaaacttgcttaaataatatttaatggtatttaagtaatatttgggccaattaaaccgaatctaattt

SEQ ID NO: 53 - DNA, 741 bp, Homo sapiens
gagaggctgagactaacccagaaacatccaattctcaaactgaagctcgcactctcgcctccagcatgaaagtctctgccgcccttctgtgcctgctgctcatagcagccaccttcattccccaagggctcgctcagccagatgcaatcaatgccccagtcacctgctgttataacttcaccaataggaagatctcagtgcagaggctcgcgagctatagaagaatcaccagcagcaagtgtcccaaagaagctgtgatcttcaagaccattgtggccaaggagatctgtgctgaccccaagcagaagtgggttcaggattccatggaccacctggacaagcaaacccaaactccgaagacttgaacactcactccacaacccaagaatctgcagctaacttattttcccctagctttccccagacaccctgttttattttattataatgaattttgtttgttgatgtgaaacattatgccttaagtaatgttaattcttatttaagttattgatgttttaagtttatctttcatggtactagtgttttttagatacagagacttggggaaattgcttttcctcttgaaccacagttctacccctgggatgttttgagggtctttgcaagaatcattaatacaaagaattttttttaacattccaatgcattgctaaaatattattgtggaaatgaatattttgtaactattacaccaaataaatatatttttgtacaaaa

SEQ ID NO: 54 - DNA, 986 bp, Mus musculus
agcaagaaaccacgccccactgaagctaccccaccatgccctggtcctggagctgtacttgccgagcacttggcccactacatgctccctgcatttccccagccatgtggctggccattctgcttgccctctgctgcctaacttctgacacccatggggcacgccccccagatttttgttccaaagatttgatctccagtgtgaagccaggattccccaaaacaatagagaccaataacccaggagtgcttaaggccgccaggcacagtgtggaaaagttcaacaactgcacaaatgacatctttttgttcaaggagtcccatgtcagcaaagccctggtacaggtggtgaaaggcctgaaatatatgctggaggtgaaaatcggccgaactacatgcaggaagaccatgcatcaccaactggacaactgtgacttccaaaccaaccctgccttgaagcggactctatattgctactctgaagtctgggtcatcccctggctccacagttttgaggtgcctgttctcctctgccagtgacttctgtctctttagcaagactgcagctgtgatacatatccactcgtgttttccccactccttactttccaccccatcctggccatctcagatcctcagggcctgcttaccagcgagcagattaacatgccagtgggtcatcagggggctggactgggagaatatagtgccctcctctccagattaactgtattcacactttcttctaaaatgaattctctggtgctacacacctagattcaggatgtgggcacgcagagagtcctttgatgacattactggagcacgtgcagagcaaagcagatacagtcaacaaggtggtagtgtgggaagcttcttgatgcccgactgcatgagcagattctgcagccgtctggtctgctaccatcagactaatattgatggggatgatttatcataaataaaaagctgatcacctaaaagcaa

SEQ ID NO: 55 - DNA, 891 bp, Homo sapiens
actgttccatgctgcccaagaaggctcagcacaggcacaaaccattgcccggcactggcccgtgctgcctgagaaggattggcacgggcacagaccactgcccccacctgccctgcgccatctacccaagaaggctcggcacgggcaccaaccactgcctccaactgccccatgctgcctgagaaggcactgcacggccacccccaactgccccgcactgtccctacccgggcagccatgcgagcggctggaactctgctggccttctgctgcctggtcttgagcaccactgggggcccttccccagatacttgttcccaggaccttaactcacgtgtgaagccaggatttcctaaaacaataaagaccaatgacccaggagtcctccaagcagccagatacagtgttgaaaagttcaacaactgcacgaacgacatgttcttgttcaaggagtcccgcatcacaagggccctagttcagatagtgaaaggcctgaaatatatgctggaggtggaaattggcagaactacctgcaagaaaaaccagcacctgcgtctggatgactgtgacttccaaaccaaccacaccttgaagcagactctgagctgctactctgaagtctgggtcgtgccctggctccagcacttcgaggtgcctgttctccgttgtcactgacccccgcctcttcagcaagaccacagccatgacaaacaccaggatgcatgctccttgtcccctcccacccgcctcatgacccagcctcacagaccctctcaggcctctgacgagtgagcgggtgaagtgccactgggtcaccgcagggcagctggaatggcagcatggtagcacctcctaacagattaaatagatcacatttgcttctaaaattaa

SEQ ID NO: 56 - DNA, 3036 bp, Mus musculus
cttccgtttcctcccgcctcttgagctggggtgctgctcctcactgccgggtacctcctagccactccataccactggtgtccacagcaacgctcctggcccccaactgtcatccctggctgctgggcctcagatgcaatgcaggccatcaagtgtgtggtggtgggtgatggagccgtgggcaagacgtgtcttctcatcagctacaccaccaacgccttccctggagaatacatccccactgtatttgacaactactcagccaatgtgatggtggacagtaagccggtgaacctggggctgtgggataccgcaggtcaggaggactatgaccgcctccggccactctcctacccacagacagatgtatttctcatctgcttctcgctagtcagcccagcctcctatgagaatgtccgtgccaagtggttccctgaggtacggcaccactgccccagcacccccatcatcctggtgggtaccaagctggaccttcgcgatgacaaggacaccatcgagaagctgaaggagaagaagctggctcccatcacctacccgcagggcctggcactggccaaggatattgattcagtcaagtacttggaatgttctgcactcacccagcgaggcctgaagaccgtcttcgatgaggcaatccgcgcagtcctctgcccacagcccacacgacagcagaagcgcccctgcagcctgctctaggggtgtcaccccagtcctcccatcccaatggtcctgaccctccagggtccccaccaaagctcagtgacgtgctggtggaattgctgtttctccgtgtggcgttctttcccagttagctgcagaacttgcctctctcctccacggaggtccctggggatgggcggatgttcataggccacatcctatttgggaggctcctatgttcccaggggccatcagggacccccaagatgcagccatccatcctcatacagagtcatatgcccacctgctccaggccttcctgacacctctctcgaagcttccggtctccatggcctgccactagtgtgttcgccatgttgggataccttcttccctgaaccaaagggagagatgtggaaatctgctcctctgttctcctttttcagaaaagcacagaacaaatctacttcagtaaatctctcatctgcccagccaagtgagggtctgagctcagccaacccctactgtctctcgagacctcctactctacttgaagggtagagctgttccttcttgggactgtccactccacctgccagtcaggacccgatccatagcaaatggaaaatacagctctcttgcttacacagaaaataaatgtgttgattcttttggtggaagtgcagtgagttcaggcacagcttgatcaaggtggggcgaagggatcagatgacaccacggagcctggcttcctgcctgttttgggtctgcctgctgctgccaggctcatttttctggccattgattcttgggacttgatcctccgaggtcaagttcaggtgatgtctgccccaggcaagctctaaggaaaggtcactctggttgaaccagcttgtcttaggcccaccttcaatcacacaagtgtgtcagagagaggctgcactgtggctggctgtgagttgtgttagagccaggagcagaggtgatgccagggagctggggtatagaatgggtgtgtgtggcgttgggggaataaattctttagggaacaaccttcttaaaactgggtgggtatccagtagctagggttctataacccccgactgtcagaggtcacggtaagtgtcctttctaccattatcagggacagtttctgccccagctggcactaagaaaaacagattttttaaatttgtttttttttgtttgtttgttttgttttgttttgttttgttttgtttgagacagggtttctctgtgtagctctggctgtcctggaactcactttgtagaccaggctgtcctcgaactcagaaatctgcctgcctctgcctcctaagtgctgggattaaaggcgtgcaccaccattgcccggctcatttgtttttgagataagattttattatatagcctgggctgacctcagacctgccatcctcctgcctcagcttcctaaattctgggtttacagatgtatacttccgtgcctggataaggttgaaattcttactagagagttctatggaagttgatgtggtgtccatatcaggcacccagggcctgggcctgagacagtcctacctacatcttccctgaattatcaatctatggtcaagaccgtggcactgtctgagcttccacgtccttctcccaacacacttttgatggcctgtctgtgtcaggtgctaccatagtctcagagattcagtgacatatgtgttgttctccacccctcccccaccccccagccctgagtctccgaggctgagagaaaatggctcccccgacattggaaagctagccctaaggagctcagcattttctgtctccaagagttccagagctgccccccaactcctcccccccaaacttaagggactccacctctggaggggcttggcccagtgagggaagcttctgttcttagcttggctcacaggagggcaagatttctctgacacagaaagaaaggttttaagcccacaggtgctgtgttctccaacacggttgagaggacctgcacccccatcgctttggggagttaaagacctggggtgcacccagagtccctcttttagctctctgctccttttctagtgcatgatactaagcaaaaccttacatgattcaaaaccgtagatctaagcccagaacctctcaaactaagcctctaagtagctaaacctccccctcctcctcccccgcccccttctgtaggaggcaaaccccggcctgttaccttgagcctctgtgtgagttgtggagcacacagccagcccactgtcaccctgacagcttatttcacccagatctcagctttcactttaatctgaataaagtccccgatacttttgc

SEQ ID NO: 57 - DNA, 1472 bp, Homo sapiens
ctcctgccccaccaccgctgctcctcagcaggcgcctcaccagcctccacaccccttgcgcccgcagaaacgcgcctggccctgagctgtcaccaccgacactctccaggctccggacacgatgcaggccatcaagtgtgtggtggtgggagatggggccgtgggcaagacctgccttctcatcagctacaccaccaacgcctttcccggagagtacatccccaccgtgtttgacaactattcagccaatgtgatggtggacagcaagccagtgaacctggggctgtgggacactgctgggcaggaggactacgaccgtctccggccgctctcctatccacagacggacgtcttcctcatctgcttctccctcgtcagcccagcctcttatgagaacgtccgcgccaagtggttcccagaagtgcggcaccactgccccagcacacccatcatcctggtgggcaccaagctggacctgcgggacgacaaggacaccatcgagaaactgaaggagaagaagctggctcccatcacctacccgcagggcctggcactggccaaggagattgactcggtgaaatacctggagtgctcagctctcacccagagaggcctgaaaaccgtgttcgacgaggccatccgggccgtgctgtgccctcagcccacgcggcagcagaagcgcgcctgcagcctcctctaggggttgcaccccagcgctcccacctagatgggtctgatcctccaggatccccacccaaagcctgatggcaccccggctggccatgctgtcccctccctgtggcgtttcttagcagatggctgcagagcttcgttgatggtcttttctgtactggaggcctcctgaggccaggaacgtgcaaatttgcaggtgctgcatcccaagcccctcatgctcctgccttcctgagggccagaggggagccccaggacccattaagccacccccgtgttcctgccgtcagtgccaactgccgcatgtggaagcatctacccgttcactccagtcccaccccacgcctgactcccctctggaaactgcaggccagatggttgctgccacaacttgtgtaccttcagggatggggctcttactccctcctgaggccagctgctctaatatcgatggtcctgcttgccagagagttcctctacccagcaaaaatgagtgtctcagaagtgtgctcctctggcctcagttctcctcttttggaacaacataaaacaaatttaattttctacgcctctggggatatctgctcagccaatggaaaatctgggttcaaccagcccctgccatttcttaagactttctgctgcactcacaggatcctgagctgcacttacctgtgagagtcttcaaacttttaaaccttgccagtcaggacttttgctattgcaaatagaaaacccaactcaacctgcttaagcagaaaataaatttattgattcaa

SEQ ID NO: 58 - DNA, 2085 bp, Mus musculus
ggggacaacatgccaggcaagcggcaaccctgaacatcgggagtcagctatcacagaggctggcagctggctggtttcagctctgtagactgcagaacacagaagatggccttcattgcagctctggggctcttgatggctgggatctgccctgctgtcctctgcttcccagatggcacgttgggaatggatgctgcagtccaagaagaccatgacaatgggacacaactggacagtctcacattggcctccatcaacactgactttgccttcagcctctacaaggagctggttttgaagaatccagataaaaatattgtcttctccccacttagcatctcagcggccttggccgtcatgtccctgggagcaaagggcaacaccctggaagagattctagaaggtctcaagttcaatcttacagagacctctgaggcagacatccaccagggctttgggcacctcctacagaggctcaaccagccaaaggaccaggtacagatcagcacgggtagtgccctgtttattgaaaagcgccagcagatcctgacagaattccaggagaaggcaagggctctgtaccaggctgaggccttcacagcagacttccagcagcctcgtcaggccaaaaagctcatcaatgactatgtgaggaaacagacccaggggatgatcaaggaactggtctcagacctggataaaaggacattgatggtgctggtgaattatatctactttaaagccaaatggaaggtgccctttgaccctcttgacacgttcaagtctgagttctacgcgggcaagaggaggcccgtgatagtgcccatgatgagcatggaggacctgaccacaccctacttccgagatgaggagcttttctgcactgtggtggagctgaagtacacaggaaatgccagtgccatgttcatcctccctgaccagggcaagatgcagcaggtggaagccagcttgcaaccagagaccctgaggaagtggaagaattctctgaaacccaggatgatagatgagctccacctgcccaagttctccatctccaccgactacagcctggaggatgtcctttcaaagctgggcatcagggaagtcttctccacacaggctgacctgtctgcaatcacaggaaccaaggatctgagagtctctcaggtggtccacaaggctgtgctggacgtggctgagacaggcacagaagcagctgctgccactggagtcaaatttgtcccaatgtctgcgaaactgtaccctctgactgtatatttcaatcggcctttcctgataatgatctttgacacagaaactgaaattgccccctttatagccaagatagccaaccccaaatgagactagaactccccaagtgttgacgcttcttcccgggagccaggcattgagcctgtctgtgggtctccatgtgcattttggcttccatgctctgcttggccttggcatgcctggattagatagtgactaactgtgttataacctcatgcacagacatccctgtgggaagtcagtgccatgctcccagacttcttggtagcactagcccatgttcctgagcctgaaatttgtcttgtcccctacccctgctctctccctgtatctgcctccacccaaaagcctgggccccatcaagtaagctcagtcccagtttagactctggttatgtctcccttcagccttgctgtcttgatgggactgtgcaaccttacaggccaacccatatggaccaagaggaaagcttgctgccccgtgtctatctgcagcatctaggactacttggtgcccagtctgcctcactctttcacttctccaggctttgcctccagcactgcccccctgcaggatctcctcactttgtccacatctggcacagagttagagccctcacttctgcagctgcatggggcctgtgggtcagagcagctcctttcccctggcactcctacttagaacaaagtagcctttcttttagttcccagctgaccaacctcacacaaaagaggaacaccaccaaccagaataaagaggtaggagcaaaagatcaataaacatataactgca

SEQ ID NO: 59 - DNA, 1576 bp, Homo sapiens
actactccagacagacggctttggaatccaccagctacatccagctccctgaggcagagttgagaatggagagaatgttacctctcctggctctggggctcttggcggctgggttctgccctgctgtcctctgccaccctaacagcccacttgacgaggagaatctgacccaggagaaccaagaccgagggacacacgtggacctcggattagcctccgccaacgtggacttcgctttcagcctgtacaagcagttagtcctgaaggcccctgataagaatgtcatcttctccccactgagcatctccaccgccttggccttcctgtctctgggggcccataataccaccctgacagagattctcaaaggcctcaagttcaacctcacggagacttctgaggcagaaattcaccagagcttccagcacctcctgcgcaccctcaatcagtccagcgatgagctgcagctgagtatgggaaatgccatgtttgtcaaagagcaactcagtctgctggacaggttcacggaggatgccaagaggctgtatggctccgaggcctttgccactgactttcaggactcagctgcagctaagaagctcatcaacgactacgtgaagaatggaactagggggaaaatcacagatctgatcaaggaccttgactcgcagacaatgatggtcctggtgaattacatcttctttaaagccaaatgggagatgccctttgacccccaagatactcatcagtcaaggttctacttgagcaagaaaaagtgggtaatggtgcccatgatgagtttgcatcacctgactataccttacttccgggacgaggagctgtcctgcaccgtggtggagctgaagtacacaggcaatgccagcgcactcttcatcctccctgatcaagacaagatggaggaagtggaagccatgctgctcccagagaccctgaagcggtggagagactctctggagttcagagagataggtgagctctacctgccaaagttttccatctcgagggactataacctgaacgacatacttctccagctgggcattgaggaagccttcaccagcaaggctgacctgtcagggatcacaggggccaggaacctagcagtctcccaggtggtccataaggctgtgcttgatgtatttgaggagggcacagaagcatctgctgccacagcagtcaaaatcaccctcctttctgcattagtggagacaaggaccattgtgcgtttcaacaggcccttcctgatgatcattgtccctacagacacccagaacatcttcttcatgagcaaagtcaccaatcccaagcaagcctagagcttgccatcaagcagtggggctctcagtaaggaacttggaatgcaagctggatgcctgggtctctgggcacagcctggcccctgtgcaccgagtggccatggcatgtgtggccctgtctgcttatccttggaaggtgacagcgattccctgtgtagctctcacatgcacaggggcccatggactcttcagtctggagggtcctgggcctcctgacagcaataaataatttcgttgga

SEQ ID NO: 60 - DNA, 485 bp, Mus musculus
aaattatttcatgagttcagccgagccagagccaacatgaagacagccacagtcttgtttctggtggctttgatcactgtggggatgaacactacctatgtagtgtcttgccccaaagaatttgaaaaacctggagcttgtcccaagccttcaccagaaagtgttggaatttgtgttgatcaatgctcaggagatggatcctgccctggcaacatgaagtgctgtagcaatagctgtggtcatgtctgcaaaactcctgtcttttaaatggttgacagccatgtggaagatggattcaatcttcataaacatgaatgatggccagccccagaagatttcttctgaattcacagagcctgtgcttggctacttcctagccctagaattgcattcttggacaaggaagatctatattgtggtgacaatgccctaatatgtctgtgtccaaaataaactacccttagcattcaaaaaaaaaaaaaaaa

SEQ ID NO: 61 - DNA, 6265 bp, Homo sapiens
agtcgcggcgtctgcctggtcctcagcagtgcagccccggcgcggagcagggagcctcggcccgcgcccggcgccctcgccctcgccctcgacccgcagccatggtgcccggggtgcccggcgcggtcctgaccctctgcctctggctggcggcctccagcggctgcctggcggccggccccggcgcggctgctgcgcggcggctggacgagtcgctgtctgccgggagcgtccagcgcgctcgctgcgcctccaggtgcctgagcctgcagatcactcgcatctccgccttcttccagcacttccagaacaatggttccctggtttggtgccagaatcacaagcaatgttctaagtgcctggagccctgcaaggaatcaggggacctgaggaaacaccagtgccaaagcttttgtgagcctctcttccccaagaagagctacgaatgcttgaccagctgtgagttcctcaaatacatcctgttggtgaagcagggggactgtccggctcctgagaaagccagtggatttgcggccgcctgtgttgaaagctgcgaagttgacaatgagtgctctggggtgaagaaatgttgttcgaatgggtgtggacacacctgtcaagtacccaagactctgtacaaaggtgtccccctgaagcccagaaaagagttacgatttacagaactgcagtctggacagctggaggttaagtggtcctcgaaattcaatatttctattgagcctgtgatctatgtggtacaaagaagatggaattatggaatccatcctagcgaagatgacgccactcactggcagacagtggcccagaccacagacgagcgagttcaactgactgacataagacccagccgatggtaccagtttcgagtggctgctgtgaatgtgcatggaactcgaggcttcactgcccccagcaaacacttccgttcttccaaagatccatctgccccaccagcaccggctaacctccggctggccaactccaccgtcaacagtgatgggagtgtgaccgtcactatagtttgggatctccccgaggagccggacatccctgtgcatcattacaaggtcttttggagctggatggtcagcagtaagtctcttgtcccaacaaagaagaagcggagaaagactacggatgggtttcaaaattctgtgatcctggagaaactccagccagactgtgactatgttgtggaattgcaagccataacgtactggggacagacacggctgaagagtgcaaaggtgtcccttcacttcacatcgacacatgcaaccaacaacaaagaacagcttgtgaaaactagaaaaggtggaattcaaacacaactcccttttcaaagacgacgacccactcgcccgctggaagtcggagctcccttctatcaggatggccaactgcaagttaaagtctactggaagaagacagaagatcccactgtcaaccgatatcatgtgcggtggtttcctgaagcgtgtgcccacaacagaacaaccggatcagaggcatcatctggcatgacccacgaaaattacataattcttcaagatctgtcattttcctgcaagtataaggtgactgtccaaccaatacggccaaaaagtcactccaaggcagaagctgttttcttcactactccaccatgctctgctcttaaggggaagagccacaagcctgttggctgcctgggcgaagcaggtcatgttctttctaaggtgctagctaagcctgagaacctttctgcttcattcatcgtccaggatgtgaacatcaccggtcacttttcttggaagatggccaaggccaatctctatcagcccatgactgggtttcaagtgacttgggctgaggtcactacggaaagcagacagaacagcctacccaacagcattatttcacagtcccagatcctgccttccgatcattatgtcctaacagtgcccaatctgagaccatctactctttaccgactggaagtgcaagtgctgaccccaggaggggaggggccggccaccatcaagacgttccggacgccggagctcccaccctcttcagcacacagatctcatcttaagcatcgtcatccacatcattacaagccttctccagaaagatactaaactgttcaaaaagattttgtgaaattgcacagatgtgtaagcttgttgaacttcggccacgagacatgcacacttccagaggcagtgggaactgctcagaggcccggactctcctatgtgactttagtgcaggaagaacttctgtcaatcatggacgcatctggagacaagtgagaaacagtagattggtgaagacagacaccagttccctacaagcatggagaaaatgaagaataggcctgtttaatgctaaattttgttttcatgtatggtgtcgctcatttctattgaattacaacagaactcagttttccctgaatttggagcaccaaactccgccccaaaaaggagagtaacaaatacacaattcacacataacactaagcgtaaatctaatcaataaaatatatttttgactaaattattgattcgatatgaaaaatcaactaagattacacagctttgtttttttgaatctttcctaagatcatttttatcctaggtgatttttaaatgaaaatgtgtaatctaaaatataccagcgaatttaaatctaaaaatgctcctactttaagtaccttgtgctgctctttatgcaaaggtaaatcaaagttccctctataaattatgatttacaaaagacacccaagccagaggaactcaatgaaataagctgctaatcagattttaccttggagaaatgaaaattatttcttggggatgccttttaatatttgatcctattatgtgagagattttcctgatatgttatcttatttatattttcccttattttcctcaatgcagataatagcttttggtgcacttttgtttcaccatctgaaaattcacaaaacttcttgcttcaaatgaaaaaatcccaactattgagcatgtttaaatctttgcagagatttgccttttcttaatcaaagaaaggtctttgtgtgctagaatattattggtaatgttttaaaaattcctttgattgatagagaaggacagttatttgcatttaattcacccatatgctttcaaatctagtatatcttactttttggaaatgttttatgctacaaattagtgccttgtagcatgaacttaagtcaaaacgtgttatcaatatagagtgttgcagtgtatattgtaacaacctaaaacgcagagaagtttaatttaatactgttttttttcttgaaggaatactcacatacatggtttgaaatgtgcatagatatgcatgtctatataattataaatgcatgtgtatatatatgcaaatatatgtacatatacatgtatatacacacagacacatgcatatacatgaatataccttgagcatgaatccctggagaaatcgttttcgtagctcaccaatggtgagtaaagatacagctcttttaaaggtcataaggataatatattttccccatcaatgctgattctgagaaaagagcaatttatcaaaattaaacactgtaaaagaaaggtgtccatatgtctttacctacctaagtaaaacaggaagaaaatcagtaacattatccttaggttttgacaatggtacttgcttcttgttgttttattgtttcctgaattcatgcagatgcctggccattcctgggaagagtggataactcagaagtcactgtactccacagagcctcactgcagtgtctaaaggtagatgcaaattaaaatgcagggaaaataacttttctgatgttgatgcatgtctttgggaaacacatttataaacatggatacctgataatagatattgaaacccatttcctgtgtgttaaaatatttaaaaagtggatattccaggaatgttttgcagctttgtacaagtaacataaattggacacctcagaatgaaagttcatgttggttctgaatggttcactgcagctcctgtcacaagctgggatggatttatcacattgagttatgaaattacctggttctaagaatttttgagtggcaaaaatagaaaacaatcttcatttgaaaacatccctaagcttgaataaatggataccatagatagcttctcttttttattctggtgtcattaccagcatctgaatttcaagttcttaaaatttcaaaaattaaaatttttcattattagctatccatttatcttttacatgaacttgtcatgaacaaattcaaatgtttatgccagcaaatttttgtactgttgcatagttaaaaatgctgggagtctctgcatagatacaaaatattattaaattattacataaatttaattttataaaatttaatcatgcttcttttgtctgggtaatagacattggacagatatttttagttcagatggtgattctgaagcttacatctcccttaaaaaaatctaaagcagctcttatgggcttctaattttaatataaataaataatttaaattttattggtgttattggaagaaaaatgctattaatgggctaataaaaaacatgtgtttctcttatggattttaataagctccagtattattcaaatgatcaaaaatatagttataattttttgaattttaaaaatgtgattgctctaataaagaataaaatctatgctttttaacaaacatagttttggtgcctaattctgtaatatgttttattgaaattagattcatttctctaatgtgagaaaaatatatccagtaatagtattgactgtttaaaaaattgagctcatcaaaaatattgtcatcaaatacaggtggttaatctgacatacattgcagttacatgcattatttttatttacaacatttgctccttaatgatgaatttatctgtgttaccctgtttttctacctggaactccatagaatgatgtttgcaaaccaacatgtgctcttttcagtcattcactgttttaatatgacatggtagagaagataaggtttatggcaggtaattttttgtaatgtgtattaaacgaagttcaaagattagaaatacatctgtgtcctgaaaaccttagatacatagccgactgtatacagaggttcatctcaacctcaacactattgacttttggggctggatagttctctgttgtgggggtttgtcttgtgcactgtaggtttttagtagcatccacactttctcctcaccagatgccagttgcaccctcccccaagttgagacaaccaaaaatgtctccagatattgccagctaccccttgagggatggtacctctggttgagaaccattgctagagaatgatctttactgaatttgccctttataagaaacccagtgaatttctagagcaagtcccaaaaactaagggacagctaagaagttattatggttgacttcaaaggcctaaactgtgttttttatgtccactaaacaacttgattaaaagacggaattttgactcgtgtctgtatcatacaagtacaaatactaattttgccctatgtatccgtaaatgtcatttgtgattttgacttatttatttaatgccctttcttatgccgtgggttttcaagtttactcatttctatggttgcaaataactctaaaacttattatataaactttcatattataggcagaacacaatggctaaatatctgttgcatgtactttaaagtttattataaaatataaacagatatataaagatgttgactcttacctgtgattttgcatggtcagactcggtgtcaggtacggagaggattctcatgactgtcttacctctactgaatattctagtgagttatatgatttacggagtgattaacagaggtctatataaagttacttttcccctttacttaattatattgtagtgtgcagataacaaaactgctaccttctcatccaagtggtctgtagaattcatgtcccttacagtggtcatttaaagtcaatatttatttatgtatgtaataaaaaaagttggatttttgtgtatgtctgtcacattatttagagagaagtaatcttgtaaaaatgttttgtaaaaaacaaaaaagtattgtaaatagtcttgatattctgtgactcattattttcatgttagagtttgtacatactggttcaataataaagtatccttaaaccaga

SEQ ID NO: 62 - DNA, 1346 bp, Mus musculus
ctctccttgggacacggaggtcttcagcacccacagagggacttacaggtcggatcataaggcagccttctgtcagtctgctctgccccttccctcgaggagcgccctgccttgctgactttctctgcctctggcttcctgtgataggtggtgtcattcccctccaacctgagtgctggcaggtacactgctggccaccagcagatgcccatgaagatgctgacaatgaagatgctggccctgtgcttggttcttgctaaatcagcctggtcggaggaacaggagaaggtggttcatggaggcccgtgtttgaaggactcccaccctttccaggctgccctctacacctcaggtcacttgctgtgtggtggggtcctcattgacccacagtgggtgctgacagctgcccactgcaaaaaaccgaatctgcaggtgatcttggggaaacacaacctacggcaaacagagactttccaaaggcaaatctcagtggacaggactattgtccatccccgctacaaccctgaaacccacgacaatgacatcatgatggtgcatctgaaaaatccagtcaaattctctaaaaagatccagcctctgcccttgaagaatgactgctctgaggagaatcccaactgccagatcctgggctggggcaagatggaaaatggtgacttcccagataccattcagtgtgctgatgtccatctggtgccccgggagcagtgtgagcgtgcctaccctggcaagatcacccagagcatggtgtgcgcaggcgacatgaaagaaggcaacgattcctgtcagggtgattctggaggtcccctagtatgtgggggtcgcctccgagggctcgtgtcatggggtgacatgccctgtggatcaaaggagaagccaggagtttacaccgatgtctgcactcatatcagatggatccaaaacatcctcagaaacaagtggctgtgacatgagacatccagttctcccccacgacgcctctgaccctcgctggctccatactctctctccctgaagccctgccctgctctcagagccttcagatgtccagctctgaccctggtacttaataaatgtagtgacacagagcacagaacactgctaaatctactttgctcaatcgttgcatccccagggagactggaggatacaggctacaatcctactctatgggtgtggttagcagatggaatcgcagtgtgcccactaacagtctgggtacccttgggaagtgcttttctttagagtgtgaatgctctcatctgtaaaattgggatactaacggagctggagaaatgctcagtggctaacagcacttatagcaagaa

SEQ ID NO: 63 - DNA, 1503 bp, Homo sapiens
acagaaccagcctcttccagggaggcctgggagctgggggtgtgtgtctggcagtccctgcagccctgggctctgcggcccctgcgtcctccgcttggctctgccactgcatctgagtgtcttctctcctcacggctccccgcatttctaactctttctgcctcctcgtctcaaagctgttccttcccccgactcaagaatccccggagcccggaggcctgcagcaggagcggccatgaagaagctgatggtggtgctgagtctgattgctgcagcctgggcagaggagcagaataagttggtgcatggcggaccctgcgacaagacatctcacccctaccaagctgccctctacacctcgggccacttgctctgtggtggggtccttatccatccactgtgggtcctcacagctgcccactgcaaaaaaccgaatcttcaggtcttcctggggaagcataaccttcggcaaagggagagttcccaggagcagagttctgttgtccgggctgtgatccaccctgactatgatgccgccagccatgaccaggacatcatgctgttgcgcctggcacgcccagccaaactctctgaactcatccagccccttcccctggagagggactgctcagccaacaccaccagctgccacatcctgggctggggcaagacagcagatggtgatttccctgacaccatccagtgtgcatacatccacctggtgtcccgtgaggagtgtgagcatgcctaccctggccagatcacccagaacatgttgtgtgctggggatgagaagtacgggaaggattcctgccagggtgattctgggggtccgctggtatgtggagaccacctccgaggccttgtgtcatggggtaacatcccctgtggatcaaaggagaagccaggagtctacaccaacgtctgcagatacacgaactggatccaaaaaaccattcaggccaagtgaccctgacatgtgacatctacctcccgacctaccaccccactggctggttccagaacgtctctcacctagaccttgcctcccctcctctcctgcccagctctgaccctgatgcttaataaacgcagcgacgtgagggtcctgattctccctggttttaccccagctccatccttgcatcactggggaggacgtgatgagtgaggacttgggtcctcggtcttacccccaccactaagagaatacaggaaaatcccttctaggcatctcctctccccaacccttccacacgtttgatttcttcctgcagaggcccagccacgtgtctggaatcccagctccgctgcttactgtcggtgtccccttgggatgtacctttcttcactgcagatttctcacctgtaagatgaagataaggatgatacagtctccataaggcagtggctgttggaaagatttaaggtttcacacctatgacatacatggaatagcacctgggccaccatgcactcaataaagaatgaattttattatga

SEQ ID NO: 64 - DNA, 1455 bp, Homo sapiens
acagaaccagcctcttccagggaggcctgggagctgggggtgtgtgtctggcagtccctgcagccctgggctctgcggcccctgcgtcctccgcttggctctgccactgcatctgagtgtcttctctcctcacggctccccgcatttctaactctttctgcctcctcgtctcaaagctgttccttcccccgactcaagaatccccggagcccggaggcctgcagcagcctgggcagaggagcagaataagttggtgcatggcggaccctgcgacaagacatctcacccctaccaagctgccctctacacctcgggccacttgctctgtggtggggtccttatccatccactgtgggtcctcacagctgcccactgcaaaaaaccgaatcttcaggtcttcctggggaagcataaccttcggcaaagggagagttcccaggagcagagttctgttgtccgggctgtgatccaccctgactatgatgccgccagccatgaccaggacatcatgctgttgcgcctggcacgcccagccaaactctctgaactcatccagccccttcccctggagagggactgctcagccaacaccaccagctgccacatcctgggctggggcaagacagcagatggtgatttccctgacaccatccagtgtgcatacatccacctggtgtcccgtgaggagtgtgagcatgcctaccctggccagatcacccagaacatgttgtgtgctggggatgagaagtacgggaaggattcctgccagggtgattctgggggtccgctggtatgtggagaccacctccgaggccttgtgtcatggggtaacatcccctgtggatcaaaggagaagccaggagtctacaccaacgtctgcagatacacgaactggatccaaaaaaccattcaggccaagtgaccctgacatgtgacatctacctcccgacctaccaccccactggctggttccagaacgtctctcacctagaccttgcctcccctcctctcctgcccagctctgaccctgatgcttaataaacgcagcgacgtgagggtcctgattctccctggttttaccccagctccatccttgcatcactggggaggacgtgatgagtgaggacttgggtcctcggtcttacccccaccactaagagaatacaggaaaatcccttctaggcatctcctctccccaacccttccacacgtttgatttcttcctgcagaggcccagccacgtgtctggaatcccagctccgctgcttactgtcggtgtccccttgggatgtacctttcttcactgcagatttctcacctgtaagatgaagataaggatgatacagtctccataaggcagtggctgttggaaagatttaaggtttcacacctatgacatacatggaatagcacctgggccaccatgcactcaataaagaatgaattttattatga

SEQ ID NO: 65 - DNA, 1272 bp, Homo sapiens
agtgtggtgacacacgctgtagctgtctccccggctggctggctcgctctctcctggggacacagaggtcggcaggcagcacacagagggacctacgggcagctgttccttcccccgactcaagaatccccggagcccggaggcctgcagcaggagcggccatgaagaagctgatggtggtgctgagtctgattgctgcaggaatcttcaggtcttcctggggaagcataaccttcggcaaagggagagttcccaggagcagagttctgttgtccgggctgtgatccaccctgactatgatgccgccagccatgaccaggacatcatgctgttgcgcctggcacgcccagccaaactctctgaactcatccagccccttcccctggagagggactgctcagccaacaccaccagctgccacatcctgggctggggcaagacagcagatggtgatttccctgacaccatccagtgtgcatacatccacctggtgtcccgtgaggagtgtgagcatgcctaccctggccagatcacccagaacatgttgtgtgctggggatgagaagtacgggaaggattcctgccagggtgattctgggggtccgctggtatgtggagaccacctccgaggccttgtgtcatggggtaacatcccctgtggatcaaaggagaagccaggagtctacaccaacgtctgcagatacacgaactggatccaaaaaaccattcaggccaagtgaccctgacatgtgacatctacctcccgacctaccaccccactggctggttccagaacgtctctcacctagaccttgcctcccctcctctcctgcccagctctgaccctgatgcttaataaacgcagcgacgtgagggtcctgattctccctggttttaccccagctccatccttgcatcactggggaggacgtgatgagtgaggacttgggtcctcggtcttacccccaccactaagagaatacaggaaaatcccttctaggcatctcctctccccaacccttccacacgtttgatttcttcctgcagaggcccagccacgtgtctggaatcccagctccgctgcttactgtcggtgtccccttgggatgtacctttcttcactgcagatttctcacctgtaagatgaagataaggatgatacagtctccataaggcagtggctgttggaaagatttaaggtttcacacctatgacatacatggaatagcacctgggccaccatgcactcaataaagaatgaattttattatga

SEQ ID NO: 66 - DNA, 1346 bp, Homo sapiens
acagaaccagcctcttccagggaggcctgggagctgggggtgtgtgtctggcagtccctgcagccctgggctctgcggcccctgcgtcctccgcttggctctgccactgcatctgagtgtcttctctcctcacggctccccgcatttctaactctttctgcctcctcgtctcaaagctgttccttcccccgactcaagaatccccggagcccggaggcctgcagcaggagcggccatgaagaagctgatggtggtgctgagtctgattgctgcaggaatcttcaggtcttcctggggaagcataaccttcggcaaagggagagttcccaggagcagagttctgttgtccgggctgtgatccaccctgactatgatgccgccagccatgaccaggacatcatgctgttgcgcctggcacgcccagccaaactctctgaactcatccagccccttcccctggagagggactgctcagccaacaccaccagctgccacatcctgggctggggcaagacagcagatggtgatttccctgacaccatccagtgtgcatacatccacctggtgtcccgtgaggagtgtgagcatgcctaccctggccagatcacccagaacatgttgtgtgctggggatgagaagtacgggaaggattcctgccagggtgattctgggggtccgctggtatgtggagaccacctccgaggccttgtgtcatggggtaacatcccctgtggatcaaaggagaagccaggagtctacaccaacgtctgcagatacacgaactggatccaaaaaaccattcaggccaagtgaccctgacatgtgacatctacctcccgacctaccaccccactggctggttccagaacgtctctcacctagaccttgcctcccctcctctcctgcccagctctgaccctgatgcttaataaacgcagcgacgtgagggtcctgattctccctggttttaccccagctccatccttgcatcactggggaggacgtgatgagtgaggacttgggtcctcggtcttacccccaccactaagagaatacaggaaaatcccttctaggcatctcctctccccaacccttccacacgtttgatttcttcctgcagaggcccagccacgtgtctggaatcccagctccgctgcttactgtcggtgtccccttgggatgtacctttcttcactgcagatttctcacctgtaagatgaagataaggatgatacagtctccataaggcagtggctgttggaaagatttaaggtttcacacctatgacatacatggaatagcacctgggccaccatgcactcaataaagaatgaattttattatga

SEQ ID NO: 67 - DNA, 1429 bp, Homo sapiens
agtgtggtgacacacgctgtagctgtctccccggctggctggctcgctctctcctggggacacagaggtcggcaggcagcacacagagggacctacgggcagctgttccttcccccgactcaagaatccccggagcccggaggcctgcagcaggagcggccatgaagaagctgatggtggtgctgagtctgattgctgcagcctgggcagaggagcagaataagttggtgcatggcggaccctgcgacaagacatctcacccctaccaagctgccctctacacctcgggccacttgctctgtggtggggtccttatccatccactgtgggtcctcacagctgcccactgcaaaaaaccgaatcttcaggtcttcctggggaagcataaccttcggcaaagggagagttcccaggagcagagttctgttgtccgggctgtgatccaccctgactatgatgccgccagccatgaccaggacatcatgctgttgcgcctggcacgcccagccaaactctctgaactcatccagccccttcccctggagagggactgctcagccaacaccaccagctgccacatcctgggctggggcaagacagcagatggtgatttccctgacaccatccagtgtgcatacatccacctggtgtcccgtgaggagtgtgagcatgcctaccctggccagatcacccagaacatgttgtgtgctggggatgagaagtacgggaaggattcctgccagggtgattctgggggtccgctggtatgtggagaccacctccgaggccttgtgtcatggggtaacatcccctgtggatcaaaggagaagccaggagtctacaccaacgtctgcagatacacgaactggatccaaaaaaccattcaggccaagtgaccctgacatgtgacatctacctcccgacctaccaccccactggctggttccagaacgtctctcacctagaccttgcctcccctcctctcctgcccagctctgaccctgatgcttaataaacgcagcgacgtgagggtcctgattctccctggttttaccccagctccatccttgcatcactggggaggacgtgatgagtgaggacttgggtcctcggtcttacccccaccactaagagaatacaggaaaatcccttctaggcatctcctctccccaacccttccacacgtttgatttcttcctgcagaggcccagccacgtgtctggaatcccagctccgctgcttactgtcggtgtccccttgggatgtacctttcttcactgcagatttctcacctgtaagatgaagataaggatgatacagtctccataaggcagtggctgttggaaagatttaaggtttcacacctatgacatacatggaatagcacctgggccaccatgcactcaataaagaatgaattttattatga

SEQ ID NO: 68 - DNA, 4687 bp, Mus musculus
gtgtgggtggaacccgctgtttgcataaagcctagctgctcctcagcacgttcaggaccagatctctggcggggagcagggtgcaaggcagccaggtctccagtcctctctgcagcatggggaagcgctggctcccaagcctggccctgctgccgctgccgccaccgctgctgctgctgctgttgctgctgctgcccacaaatgcctcagcaccacagaaaccaatctacatggtgatggttccctccctgctccacgctggcacccctgagaagggctgcctcctgttcaaccacctaaacgagacagtaacagtgaaagtatccatggagtctgtccgtgggaaccaaagcctcttcactgaccttgttgttgacaaggacttattccactgtgcctccttcatcgtcccacagtcttcatccaatgaggtgatgtttctcactgtccaagtaaaaggaccaactcatgagttcaggaggaggagcacggtgctgatcaagactaaagagagcctggtctttgctcagactgacaagcccatctacaaaccaggacagatggtgagatttcgtgttgtctcattggacgaaaatttccacccccttaatgaattgattcctctactgtacattcaggattcaaaaaaaaatcgcattgcacagtggcagaatttccgcttagagggtggcctcaaacagctgtccttccccctctcctcagagcccactcagggctcctacaaggtggtgatacgtacagaatcaggcaggaccgtcgagcaccccttctctgtgaaggaatttgtgcttcccaagtttgaagtcaaagttgcagtaccagagacaatcaccatcctggaggaagagatgaatgtgtccgtgtgtggcatatacacctatgggaagcctgttccaggacacgtgactgtgaacatttgcagaaagtacagtaatccttctagctgctttggtgaagaatcgctggctttctgtgagaaattcagtcaacagctagatggccgtggctgcttctcacagctagtgaaaaccaagtctttccagctaaagaggcaagagtatgagatgcagcttgatgtgaatgccaagatccaagaagaaggaacaggtgtggaagaaaccggtaaagggctcactaagatcacaagaactataacaaaactatcatttgtgaacgtggatacacatttcagacaaggaattcctttcgttgggcaggtgctcctggtggatgggagaggcacccctattccatatgaaatgatcttcattggagctgatgaagcaaaccagaacataaatactaccactgataagaatggcctggcacggttctccatcaacactgatgacatcatgggcacgtccctaactgtcagggccaaatacaaagatagcaatgtctgctatggatttagatggttgacagaagagaacgtagaggcttggcacactgccaacgctgtcttctcaccgagcagaagcttcgtgcacctggaatccctgccctataaactgcgctgtgagcaaaccctggcggtccaggctcattatattctaaatgacgaggctgtgctggagcggaaggagttggtcttctattatctgatgatggcaaagggaggcattgttcgggcagggactcacgttctgcctgtgacgcagggacacaagaaaggccatttctccatcctcatctcgatggagacagacctggctcctgtagctcgactggtcctttataccattctgcccaatggagaagtggttggagatactgttaaatatgagattgaaaagtgcctggccaacaaggtggatttggtcttccacccaaatatcggtcttccggccacacgtgccttcctcagtgtcatggcttctcctcagtctctctgtggcctgcgagctgtggaccaaagcgtactgctcacaaagcctgaggccgaactctctgcatccctggtttatgatctgctaccagtgaaagacctcactggcttccctaagggtgtgaatcaacaggaagaagacactaatggctgccttaagcaaaatgacacttacattaatggaatcctgtactccccagtacagaatacaaatgaagaggacatgtatggcttcctaaaggatatgggcttaaaggtattcaccaacttgaacatccgtaaacccaaagtctgtgaacgccttggagtcaataaaataccagctgcataccaccttgtaagccaaggccacatggatgcttttctagagtcttcagagtctcccacagagactacacgaagctacttccctgagacgtggatctgggacttggtgatcgtggactcaacaggagtggctgaaatggaagtgacagtccctgacaccatcactgaatggaaggctggggccttctgcctgtccaatgacactgggttgggcctctctcctgtgatcgatttccaagccttccagcccttcttcgtggatctcacaatgccctactccgtgatccgtggagaggccttcacgctcaaggccactgtgctgaactacctccagacatgcatccgggttggtgtacagctggaggcctctcctgatttcctagctaccccagaggagaaggaacaaaagtctcactgcatctgtatgaacgagcggcataccatgtcctgggcggtgatccccaagtcattaggaaatgtgaatttcacagtgagtgcagaggcactggactctaaggagctgtgtaggaatgaggtgccagtggttcctgaacgtggaaagaaagacacgatcatcaagtccctgctggttgaacctgaaggtctagagaatgaagtgacattcaacagtttgctttgtccaacaggtgctgaggtatcggaacagatatctctgaaactgccatcagatgtggtagaggaatctgcccgagcttctgtcacagttttgggagatatattgggttctgctatgcagaacacacaggatctccttaagatgccctatggctgtggagaacagaacatggttctgtttgctcctaatatctatgtcctggactatctgaatgaaacagagcagctgacacaggagatcaagaccaaggccattacctatctcaatacgggttaccaaagacaattaaactacaagcaccgggatggctcctacagtacttttggggataaacctggtaggagtcatgccaatacctggctcacagcctttgtactgaagagttttgctcaggctcgaagatatatcttcatcgatgaatcacacatcacccaagccctcacctggctctcccagcagcagaaggacaatggctgcttcaggagctccgggtcactgctcaacaatgccatgaagggaggagtagaagatgaagtcactttgtctgcctacatcaccattgctctcctggagatgtctcttcctgtcactcatcctgttgtccgaaatgccctcttttgcctggacacagcctggaagtcagcgaggagaggagccagcggcaaccatgtctacactaaggcactgttggcctatgcatttgcccttgctggtaaccaggacacgaagaaggagatactgaaatcactcgatgaggaggcggtaaaagaagacaattctgtccactggaccagagctcagaaacccagagtgccagcagatctctggtaccaaccccaggctccctcggctgaggtagagatgaccgcttatgtgctcctggcttatcttaccactgagctggttccaacccgagaggacctgactgctgcaatgctcattgtgaagtggctcacaaagcagcagaattcccacggtggcttctcctccacccaggacacggtagtggctctccatgctttgtccaaatacggagcagctactttcacaagagcgaagaaagctgcacatgtgaccatccagtcttctggcgcattttatacaaaattccaagtgaacaacgacaaccagttattattacagagagtcacattgccaactgtgcctggggattacaccgcaaaggtagctggagaagggtgtgtctacctccagacatccttgaaatatagtgttctcccgagggagaaggagtttccatttgctttggtggtgcagactctgcctgggacttgtgaggatctcaaagctcacaccaccttccagatctcactcaatatcagttacattggaagccgttctgactccaacatggcaattgctgatgtgaagatggtgtctggcttcatccccttgaaaccaacagtgaaaatgcttgaaagatctgtgcatgtgagccggacggaagtcagcaataaccatgtcttgatttacttggataaggtgtcaaatcagatgctgaccttgttcttcatggtgcagcaagatattccagtgagagacctgaagccagccatagtgaaagtctatgattactacgagaaagatgagtttgcagttgcaaaatacagtgctccctgcagtgcaggttatggaaatgcctgaagacactgtgaataagaagtgtttcaccagagccctgttcttaggacttctcaagaaaaagtggtttttgtatttccagagatttgataaataaagcattctttcatatctatccatcaccattccttcaaaaaaaaaaaaaaaaa

SEQ ID NO: 69 - DNA, 4610 bp, Homo sapiens
gggaccagatggattgtagggagtagggtacaatacagtctgttctcctccagctccttctttctgcaacatggggaagaacaaactccttcatccaagtctggttcttctcctcttggtcctcctgcccacagacgcctcagtctctggaaaaccgcagtatatggttctggtcccctccctgctccacactgagaccactgagaagggctgtgtccttctgagctacctgaatgagacagtgactgtaagtgcttccttggagtctgtcaggggaaacaggagcctcttcactgacctggaggcggagaatgacgtactccactgtgtcgccttcgctgtcccaaagtcttcatccaatgaggaggtaatgttcctcactgtccaagtgaaaggaccaacccaagaatttaagaagcggaccacagtgatggttaagaacgaggacagtctggtctttgtccagacagacaaatcaatctacaaaccagggcagacagtgaaatttcgtgttgtctccatggatgaaaactttcaccccctgaatgagttgattccactagtatacattcaggatcccaaaggaaatcgcatcgcacaatggcagagtttccagttagagggtggcctcaagcaattttcttttcccctctcatcagagcccttccagggctcctacaaggtggtggtacagaagaaatcaggtggaaggacagagcaccctttcaccgtggaggaatttgttcttcccaagtttgaagtacaagtaacagtgccaaagataatcaccatcttggaagaagagatgaatgtatcagtgtgtggcctatacacatatgggaagcctgtccctggacatgtgactgtgagcatttgcagaaagtatagtgacgcttccgactgccacggtgaagattcacaggctttctgtgagaaattcagtggacagctaaacagccatggctgcttctatcagcaagtaaaaaccaaggtcttccagctgaagaggaaggagtatgaaatgaaacttcacactgaggcccagatccaagaagaaggaacagtggtggaattgactggaaggcagtccagtgaaatcacaagaaccataaccaaactctcatttgtgaaagtggactcacactttcgacagggaattcccttctttgggcaggtgcgcctagtagatgggaaaggcgtccctataccaaataaagtcatattcatcagaggaaatgaagcaaactattactccaatgctaccacggatgagcatggccttgtacagttctctatcaacaccaccaatgttatgggtacctctcttactgttagggtcaattacaaggatcgtagtccctgttacggctaccagtgggtgtcagaagaacacgaagaggcacatcacactgcttatcttgtgttctccccaagcaagagctttgtccaccttgagcccatgtctcatgaactaccctgtggccatactcagacagtccaggcacattatattctgaatggaggcaccctgctggggctgaagaagctctccttctattatctgataatggcaaagggaggcattgtccgaactgggactcatggactgcttgtgaagcaggaagacatgaagggccatttttccatctcaatccctgtgaagtcagacattgctcctgtcgctcggttgctcatctatgctgttttacctaccggggacgtgattggggattctgcaaaatatgatgttgaaaattgtctggccaacaaggtggatttgagcttcagcccatcacaaagtctcccagcctcacacgcccacctgcgagtcacagcggctcctcagtccgtctgcgccctccgtgctgtggaccaaagcgtgctgctcatgaagcctgatgctgagctctcggcgtcctcggtttacaacctgctaccagaaaaggacctcactggcttccctgggcctttgaatgaccaggacaatgaagactgcatcaatcgtcataatgtctatattaatggaatcacatatactccagtatcaagtacaaatgaaaaggatatgtacagcttcctagaggacatgggcttaaaggcattcaccaactcaaagattcgtaaacccaaaatgtgtccacagcttcaacagtatgaaatgcatggacctgaaggtctacgtgtaggtttttatgagtcagatgtaatgggaagaggccatgcacgcctggtgcatgttgaagagcctcacacggagaccgtacgaaagtacttccctgagacatggatctgggatttggtggtggtaaactcagcaggtgtggctgaggtaggagtaacagtccctgacaccatcaccgagtggaaggcaggggccttctgcctgtctgaagatgctggacttggtatctcttccactgcctctctccgagccttccagcccttctttgtggagctcacaatgccttactctgtgattcgtggagaggccttcacactcaaggccacggtcctaaactaccttcccaaatgcatccgggtcagtgtgcagctggaagcctctcccgccttcctagctgtcccagtggagaaggaacaagcgcctcactgcatctgtgcaaacgggcggcaaactgtgtcctgggcagtaaccccaaagtcattaggaaatgtgaatttcactgtgagcgcagaggcactagagtctcaagagctgtgtgggactgaggtgccttcagttcctgaacacggaaggaaagacacagtcatcaagcctctgttggttgaacctgaaggactagagaaggaaacaacattcaactccctactttgtccatcaggtggtgaggtttctgaagaattatccctgaaactgccaccaaatgtggtagaagaatctgcccgagcttctgtctcagttttgggagacatattaggctctgccatgcaaaacacacaaaatcttctccagatgccctatggctgtggagagcagaatatggtcctctttgctcctaacatctatgtactggattatctaaatgaaacacagcagcttactccagagatcaagtccaaggccattggctatctcaacactggttaccagagacagttgaactacaaacactatgatggctcctacagcacctttggggagcgatatggcaggaaccagggcaacacctggctcacagcctttgttctgaagacttttgcccaagctcgagcctacatcttcatcgatgaagcacacattacccaagccctcatatggctctcccagaggcagaaggacaatggctgtttcaggagctctgggtcactgctcaacaatgccataaagggaggagtagaagatgaagtgaccctctccgcctatatcaccatcgcccttctggagattcctctcacagtcactcaccctgttgtccgcaatgccctgttttgcctggagtcagcctggaagacagcacaagaaggggaccatggcagccatgtatataccaaagcactgctggcctatgcttttgccctggcaggtaaccaggacaagaggaaggaagtactcaagtcacttaatgaggaagctgtgaagaaagacaactctgtccattgggagcgccctcagaaacccaaggcaccagtggggcatttttacgaaccccaggctccctctgctgaggtggagatgacatcctatgtgctcctcgcttatctcacggcccagccagccccaacctcggaggacctgacctctgcaaccaacatcgtgaagtggatcacgaagcagcagaatgcccagggcggtttctcctccacccaggacacagtggtggctctccatgctctgtccaaatatggagcagccacatttaccaggactgggaaggctgcacaggtgactatccagtcttcagggacattttccagcaaattccaagtggacaacaacaaccgcctgttactgcagcaggtctcattgccagagctgcctggggaatacagcatgaaagtgacaggagaaggatgtgtctacctccagacatccttgaaatacaatattctcccagaaaaggaagagttcccctttgctttaggagtgcagactctgcctcaaacttgtgatgaacccaaagcccacaccagcttccaaatctccctaagtgtcagttacacagggagccgctctgcctccaacatggcgatcgttgatgtgaagatggtctctggcttcattcccctgaagccaacagtgaaaatgcttgaaagatctaaccatgtgagccggacagaagtcagcagcaaccatgtcttgatttaccttgataaggtgtcaaatcagacactgagcttgttcttcacggttctgcaagatgtcccagtaagagatctgaaaccagccatagtgaaagtctatgattactacgagacggatgagtttgcaattgctgagtacaatgctccttgcagcaaagatcttggaaatgcttgaagaccacaaggctgaaaagtgctttgctggagtcctgttctcagagctccacagaagacacgtgtttttgtatctttaaagacttgatgaataaacactttttctggtcaatgtc

SEQ ID NO: 70 - DNA, 4659 bp, Homo sapiens
atacaagagatgtgagaagcaccataaaaggcgttgtgaggagttgtgggggagtgagggagagaagaggttgaaaagcttattagctgctgtacggtaaaactccttctttctgcaacatggggaagaacaaactccttcatccaagtctggttcttctcctcttggtcctcctgcccacagacgcctcagtctctggaaaaccgcagtatatggttctggtcccctccctgctccacactgagaccactgagaagggctgtgtccttctgagctacctgaatgagacagtgactgtaagtgcttccttggagtctgtcaggggaaacaggagcctcttcactgacctggaggcggagaatgacgtactccactgtgtcgccttcgctgtcccaaagtcttcatccaatgaggaggtaatgttcctcactgtccaagtgaaaggaccaacccaagaatttaagaagcggaccacagtgatggttaagaacgaggacagtctggtctttgtccagacagacaaatcaatctacaaaccagggcagacagtgaaatttcgtgttgtctccatggatgaaaactttcaccccctgaatgagttgattccactagtatacattcaggatcccaaaggaaatcgcatcgcacaatggcagagtttccagttagagggtggcctcaagcaattttcttttcccctctcatcagagcccttccagggctcctacaaggtggtggtacagaagaaatcaggtggaaggacagagcaccctttcaccgtggaggaatttgttcttcccaagtttgaagtacaagtaacagtgccaaagataatcaccatcttggaagaagagatgaatgtatcagtgtgtggcctatacacatatgggaagcctgtccctggacatgtgactgtgagcatttgcagaaagtatagtgacgcttccgactgccacggtgaagattcacaggctttctgtgagaaattcagtggacagctaaacagccatggctgcttctatcagcaagtaaaaaccaaggtcttccagctgaagaggaaggagtatgaaatgaaacttcacactgaggcccagatccaagaagaaggaacagtggtggaattgactggaaggcagtccagtgaaatcacaagaaccataaccaaactctcatttgtgaaagtggactcacactttcgacagggaattcccttctttgggcaggtgcgcctagtagatgggaaaggcgtccctataccaaataaagtcatattcatcagaggaaatgaagcaaactattactccaatgctaccacggatgagcatggccttgtacagttctctatcaacaccaccaatgttatgggtacctctcttactgttagggtcaattacaaggatcgtagtccctgttacggctaccagtgggtgtcagaagaacacgaagaggcacatcacactgcttatcttgtgttctccccaagcaagagctttgtccaccttgagcccatgtctcatgaactaccctgtggccatactcagacagtccaggcacattatattctgaatggaggcaccctgctggggctgaagaagctctccttctattatctgataatggcaaagggaggcattgtccgaactgggactcatggactgcttgtgaagcaggaagacatgaagggccatttttccatctcaatccctgtgaagtcagacattgctcctgtcgctcggttgctcatctatgctgttttacctaccggggacgtgattggggattctgcaaaatatgatgttgaaaattgtctggccaacaaggtggatttgagcttcagcccatcacaaagtctcccagcctcacacgcccacctgcgagtcacagcggctcctcagtccgtctgcgccctccgtgctgtggaccaaagcgtgctgctcatgaagcctgatgctgagctctcggcgtcctcggtttacaacctgctaccagaaaaggacctcactggcttccctgggcctttgaatgaccaggacaatgaagactgcatcaatcgtcataatgtctatattaatggaatcacatatactccagtatcaagtacaaatgaaaaggatatgtacagcttcctagaggacatgggcttaaaggcattcaccaactcaaagattcgtaaacccaaaatgtgtccacagcttcaacagtatgaaatgcatggacctgaaggtctacgtgtaggtttttatgagtcagatgtaatgggaagaggccatgcacgcctggtgcatgttgaagagcctcacacggagaccgtacgaaagtacttccctgagacatggatctgggatttggtggtggtaaactcagcaggtgtggctgaggtaggagtaacagtccctgacaccatcaccgagtggaaggcaggggccttctgcctgtctgaagatgctggacttggtatctcttccactgcctctctccgagccttccagcccttctttgtggagctcacaatgccttactctgtgattcgtggagaggccttcacactcaaggccacggtcctaaactaccttcccaaatgcatccgggtcagtgtgcagctggaagcctctcccgccttcctagctgtcccagtggagaaggaacaagcgcctcactgcatctgtgcaaacgggcggcaaactgtgtcctgggcagtaaccccaaagtcattaggaaatgtgaatttcactgtgagcgcagaggcactagagtctcaagagctgtgtgggactgaggtgccttcagttcctgaacacggaaggaaagacacagtcatcaagcctctgttggttgaacctgaaggactagagaaggaaacaacattcaactccctactttgtccatcaggtggtgaggtttctgaagaattatccctgaaactgccaccaaatgtggtagaagaatctgcccgagcttctgtctcagttttgggagacatattaggctctgccatgcaaaacacacaaaatcttctccagatgccctatggctgtggagagcagaatatggtcctctttgctcctaacatctatgtactggattatctaaatgaaacacagcagcttactccagagatcaagtccaaggccattggctatctcaacactggttaccagagacagttgaactacaaacactatgatggctcctacagcacctttggggagcgatatggcaggaaccagggcaacacctggctcacagcctttgttctgaagacttttgcccaagctcgagcctacatcttcatcgatgaagcacacattacccaagccctcatatggctctcccagaggcagaaggacaatggctgtttcaggagctctgggtcactgctcaacaatgccataaagggaggagtagaagatgaagtgaccctctccgcctatatcaccatcgcccttctggagattcctctcacagtcactcaccctgttgtccgcaatgccctgttttgcctggagtcagcctggaagacagcacaagaaggggaccatggcagccatgtatataccaaagcactgctggcctatgcttttgccctggcaggtaaccaggacaagaggaaggaagtactcaagtcacttaatgaggaagctgtgaagaaagacaactctgtccattgggagcgccctcagaaacccaaggcaccagtggggcatttttacgaaccccaggctccctctgctgaggtggagatgacatcctatgtgctcctcgcttatctcacggcccagccagccccaacctcggaggacctgacctctgcaaccaacatcgtgaagtggatcacgaagcagcagaatgcccagggcggtttctcctccacccaggacacagtggtggctctccatgctctgtccaaatatggagcagccacatttaccaggactgggaaggctgcacaggtgactatccagtcttcagggacattttccagcaaattccaagtggacaacaacaaccgcctgttactgcagcaggtctcattgccagagctgcctggggaatacagcatgaaagtgacaggagaaggatgtgtctacctccagacatccttgaaatacaatattctcccagaaaaggaagagttcccctttgctttaggagtgcagactctgcctcaaacttgtgatgaacccaaagcccacaccagcttccaaatctccctaagtgtcagttacacagggagccgctctgcctccaacatggcgatcgttgatgtgaagatggtctctggcttcattcccctgaagccaacagtgaaaatgcttgaaagatctaaccatgtgagccggacagaagtcagcagcaaccatgtcttgatttaccttgataaggtgtcaaatcagacactgagcttgttcttcacggttctgcaagatgtcccagtaagagatctgaaaccagccatagtgaaagtctatgattactacgagacggatgagtttgcaattgctgagtacaatgctccttgcagcaaagatcttggaaatgcttgaagaccacaaggctgaaaagtgctttgctggagtcctgttctcagagctccacagaagacacgtgtttttgtatctttaaagacttgatgaataaacactttttctggtcaatgtc

SEQ ID NO: 71 - DNA, 4763 bp, Homo sapiens
gggaccagatggattgtagggagtagggtacaatacagtctgttctcctccagctccttctttctgcaacatggggaagaacaaactccttcatccaagtctggttcttctcctcttggtcctcctgcccacagacgcctcagtctctggaaaaccgcagtatatggttctggtcccctccctgctccacactgagaccactgagaagggctgtgtccttctgagctacctgaatgagacagtgactgtaagtgcttccttggagtctgtcaggggaaacaggagcctcttcactgacctggaggcggagaatgacgtactccactgtgtcgccttcgctaagtgattcctgtccatgccaactttccctgctgagaacaagggagtgaagttaagtaagaagggcaagatctccagggaagagtgcaacagcaaataggggaggagacctgcgggtgctgaatggggtttcaggatcggtcctgtatttcaggtcccaaagtcttcatccaatgaggaggtaatgttcctcactgtccaagtgaaaggaccaacccaagaatttaagaagcggaccacagtgatggttaagaacgaggacagtctggtctttgtccagacagacaaatcaatctacaaaccagggcagacagtgaaatttcgtgttgtctccatggatgaaaactttcaccccctgaatgagttgattccactagtatacattcaggatcccaaaggaaatcgcatcgcacaatggcagagtttccagttagagggtggcctcaagcaattttcttttcccctctcatcagagcccttccagggctcctacaaggtggtggtacagaagaaatcaggtggaaggacagagcaccctttcaccgtggaggaatttgttcttcccaagtttgaagtacaagtaacagtgccaaagataatcaccatcttggaagaagagatgaatgtatcagtgtgtggcctatacacatatgggaagcctgtccctggacatgtgactgtgagcatttgcagaaagtatagtgacgcttccgactgccacggtgaagattcacaggctttctgtgagaaattcagtggacagctaaacagccatggctgcttctatcagcaagtaaaaaccaaggtcttccagctgaagaggaaggagtatgaaatgaaacttcacactgaggcccagatccaagaagaaggaacagtggtggaattgactggaaggcagtccagtgaaatcacaagaaccataaccaaactctcatttgtgaaagtggactcacactttcgacagggaattcccttctttgggcaggtgcgcctagtagatgggaaaggcgtccctataccaaataaagtcatattcatcagaggaaatgaagcaaactattactccaatgctaccacggatgagcatggccttgtacagttctctatcaacaccaccaatgttatgggtacctctcttactgttagggtcaattacaaggatcgtagtccctgttacggctaccagtgggtgtcagaagaacacgaagaggcacatcacactgcttatcttgtgttctccccaagcaagagctttgtccaccttgagcccatgtctcatgaactaccctgtggccatactcagacagtccaggcacattatattctgaatggaggcaccctgctggggctgaagaagctctccttctattatctgataatggcaaagggaggcattgtccgaactgggactcatggactgcttgtgaagcaggaagacatgaagggccatttttccatctcaatccctgtgaagtcagacattgctcctgtcgctcggttgctcatctatgctgttttacctaccggggacgtgattggggattctgcaaaatatgatgttgaaaattgtctggccaacaaggtggatttgagcttcagcccatcacaaagtctcccagcctcacacgcccacctgcgagtcacagcggctcctcagtccgtctgcgccctccgtgctgtggaccaaagcgtgctgctcatgaagcctgatgctgagctctcggcgtcctcggtttacaacctgctaccagaaaaggacctcactggcttccctgggcctttgaatgaccaggacaatgaagactgcatcaatcgtcataatgtctatattaatggaatcacatatactccagtatcaagtacaaatgaaaaggatatgtacagcttcctagaggacatgggcttaaaggcattcaccaactcaaagattcgtaaacccaaaatgtgtccacagcttcaacagtatgaaatgcatggacctgaaggtctacgtgtaggtttttatgagtcagatgtaatgggaagaggccatgcacgcctggtgcatgttgaagagcctcacacggagaccgtacgaaagtacttccctgagacatggatctgggatttggtggtggtaaactcagcaggtgtggctgaggtaggagtaacagtccctgacaccatcaccgagtggaaggcaggggccttctgcctgtctgaagatgctggacttggtatctcttccactgcctctctccgagccttccagcccttctttgtggagctcacaatgccttactctgtgattcgtggagaggccttcacactcaaggccacggtcctaaactaccttcccaaatgcatccgggtcagtgtgcagctggaagcctctcccgccttcctagctgtcccagtggagaaggaacaagcgcctcactgcatctgtgcaaacgggcggcaaactgtgtcctgggcagtaaccccaaagtcattaggaaatgtgaatttcactgtgagcgcagaggcactagagtctcaagagctgtgtgggactgaggtgccttcagttcctgaacacggaaggaaagacacagtcatcaagcctctgttggttgaacctgaaggactagagaaggaaacaacattcaactccctactttgtccatcaggtggtgaggtttctgaagaattatccctgaaactgccaccaaatgtggtagaagaatctgcccgagcttctgtctcagttttgggagacatattaggctctgccatgcaaaacacacaaaatcttctccagatgccctatggctgtggagagcagaatatggtcctctttgctcctaacatctatgtactggattatctaaatgaaacacagcagcttactccagagatcaagtccaaggccattggctatctcaacactggttaccagagacagttgaactacaaacactatgatggctcctacagcacctttggggagcgatatggcaggaaccagggcaacacctggctcacagcctttgttctgaagacttttgcccaagctcgagcctacatcttcatcgatgaagcacacattacccaagccctcatatggctctcccagaggcagaaggacaatggctgtttcaggagctctgggtcactgctcaacaatgccataaagggaggagtagaagatgaagtgaccctctccgcctatatcaccatcgcccttctggagattcctctcacagtcactcaccctgttgtccgcaatgccctgttttgcctggagtcagcctggaagacagcacaagaaggggaccatggcagccatgtatataccaaagcactgctggcctatgcttttgccctggcaggtaaccaggacaagaggaaggaagtactcaagtcacttaatgaggaagctgtgaagaaagacaactctgtccattgggagcgccctcagaaacccaaggcaccagtggggcatttttacgaaccccaggctccctctgctgaggtggagatgacatcctatgtgctcctcgcttatctcacggcccagccagccccaacctcggaggacctgacctctgcaaccaacatcgtgaagtggatcacgaagcagcagaatgcccagggcggtttctcctccacccaggacacagtggtggctctccatgctctgtccaaatatggagcagccacatttaccaggactgggaaggctgcacaggtgactatccagtcttcagggacattttccagcaaattccaagtggacaacaacaaccgcctgttactgcagcaggtctcattgccagagctgcctggggaatacagcatgaaagtgacaggagaaggatgtgtctacctccagacatccttgaaatacaatattctcccagaaaaggaagagttcccctttgctttaggagtgcagactctgcctcaaacttgtgatgaacccaaagcccacaccagcttccaaatctccctaagtgtcagttacacagggagccgctctgcctccaacatggcgatcgttgatgtgaagatggtctctggcttcattcccctgaagccaacagtgaaaatgcttgaaagatctaaccatgtgagccggacagaagtcagcagcaaccatgtcttgatttaccttgataaggtgtcaaatcagacactgagcttgttcttcacggttctgcaagatgtcccagtaagagatctgaaaccagccatagtgaaagtctatgattactacgagacggatgagtttgcaattgctgagtacaatgctccttgcagcaaagatcttggaaatgcttgaagaccacaaggctgaaaagtgctttgctggagtcctgttctcagagctccacagaagacacgtgtttttgtatctttaaagacttgatgaataaacactttttctggtcaatgtc

SEQ ID NO: 72 - DNA, 4450 bp, Homo sapiens
gggaccagatggattgtagggagtagggtacaatacagtctgttctcctccagctccttctttctgcaacatggggaagaacaaactccttcatccaagtctggttcttctcctcttggtcctcctgcccacagacgcctcagtctctggaaaaccgcagtatatggttctggtcccctccctgctccacactgagaccactgagaagggctgtgtccttctgagctacctgaatgagacagtgactgtaagtgcttccttggagtctgtcaggggaaacaggagcctcttcactgacctggaggcggagaatgacgtactccactgtgtcgccttcgcttgaaatttcgtgttgtctccatggatgaaaactttcaccccctgaatgagttgattccactagtatacattcaggatcccaaaggaaatcgcatcgcacaatggcagagtttccagttagagggtggcctcaagcaattttcttttcccctctcatcagagcccttccagggctcctacaaggtggtggtacagaagaaatcaggtggaaggacagagcaccctttcaccgtggaggaatttgttcttcccaagtttgaagtacaagtaacagtgccaaagataatcaccatcttggaagaagagatgaatgtatcagtgtgtggcctatacacatatgggaagcctgtccctggacatgtgactgtgagcatttgcagaaagtatagtgacgcttccgactgccacggtgaagattcacaggctttctgtgagaaattcagtggacagctaaacagccatggctgcttctatcagcaagtaaaaaccaaggtcttccagctgaagaggaaggagtatgaaatgaaacttcacactgaggcccagatccaagaagaaggaacagtggtggaattgactggaaggcagtccagtgaaatcacaagaaccataaccaaactctcatttgtgaaagtggactcacactttcgacagggaattcccttctttgggcaggtgcgcctagtagatgggaaaggcgtccctataccaaataaagtcatattcatcagaggaaatgaagcaaactattactccaatgctaccacggatgagcatggccttgtacagttctctatcaacaccaccaatgttatgggtacctctcttactgttagggtcaattacaaggatcgtagtccctgttacggctaccagtgggtgtcagaagaacacgaagaggcacatcacactgcttatcttgtgttctccccaagcaagagctttgtccaccttgagcccatgtctcatgaactaccctgtggccatactcagacagtccaggcacattatattctgaatggaggcaccctgctggggctgaagaagctctccttctattatctgataatggcaaagggaggcattgtccgaactgggactcatggactgcttgtgaagcaggaagacatgaagggccatttttccatctcaatccctgtgaagtcagacattgctcctgtcgctcggttgctcatctatgctgttttacctaccggggacgtgattggggattctgcaaaatatgatgttgaaaattgtctggccaacaaggtggatttgagcttcagcccatcacaaagtctcccagcctcacacgcccacctgcgagtcacagcggctcctcagtccgtctgcgccctccgtgctgtggaccaaagcgtgctgctcatgaagcctgatgctgagctctcggcgtcctcggtttacaacctgctaccagaaaaggacctcactggcttccctgggcctttgaatgaccaggacaatgaagactgcatcaatcgtcataatgtctatattaatggaatcacatatactccagtatcaagtacaaatgaaaaggatatgtacagcttcctagaggacatgggcttaaaggcattcaccaactcaaagattcgtaaacccaaaatgtgtccacagcttcaacagtatgaaatgcatggacctgaaggtctacgtgtaggtttttatgagtcagatgtaatgggaagaggccatgcacgcctggtgcatgttgaagagcctcacacggagaccgtacgaaagtacttccctgagacatggatctgggatttggtggtggtaaactcagcaggtgtggctgaggtaggagtaacagtccctgacaccatcaccgagtggaaggcaggggccttctgcctgtctgaagatgctggacttggtatctcttccactgcctctctccgagccttccagcccttctttgtggagctcacaatgccttactctgtgattcgtggagaggccttcacactcaaggccacggtcctaaactaccttcccaaatgcatccgggtcagtgtgcagctggaagcctctcccgccttcctagctgtcccagtggagaaggaacaagcgcctcactgcatctgtgcaaacgggcggcaaactgtgtcctgggcagtaaccccaaagtcattaggaaatgtgaatttcactgtgagcgcagaggcactagagtctcaagagctgtgtgggactgaggtgccttcagttcctgaacacggaaggaaagacacagtcatcaagcctctgttggttgaacctgaaggactagagaaggaaacaacattcaactccctactttgtccatcaggtggtgaggtttctgaagaattatccctgaaactgccaccaaatgtggtagaagaatctgcccgagcttctgtctcagttttgggagacatattaggctctgccatgcaaaacacacaaaatcttctccagatgccctatggctgtggagagcagaatatggtcctctttgctcctaacatctatgtactggattatctaaatgaaacacagcagcttactccagagatcaagtccaaggccattggctatctcaacactggttaccagagacagttgaactacaaacactatgatggctcctacagcacctttggggagcgatatggcaggaaccagggcaacacctggctcacagcctttgttctgaagacttttgcccaagctcgagcctacatcttcatcgatgaagcacacattacccaagccctcatatggctctcccagaggcagaaggacaatggctgtttcaggagctctgggtcactgctcaacaatgccataaagggaggagtagaagatgaagtgaccctctccgcctatatcaccatcgcccttctggagattcctctcacagtcactcaccctgttgtccgcaatgccctgttttgcctggagtcagcctggaagacagcacaagaaggggaccatggcagccatgtatataccaaagcactgctggcctatgcttttgccctggcaggtaaccaggacaagaggaaggaagtactcaagtcacttaatgaggaagctgtgaagaaagacaactctgtccattgggagcgccctcagaaacccaaggcaccagtggggcatttttacgaaccccaggctccctctgctgaggtggagatgacatcctatgtgctcctcgcttatctcacggcccagccagccccaacctcggaggacctgacctctgcaaccaacatcgtgaagtggatcacgaagcagcagaatgcccagggcggtttctcctccacccaggacacagtggtggctctccatgctctgtccaaatatggagcagccacatttaccaggactgggaaggctgcacaggtgactatccagtcttcagggacattttccagcaaattccaagtggacaacaacaaccgcctgttactgcagcaggtctcattgccagagctgcctggggaatacagcatgaaagtgacaggagaaggatgtgtctacctccagacatccttgaaatacaatattctcccagaaaaggaagagttcccctttgctttaggagtgcagactctgcctcaaacttgtgatgaacccaaagcccacaccagcttccaaatctccctaagtgtcagttacacagggagccgctctgcctccaacatggcgatcgttgatgtgaagatggtctctggcttcattcccctgaagccaacagtgaaaatgcttgaaagatctaaccatgtgagccggacagaagtcagcagcaaccatgtcttgatttaccttgataaggtgtcaaatcagacactgagcttgttcttcacggttctgcaagatgtcccagtaagagatctgaaaccagccatagtgaaagtctatgattactacgagacggatgagtttgcaattgctgagtacaatgctccttgcagcaaagatcttggaaatgcttgaagaccacaaggctgaaaagtgctttgctggagtcctgttctcagagctccacagaagacacgtgtttttgtatctttaaagacttgatgaataaacactttttctggtcaatgtc

SEQ ID NO: 73 - DNA, 1324 bp, Mus musculus
caagcttgcaagctcctttctgtaactcagcagtcatgagagtttctgtgtgatgtgttatgcgtgactctactgggtgttgtgagaggaggttagtcaagctcagaactccaaacatgtgtcttcgctggatgctgtgaatttagctcaagcaagctcagaacttcacacatggatttagtcacctatgatgacgtgcaggtgaacttcactcaggatgagtgggctttgctggatccttctcagaagagtctctacaagggtgtgatgctagagacctacaggaatctcacagctataggttacatttgggaagaacatacgattgaagaccattttcaaacttctcgaagtcatggaaggtaattttactctgcaagctgaggagaaaatgcctatgaagaaagtttaacttgtggtacaagtagtaaagaaaaccaatagggtacaataagcactgctttcagtgatggatgtttactgactttcataaaaatcatatatgtttatggcagatatgtaactgttgtttgcaagacattccattaggtcaaagacagagaaataatggcttaacacatatgttactgtttaaatcaagcctagtacagccatgctatacaagtgtgagtgtcttcagtcttatatcgcttagctattgcaaaaggaacacatagtgattaggtgacaagtatatgtctaaaacctagtaatgagcaaataatccatagtatatctgagctcaatgatatacttgtaataacattgctaaatttagtgagatgaacagttcataagattcaaaaatggttttgtggaaaaaccttaatctctgtaccacatctctgtgacaaaaaaaagtcagctgtgaatgtaatgtggaattttcacttgttattcttcttttgatgtggatgtcataggttacaattgatacaagccttgtgatcactggggcattgaaagaagccacatacctttcacttttccagaacaattagaggatatgcagtataacatattttgaacaacatacttaatgtgctatataagtttataaaaaatttgtttccgaacattgctgggaacatttaccaactctaactgctgaaaatagtaatgagaattaaggcagtagaaaatttttttcttttgcatttgttcatattccaaatgtagtattactctcatgataacaaaatttgtgaatgcaatcattgtgcaaacactgtgagttcttcctgtttttttcaaatatgtgagtaaccttttatagaaaaagtatgttataaatgtgagcctgataatcaaaaaaaaaaaaaaa

SEQ ID NO: 74 - DNA, 1475 bp, Mus musculus
agccaccagcagctcacactgaagaagcatccttgcttgggtttgcagtcttctgcggcaggcattctcggaggaaaccagccaaggtaagcctgcagtggcccatgaggctgcagttctcctggctgaattctgagggactaactacgaccatgagattggcagtgatttgcttttgcctgtttggcattgcctcctccctcccggtgaaagtgactgattctggcagctcagaggagaagaagctttacagcctgcacccagatcctatagccacatggctggtgcctgacccatctcagaagcagaatctccttgcgccacagaatgctgtgtcctctgaagaaaaggatgactttaagcaagaaactcttccaagcaattccaatgaaagccatgaccacatggacgacgatgatgacgatgatgatgacgatggagaccatgcagagagcgaggattctgtggactcggatgaatctgacgaatctcaccattcggatgagtctgatgagaccgtcactgctagtacacaagcagacactttcactccaatcgtccctacagtcgatgtccccaacggccgaggtgatagcttggcttatggactgaggtcaaagtctaggagtttccaggtttctgatgaacagtatcctgatgccacagatgaggacctcacctctcacatgaagagcggtgagtctaaggagtccctcgatgtcatccctgttgcccagcttctgagcatgccctctgatcaggacaacaacggaaagggcagccatgagtcaagtcagctggatgaaccaagtctggaaacacacagacttgagcattccaaagagagccaggagagtgccgatcagtcggatgtgatcgatagtcaagcaagttccaaagccagcctggaacatcagagccacaagtttcacagccacaaggacaagctagtcctagaccctaagagtaaggaagatgataggtatctgaaattccgaatttctcatgaattagagagttcatcttctgaggtcaactaaagaagaggcaaaaacacagttccttactttgcatttagtaaaaacaagaaaaagtgttagtgagggttaagcaggaatactaactgctcatttctcagttcagtggatatatgtatgtagagaaagagaggtaatattttgggctcttagcttagtctgttgtttcatgcaaacaccgttgtaaccaaaagcttctgcactttgcttctgttcttcctgtacaagaaatgcaaacggccactgcattttaatgattgttattcttttatgaataaaatgtatgtagaaacaagcaaatttactgaaacaagcagaattaaaagagaaactgtaacagtctatatcactatacccttttagttttataattagcatatattttgttgtgattattttttttgttggtgtgaataaatcttgtaacgaatgtaagga

SEQ ID NO: 75 - DNA, 1480 bp, Mus musculus
agccaccagcagctcacactgaagaagcatccttgcttgggtttgcagtcttctgcggcaggcattctcggaggaaaccagccaaggtaagcctgcagtggcccatgaggctgcagttctcctggctgaattctgagggactaactacgaccatgagattggcagtgatttgcttttgcctgtttggcattgcctcctccctcccggtgaaagtgactgattctggcagctcagaggagaagctttacagcctgcacccagatcctatagccacatggctggtgcctgacccatctcagaagcagaatctccttgcgccacagaatgctgtgtcctctgaagaaaaggatgactttaagcaagaaactcttccaagcaattccaatgaaagccatgaccacatggacgacgatgatgacgatgatgatgacgatggagaccatgcagagagcgaggattctgtggactcggatgaatctgacgaatctcaccattcggatgagtctgatgagaccgtcactgctagtacacaagcagacactttcactccaatcgtccctacagtcgatgtccccaacggccgaggtgatagcttggcttatggactgaggtcaaagtctaggagtttccaggtttctgatgaacagtatcctgatgccacagatgaggacctcacctctcacatgaagagcggtgagtctaaggagtccctcgatgtcatccctgttgcccagcttctgagcatgccctctgatcaggacaacaacggaaagggcagccatgagtcaagtcagctggatgaaccaagtctggaaacacacagacttgagcattccaaagagagccaggagagtgccgatcagtcggatgtgatcgatagtcaagcaagttccaaagccagcctggaacatcagagccacaagtttcacagccacaaggacaagctagtcctagaccctaagagtaaggaagatgataggtatctgaaattccgaatttctcatgaattagagagttcatcttctgaggtcaactaaagaagaggcaaaaacacagttccttactttgcatttagtaaaaacaagaaaaagtgttagtgagggttaagcaggaatactaactgctcatttctcagttcagtggatatatgtatgtagagaaagagaggtaatattttgggctcttagcttagtctgttgtttcatgcaaacaccgttgtaaccaaaagcttctgcactttgcttctgttcttcctgtacaagaaatgcaaacggccactgcattttaatgattgttattcttttatgaataaaatgtatgtagaaacaagcaaatttactgaaacaagcagaattaaaagagaaactgtaacagtctatatcactatacccttttagttttataattagcatatattttgttgtgattattttttttgttggtgtgaataaatcttgtaacgaatgtaaggaaaaaaaaa

SEQ ID NO: 76 - DNA, 1423 bp, Mus musculus
agccaccagcagctcacactgaagaagcatccttgcttgggtttgcagtcttctgcggcaggcattctcggaggaaaccagccaaggactaactacgaccatgagattggcagtgatttgcttttgcctgtttggcattgcctcctccctcccggtgaaagtgactgattctggcagctcagaggagaagaagctttacagcctgcacccagatcctatagccacatggctggtgcctgacccatctcagaagcagaatctccttgcgccacagaatgctgtgtcctctgaagaaaaggatgactttaagcaagaaactcttccaagcaattccaatgaaagccatgaccacatggacgacgatgatgacgatgatgatgacgatggagaccatgcagagagcgaggattctgtggactcggatgaatctgacgaatctcaccattcggatgagtctgatgagaccgtcactgctagtacacaagcagacactttcactccaatcgtccctacagtcgatgtccccaacggccgaggtgatagcttggcttatggactgaggtcaaagtctaggagtttccaggtttctgatgaacagtatcctgatgccacagatgaggacctcacctctcacatgaagagcggtgagtctaaggagtccctcgatgtcatccctgttgcccagcttctgagcatgccctctgatcaggacaacaacggaaagggcagccatgagtcaagtcagctggatgaaccaagtctggaaacacacagacttgagcattccaaagagagccaggagagtgccgatcagtcggatgtgatcgatagtcaagcaagttccaaagccagcctggaacatcagagccacaagtttcacagccacaaggacaagctagtcctagaccctaagagtaaggaagatgataggtatctgaaattccgaatttctcatgaattagagagttcatcttctgaggtcaactaaagaagaggcaaaaacacagttccttactttgcatttagtaaaaacaagaaaaagtgttagtgagggttaagcaggaatactaactgctcatttctcagttcagtggatatatgtatgtagagaaagagaggtaatattttgggctcttagcttagtctgttgtttcatgcaaacaccgttgtaaccaaaagcttctgcactttgcttctgttcttcctgtacaagaaatgcaaacggccactgcattttaatgattgttattcttttatgaataaaatgtatgtagaaacaagcaaatttactgaaacaagcagaattaaaagagaaactgtaacagtctatatcactatacccttttagttttataattagcatatattttgttgtgattattttttttgttggtgtgaataaatcttgtaacgaatgtaagga

SEQ ID NO: 77 - DNA, 1517 bp, Mus musculus
tttccttgctaaggatgagaggtggagaggtagaaaaggcacacaaatattgactcactgaaattttctctgagatgtagaaagattccataaattattggtgacttggtggtgatctagtggtgccaagagtgtgtttgaacctgacaagacatcaactgtgcctcataaaatatgttgcaggactaactacgaccatgagattggcagtgatttgcttttgcctgtttggcattgcctcctccctcccggtgaaagtgactgattctggcagctcagaggagaagctttacagcctgcacccagatcctatagccacatggctggtgcctgacccatctcagaagcagaatctccttgcgccacagaatgctgtgtcctctgaagaaaaggatgactttaagcaagaaactcttccaagcaattccaatgaaagccatgaccacatggacgacgatgatgacgatgatgatgacgatggagaccatgcagagagcgaggattctgtggactcggatgaatctgacgaatctcaccattcggatgagtctgatgagaccgtcactgctagtacacaagcagacactttcactccaatcgtccctacagtcgatgtccccaacggccgaggtgatagcttggcttatggactgaggtcaaagtctaggagtttccaggtttctgatgaacagtatcctgatgccacagatgaggacctcacctctcacatgaagagcggtgagtctaaggagtccctcgatgtcatccctgttgcccagcttctgagcatgccctctgatcaggacaacaacggaaagggcagccatgagtcaagtcagctggatgaaccaagtctggaaacacacagacttgagcattccaaagagagccaggagagtgccgatcagtcggatgtgatcgatagtcaagcaagttccaaagccagcctggaacatcagagccacaagtttcacagccacaaggacaagctagtcctagaccctaagagtaaggaagatgataggtatctgaaattccgaatttctcatgaattagagagttcatcttctgaggtcaactaaagaagaggcaaaaacacagttccttactttgcatttagtaaaaacaagaaaaagtgttagtgagggttaagcaggaatactaactgctcatttctcagttcagtggatatatgtatgtagagaaagagaggtaatattttgggctcttagcttagtctgttgtttcatgcaaacaccgttgtaaccaaaagcttctgcactttgcttctgttcttcctgtacaagaaatgcaaacggccactgcattttaatgattgttattcttttatgaataaaatgtatgtagaaacaagcaaatttactgaaacaagcagaattaaaagagaaactgtaacagtctatatcactatacccttttagttttataattagcatatattttgttgtgattattttttttgttggtgtgaataaatcttgtaacgaatgtaagga

SEQ ID NO: 78 - DNA, 1428 bp, Mus musculus
agccaccagcagctcacactgaagaagcatccttgcttgggtttgcagtcttctgcggcaggcattctcggaggaaaccagccaaggactaactacgaccatgagattggcagtgatttgcttttgcctgtttggcattgcctcctccctcccggtgaaagtgactgattctggcagctcagaggagaagctttacagcctgcacccagatcctatagccacatggctggtgcctgacccatctcagaagcagaatctccttgcgccacagaatgctgtgtcctctgaagaaaaggatgactttaagcaagaaactcttccaagcaattccaatgaaagccatgaccacatggacgacgatgatgacgatgatgatgacgatggagaccatgcagagagcgaggattctgtggactcggatgaatctgacgaatctcaccattcggatgagtctgatgagaccgtcactgctagtacacaagcagacactttcactccaatcgtccctacagtcgatgtccccaacggccgaggtgatagcttggcttatggactgaggtcaaagtctaggagtttccaggtttctgatgaacagtatcctgatgccacagatgaggacctcacctctcacatgaagagcggtgagtctaaggagtccctcgatgtcatccctgttgcccagcttctgagcatgccctctgatcaggacaacaacggaaagggcagccatgagtcaagtcagctggatgaaccaagtctggaaacacacagacttgagcattccaaagagagccaggagagtgccgatcagtcggatgtgatcgatagtcaagcaagttccaaagccagcctggaacatcagagccacaagtttcacagccacaaggacaagctagtcctagaccctaagagtaaggaagatgataggtatctgaaattccgaatttctcatgaattagagagttcatcttctgaggtcaactaaagaagaggcaaaaacacagttccttactttgcatttagtaaaaacaagaaaaagtgttagtgagggttaagcaggaatactaactgctcatttctcagttcagtggatatatgtatgtagagaaagagaggtaatattttgggctcttagcttagtctgttgtttcatgcaaacaccgttgtaaccaaaagcttctgcactttgcttctgttcttcctgtacaagaaatgcaaacggccactgcattttaatgattgttattcttttatgaataaaatgtatgtagaaacaagcaaatttactgaaacaagcagaattaaaagagaaactgtaacagtctatatcactatacccttttagttttataattagcatatattttgttgtgattattttttttgttggtgtgaataaatcttgtaacgaatgtaaggaaaaaaaaa

SEQ ID NO: 79 - DNA, 1519 bp, Homo sapiens
agcagcaggaggaggcagagcacagcatcgtcgggaccagactcgtctcaggccagttgcagccttctcagccaaacgccgaccaaggaaaactcactaccatgagaattgcagtgatttgcttttgcctcctaggcatcacctgtgccataccagttaaacaggctgattctggaagttctgaggaaaagcagctttacaacaaatacccagatgctgtggccacatggctaaaccctgacccatctcagaagcagaatctcctagccccacagacccttccaagtaagtccaacgaaagccatgaccacatggatgatatggatgatgaagatgatgatgaccatgtggacagccaggactccattgactcgaacgactctgatgatgtagatgacactgatgattctcaccagtctgatgagtctcaccattctgatgaatctgatgaactggtcactgattttcccacggacctgccagcaaccgaagttttcactccagttgtccccacagtagacacatatgatggccgaggtgatagtgtggtttatggactgaggtcaaaatctaagaagtttcgcagacctgacatccagtaccctgatgctacagacgaggacatcacctcacacatggaaagcgaggagttgaatggtgcatacaaggccatccccgttgcccaggacctgaacgcgccttctgattgggacagccgtgggaaggacagttatgaaacgagtcagctggatgaccagagtgctgaaacccacagccacaagcagtccagattatataagcggaaagccaatgatgagagcaatgagcattccgatgtgattgatagtcaggaactttccaaagtcagccgtgaattccacagccatgaatttcacagccatgaagatatgctggttgtagaccccaaaagtaaggaagaagataaacacctgaaatttcgtatttctcatgaattagatagtgcatcttctgaggtcaattaaaaggagaaaaaatacaatttctcactttgcatttagtcaaaagaaaaaatgctttatagcaaaatgaaagagaacatgaaatgcttctttctcagtttattggttgaatgtgtatctatttgagtctggaaataactaatgtgtttgataattagtttagtttgtggcttcatggaaactccctgtaaactaaaagcttcagggttatgtctatgttcattctatagaagaaatgcaaactatcactgtattttaatatttgttattctctcatgaatagaaatttatgtagaagcaaacaaaatacttttacccacttaaaaagagaatataacattttatgtcactataatcttttgttttttaagttagtgtatattttgttgtgattatctttttgtggtgtgaataaatcttttatcttgaatgtaataagaatttggtggtgtcaattgcttatttgttttcccacggttgtccagcaattaataaaacataaccttttttactgccta

SEQ ID NO: 80 - DNA, 1561 bp, Homo sapiens
agcagcaggaggaggcagagcacagcatcgtcgggaccagactcgtctcaggccagttgcagccttctcagccaaacgccgaccaaggaaaactcactaccatgagaattgcagtgatttgcttttgcctcctaggcatcacctgtgccataccagttaaacaggctgattctggaagttctgaggaaaagcagctttacaacaaatacccagatgctgtggccacatggctaaaccctgacccatctcagaagcagaatctcctagccccacagaatgctgtgtcctctgaagaaaccaatgactttaaacaagagacccttccaagtaagtccaacgaaagccatgaccacatggatgatatggatgatgaagatgatgatgaccatgtggacagccaggactccattgactcgaacgactctgatgatgtagatgacactgatgattctcaccagtctgatgagtctcaccattctgatgaatctgatgaactggtcactgattttcccacggacctgccagcaaccgaagttttcactccagttgtccccacagtagacacatatgatggccgaggtgatagtgtggtttatggactgaggtcaaaatctaagaagtttcgcagacctgacatccagtaccctgatgctacagacgaggacatcacctcacacatggaaagcgaggagttgaatggtgcatacaaggccatccccgttgcccaggacctgaacgcgccttctgattgggacagccgtgggaaggacagttatgaaacgagtcagctggatgaccagagtgctgaaacccacagccacaagcagtccagattatataagcggaaagccaatgatgagagcaatgagcattccgatgtgattgatagtcaggaactttccaaagtcagccgtgaattccacagccatgaatttcacagccatgaagatatgctggttgtagaccccaaaagtaaggaagaagataaacacctgaaatttcgtatttctcatgaattagatagtgcatcttctgaggtcaattaaaaggagaaaaaatacaatttctcactttgcatttagtcaaaagaaaaaatgctttatagcaaaatgaaagagaacatgaaatgcttctttctcagtttattggttgaatgtgtatctatttgagtctggaaataactaatgtgtttgataattagtttagtttgtggcttcatggaaactccctgtaaactaaaagcttcagggttatgtctatgttcattctatagaagaaatgcaaactatcactgtattttaatatttgttattctctcatgaatagaaatttatgtagaagcaaacaaaatacttttacccacttaaaaagagaatataacattttatgtcactataatcttttgttttttaagttagtgtatattttgttgtgattatctttttgtggtgtgaataaatcttttatcttgaatgtaataagaatttggtggtgtcaattgcttatttgttttcccacggttgtccagcaattaataaaacataaccttttttactgccta

SEQ ID NO: 81 - DNA, 2219 bp, Mus musculus
gaggtttacaaagcatttcctgggacgaggctgaggaaagccacatggtggagcttttctctgctgaacagtctacagaaggcttccagttgcagccaggaaggaggctccaggactgccttcagccactgcctcgctgcctgagggacagttgagtccctctcttgctcccagggttgggcttctaggccaggcaatggctctcctgtggctcctctctgtgttcttgctggttccagggactcaaggtacagaagatggagacatgcgcttggttaacggggcctcagccaatgagggccgcgtggagatcttctacagaggccggtgggggacagtgtgtgacaacctctggaaccttttggatgcccacgtcgtctgccgggccctgggctatgagaacgccacccaagcactgggcagagctgccttcgggccaggaaagggaccgatcatgctggatgaggtggaatgtacagggaccgagtcctcactggccagttgcagatccctgggttggatggtgagccgctgtgggcacgagaaggacgcaggcgtggtctgctccaacgataccacggggcttcacatcctggacctctctggagagctctcagatgcactgggccagatctttgacagccagcagggctgcgacctattcatccaggtgacagggcaggggtatgaggacctgagcctctgtgcccacacgctgatcctgcgcaccaaccccgaggcccaggccctgtggcaagtggtgggcagcagcgtcatcatgagagtggatgctgagtgcatgcctgtcgtcagagacttcctcaggtacttttactcccgaagaatcgaggtcagcatgtcttctgttaagtgcttgcacaagctagcctctgcctatggggccacagagcttcaggactactgtggacggctttttgccaccctcctcccccaagaccccactttccatactcccttggacctttatgcgtacgcacgggccaccggggactctatgctggaagatctgtgtgtacagtttctggcctggaacttcgagcctctgacacagtctgagtcctggtcggctgttcccaccaccttgatccaggctctcctccccaagagtgagctggctgtgtctagtgagctggatctgctgaaggcagtggaccagtggagcacagaaaccattgcctcacacgaggatatagagcgcctggtggaacaggtccgcttccccatgatgctgccccaggagctgttcgagctgcagttcaacctgtccttgtaccaagatcaccaggcactgttccagaggaagaccatgcaggccttggagttccacacagtgcctgtcgaagtgctggccaagtacaaaggcctgaacctcacggaggacacctacaagccccgcctttacacctcttccacctggagtagcttggtgatggcctccacctggagggcacaaagatatgaatacaatcgatacaatcagctctatacatatggctatggctcagtagcccggtacaatagctaccagtccttccaaaccccacaacaccccagcttcctcttcaaggacaagcagatctcctggtcagccacctacctccccaccatgcagagctgctggaactatggcttctcgtgtacctctaacgagctccctgtactgggcctcaccacatccagctactccaatccgacaattggctatgagaacagagtactgatcctctgcggaggctacagtgtggtggatgtcaccagctttgaaggctccaaggcccctattcccactgccctggacaccaatagttccaagactccctccctctttccctgtgcctcaggggcctttagcagcttccgtgtggtcatacgccccttctacctcactaactccactgacatggtgtaaatggtacatctcagtggtggggacgcagacattcctgtgtcccctccttcgcctccagctgctttgtaagcataaactgattgtattcaaatgaaaatttactagaaggtttcagccagcactcactccaggactgagagtcccagggccctcactgcaggtacaagcaggttccatgaggtcctgtgggatttcctgtgcctactgcagtagccccatctgtcacagtcactcatcaaaaatcattaaagtctcacgtgcttctcacgaaaaaaaaaaaaaaaaaaaa

SEQ ID NO: 82 - DNA, 2202 bp, Homo sapiens
atactgggagaggcttctgggtcaaaggaccagtctgcagagggatcctgtggctggaagcgaggaggctccacacggccgttgcagctaccgcagccaggatctgggcatccaggcacggccatgacccctccgaggctcttctgggtgtggctgctggttgcaggaacccaaggcgtgaacgatggtgacatgcggctggccgatgggggcgccaccaaccagggccgcgtggagatcttctacagaggccagtggggcactgtgtgtgacaacctgtgggacctgactgatgccagcgtcgtctgccgggccctgggcttcgagaacgccacccaggctctgggcagagctgccttcgggcaaggatcaggccccatcatgctggatgaggtccagtgcacgggaaccgaggcctcactggccgactgcaagtccctgggctggctgaagagcaactgcaggcacgagagagacgctggtgtggtctgcaccaatgaaaccaggagcacccacaccctggacctctccagggagctctcggaggcccttggccagatctttgacagccagcggggctgcgacctgtccatcagcgtgaatgtgcagggcgaggacgccctgggcttctgtggccacacggtcatcctgactgccaacctggaggcccaggccctgtggaaggagccgggcagcaatgtcaccatgagtgtggatgctgagtgtgtgcccatggtcagggaccttctcaggtacttctactcccgaaggattgacatcaccctgtcgtcagtcaagtgcttccacaagctggcctctgcctatggggccaggcagctgcagggctactgcgcaagcctctttgccatcctcctcccccaggacccctcgttccagatgcccctggacctgtatgcctatgcagtggccacaggggacgccctgctggagaagctctgcctacagttcctggcctggaacttcgaggccttgacgcaggccgaggcctggcccagtgtccccacagacctgctccaactgctgctgcccaggagcgacctggcggtgcccagcgagctggccctactgaaggccgtggacacctggagctggggggagcgtgcctcccatgaggaggtggagggcttggtggagaagatccgcttccccatgatgctccctgaggagctctttgagctgcagttcaacctgtccctgtactggagccacgaggccctgttccagaagaagactctgcaggccctggaattccacactgtgcccttccagttgctggcccggtacaaaggcctgaacctcaccgaggatacctacaagccccggatttacacctcgcccacctggagtgcctttgtgacagacagttcctggagtgcacggaagtcacaactggtctatcagtccagacgggggcctttggtcaaatattcttctgattacttccaagccccctctgactacagatactacccctaccagtccttccagactccacaacaccccagcttcctcttccaggacaagagggtgtcctggtccctggtctacctccccaccatccagagctgctggaactacggcttctcctgctcctcggacgagctccctgtcctgggcctcaccaagtctggcggctcagatcgcaccattgcctacgaaaacaaagccctgatgctctgcgaagggctcttcgtggcagacgtcaccgatttcgagggctggaaggctgcgattcccagtgccctggacaccaacagctcgaagagcacctcctccttcccctgcccggcagggcacttcaacggcttccgcacggtcatccgccccttctacctgaccaactcctcaggtgtggactagacggcgtggcccaagggtggtgagaaccggagaaccccaggacgccctcactgcaggctcccctcctcggcttccttcctctctgcaatgaccttcaacaaccggccaccagatgtcgccctactcacctgagcgctcagcttcaagaaattactggaaggcttccactagggtccaccaggagttctcccaccacctcaccagtttccaggtggtaagcaccaggacgccctcgaggttgctctgggatccccccacagcccctggtcagtctgcccttgtcactggtctgaggtcattaaaattacattgaggttccta

SEQ ID NO: 83 - DNA, 432 bp, Mus musculus
gtgcaggatcctcccaccgccatgggcctcctgagagatccttagatccagggtgcccctccaaccaggatgaggctcttcatcgctcttcctgtcctgattgtggtcgtagccatgaccttggaaggcccagcccccgcccaggcggccccggatttgtccggaacattggagagcataccggataaactgaaggagtttgggaacactttggaagacaaggcccgggcagccattgaacatatcaaacagaaggaaattttgaccaagacccgggcctggttctcagaggcatttggcaaagtgaaggagaagttgaagaccacgttctcctgagcacctggcgggccacctcgaagcatcaaggacatccacgtaatgtgccaggtccctcttcatcacagaccaataaaaaacgtgtagaaggcaaac

SEQ ID NO: 84 - DNA, 554 bp, Mus musculus
gtgcaggatcctcccaccgccatgggcctcctgagagatccttagatccaggttagtgcataggaaagtgtccccccactacctacagctaagggattggggtggtgggatcatggtggagggcggtggtgaatactagcgatgtcccccgctacccgtgcgtctgcctccagggtgcccctccaaccaggatgaggctcttcatcgctcttcctgtcctgattgtggtcgtagccatgaccttggaaggcccagcccccgcccaggcggccccggatttgtccggaacattggagagcataccggataaactgaaggagtttgggaacactttggaagacaaggcccgggcagccattgaacatatcaaacagaaggaaattttgaccaagacccgggcctggttctcagaggcatttggcaaagtgaaggagaagttgaagaccacgttctcctgagcacctggcgggccacctcgaagcatcaaggacatccacgtaatgtgccaggtccctcttcatcacagaccaataaaaaacgtgtagaaggcaaac

SEQ ID NO: 85 - DNA, 553 bp, Homo sapiens
gagctcggctcttgagacaggaatcttgcccattccccgaacgaataaaccccttccttaactcagcgtctgaggaattttgtctgcggctcctcctgctacattctgagtggggaaagggactaaggtggtctgaggaccccacagagtcaggaagattgagagagtgcccctccggcctcgccatgaggctcttcctgtcgctcccggtcctggtggtggttctgtcgatcgtcttggaaggcccagccccagcccaggggaccccagacgtctccagtgccttggataagctgaaggagtttggaaacacactggaggacaaggctcgggaactcatcagccgcatcaaacagagtgaactttctgccaagatgcgggagtggttttcagagacatttcagaaagtgaaggagaaactcaagattgactcatgaggacctgaagggtgacatcccaggaggggcctctgaaatttcccacaccccagcgcctgtgctgaggactccctccatgtggccccaggtgccaccaataaaaatcctacagaaaa

SEQ ID NO: 86 - DNA, 615 bp, Homo sapiens
gagctcggctcttgagacaggaatcttgcccattccccgaacgaataaaccccttccttaactcagcgtctgaggaattttgtctgcggctcctcctgctacattctgagtggggaaagggactaaggtggtctgaggaccccacagagtcaggaagattgagagcctgataaaggtcctgcgggcaggacaggacctcccaaccaagccctccagcaaggattcagagtgcccctccggcctcgccatgaggctcttcctgtcgctcccggtcctggtggtggttctgtcgatcgtcttggaaggcccagccccagcccaggggaccccagacgtctccagtgccttggataagctgaaggagtttggaaacacactggaggacaaggctcgggaactcatcagccgcatcaaacagagtgaactttctgccaagatgcgggagtggttttcagagacatttcagaaagtgaaggagaaactcaagattgactcatgaggacctgaagggtgacatcccaggaggggcctctgaaatttcccacaccccagcgcctgtgctgaggactccctccatgtggccccaggtgccaccaataaaaatcctacagaaaa

SEQ ID NO: 87 - DNA, 595 bp, Homo sapiens
cctgataaaggtcctgcgggcaggacaggacctcccaaccaagccctccagcaaggattcagagtgcccctccggcctcgccatgaggctcttcctgtcgctcccggtcctggtggtggttctgtcgatcgtcttggaaggcccagccccagcccaggggaccccagacgtctccagtgccttggataagctgaaggagtttggaaacacactggaggacaaggctcgggaactcatcagccgcatcaaacagagtgaactttctgccaagatgcggttagaacccttcccagggcacgggagagctggggtgtgtttttgggtggagccctggcagatggtccaagatgaacagattgaaaaaaaaacaagtcctggagaggctgacaacatccctctggtcacacagctagatctcaagggagtggttttcagagacatttcagaaagtgaaggagaaactcaagattgactcatgaggacctgaagggtgacatcccaggaggggcctctgaaatttcccacaccccagcgcctgtgctgaggactccctccatgtggccccaggtgccaccaataaaaatcctacagaaaa

SEQ ID NO: 88 - DNA, 514 bp, Homo sapiens
aggcggtcaggggaaggctcaggaggagggagatcaacatcaacctgccccgccccctccccagcctgataaaggtcctgcgggcaggacaggacctcccaaccaagccctccagcaaggattcagagtgcccctccggcctcgccatgaggctcttcctgtcgctcccggtcctggtggtggttctgtcgatcgtcttggaaggcccagccccagcccaggggaccccagacgtctccagtgccttggataagctgaaggagtttggaaacacactggaggacaaggctcgggaactcatcagccgcatcaaacagagtgaactttctgccaagatgcgggagtggttttcagagacatttcagaaagtgaaggagaaactcaagattgactcatgaggacctgaagggtgacatcccaggaggggcctctgaaatttcccacaccccagcgcctgtgctgaggactccctccatgtggccccaggtgccaccaataaaaatcctacagaaaa

SEQ ID NO: 89 - protein, 589 aa, Mus musculus
MWVLMSWLAFAAGLVAGTQCPDGQFCPVACCLDQGGANYSCCNPLLDTWPRITSHHLDGSCQTHGHCPAGYSCLLTVSGTSSCCPFSKGVSCGDGYHCCPQGFHCSADGKSCFQMSDNPLGAVQCPGSQFECPDSATCCIMVDGSWGCCPMPQASCCEDRVHCCPHGASCDLVHTRCVSPTGTHTLLKKFPAQKTNRAVSLPFSVVCPDAKTQCPDDSTCCELPTGKYGCCPMPNAICCSDHLHCCPQDTVCDLIQSKCLSKNYTTDLLTKLPGYPVKEVKCDMEVSCPEGYTCCRLNTGAWGCCPFAKAVCCEDHIHCCPAGFQCHTEKGTCEMGILQVPWMKKVIAPLRLPDPQILKSDTPCDDFTRCPTNNTCCKLNSGDWGCCPIPEAVCCSDNQHCCPQGFTCLAQGYCQKGDTMVAGLEKIPARQTTPLQIGDIGCDQHTSCPVGQTCCPSLKGSWACCQLPHAVCCEDRQHCCPAGYTCNVKARTCEKDVDFIQPPVLLTLGPKVGNVECGEGHFCHDNQTCCKDSAGVWACCPYLKGVCCRDGRHCCPGGFHCSARGTKCLRKKIPRWDMFLRDPVPRPLL

SEQ ID NO: 90 - protein, 593 aa, Homo sapiens
MWTLVSWVALTAGLVAGTRCPDGQFCPVACCLDPGGASYSCCRPLLDKWPTTLSRHLGGPCQVDAHCSAGHSCIFTVSGTSSCCPFPEAVACGDGHHCCPRGFHCSADGRSCFQRSGNNSVGAIQCPDSQFECPDFSTCCVMVDGSWGCCPMPQASCCEDRVHCCPHGAFCDLVHTRCITPTGTHPLAKKLPAQRTNRAVALSSSVMCPDARSRCPDGSTCCELPSGKYGCCPMPNATCCSDHLHCCPQDTVCDLIQSKCLSKENATTDLLTKLPAHTVGDVKCDMEVSCPDGYTCCRLQSGAWGCCPFTQAVCCEDHIHCCPAGFTCDTQKGTCEQGPHQVPWMEKAPAHLSLPDPQALKRDVPCDNVSSCPSSDTCCQLTSGEWGCCPIPEAVCCSDHQHCCPQGYTCVAEGQCQRGSEIVAGLEKMPARRASLSHPRDIGCDQHTSCPVGQTCCPSLGGSWACCQLPHAVCCEDRQHCCPAGYTCNVKARSCEKEVVSAQPATFLARSPHVGVKDVECGEGHFCHDNQTCCRDNRQGWACCPYRQGVCCADRRHCCPAGFRCAARGTKCLRREAPRWDAPLRDPALRQLL

SEQ ID NO: 91 - protein, 410 aa, Mus musculus
MKTPGVLLLILGLLASSSFAIIRIPLRKFTSIRRTMTEVGGSVEDLILKGPITKYSMQSSPKTTEPVSELLKNYLDAQYYGDIGIGTPPQCFTVVFDTGSSNLWVPSIHCKILDIACWVHHKYNSDKSSTYVKNGTSFDIHYGSGSLSGYLSQDTVSVPCKSDQSKARGIKVEKQIFGEATKQPGIVFVAAKFDGILGMGYPHISVNNVLPVFDNLMQQKLVDKNIFSFYLNRDPEGQPGGELMLGGTDSKYYHGELSYLNVTRKAYWQVHMDQLEVGNELTLCKGGCEAIVDTGTSLLVGPVEEVKELQKAIGAVPLIQGEYMIPCEKVSSLPTVYLKLGGKNYELHPDKYILKVSQGGKTICLSGFMGMDIPPPSGPLWILGDVFIGSYYTVFDRDNNRVGFANAVVL

SEQ ID NO: 92 - protein, 412 aa, Homo sapiens
MQPSSLLPLALCLLAAPASALVRIPLHKFTSIRRTMSEVGGSVEDLIAKGPVSKYSQAVPAVTEGPIPEVLKNYMDAQYYGEIGIGTPPQCFTVVFDTGSSNLWVPSIHCKLLDIACWIHHKYNSDKSSTYVKNGTSFDIHYGSGSLSGYLSQDTVSVPCQSASSASALGGVKVERQVFGEATKQPGITFIAAKFDGILGMAYPRISVNNVLPVFDNLMQQKLVDQNIFSFYLSRDPDAQPGGELMLGGTDSKYYKGSLSYLNVTRKAYWQVHLDQVEVASGLTLCKEGCEAIVDTGTSLMVGPVDEVRELQKAIGAVPLIQGEYMIPCEKVSTLPAITLKLGGKGYKLSPEDYTLKVSQAGKTLCLSGFMGMDIPPPSGPLWILGDVFIGRYYTVFDRDNNRVGFAEAARL

SEQ ID NO: 93 - protein, 341 aa, Mus musculus
MRAPGHAAIRRWLFWMPLVCSVAMEQLQRDPTLDYHWDLWKKTHEKEYKDKNEEEVRRLIWEKNLKFIMIHNLEYSMGMHTYQVGMNDMGDMTNEEILCRMGALRIPRQSPKTVTFRSYSNRTLPDTVDWREKGCVTEVKYQGSCGACWAFSAVGALEGQLKLKTGKLISLSAQNLVDCSNEEKYGNKGCGGGYMTEAFQYIIDNGGIEADASYPYKATDEKCHYNSKNRAATCSRYIQLPFGDEDALKEAVATKGPVSVGIDASHSSFFFYKSGVYDDPSCTGNVNHGVLVVGYGTLDGKDYWLVKNSWGLNFGDQGYIRMARNNKNHCGIASYCSYPEI

SEQ ID NO: 94 - protein, 340 aa, Mus musculus
MRAPGHAAIRWLFWMPLVCSVAMEQLQRDPTLDYHWDLWKKTHEKEYKDKNEEEVRRLIWEKNLKFIMIHNLEYSMGMHTYQVGMNDMGDMTNEEILCRMGALRIPRQSPKTVTFRSYSNRTLPDTVDWREKGCVTEVKYQGSCGACWAFSAVGALEGQLKLKTGKLISLSAQNLVDCSNEEKYGNKGCGGGYMTEAFQYIIDNGGIEADASYPYKATDEKCHYNSKNRAATCSRYIQLPFGDEDALKEAVATKGPVSVGIDASHSSFFFYKSGVYDDPSCTGNVNHGVLVVGYGTLDGKDYWLVKNSWGLNFGDQGYIRMARNNKNHCGIASYCSYPEI

SEQ ID NO: 95 - protein, 331 aa, Homo sapiens
MKRLVCVLLVCSSAVAQLHKDPTLDHHWHLWKKTYGKQYKEKNEEAVRRLIWEKNLKFVMLHNLEHSMGMHSYDLGMNHLGDMTSEEVMSLMSSLRVPSQWQRNITYKSNPNRILPDSVDWREKGCVTEVKYQGSCGACWAFSAVGALEAQLKLKTGKLVSLSAQNLVDCSTEKYGNKGCNGGFMTTAFQYIIDNKGIDSDASYPYKAMDQKCQYDSKYRAATCSKYTELPYGREDVLKEAVANKGPVSVGVDARHPSFFLYRSGVYYEPSCTQNVNHGVLVVGYGDLNGKEYWLVKNSWGHNFGEEGYIRMARNKGNHCGIASFPSYPEI

SEQ ID NO: 96 - protein, 281 aa, Homo sapiens
MKRLVCVLLVCSSAVAQLHKDPTLDHHWHLWKKTYGKQYKEKNEEAVRRLIWEKNLKFVMLHNLEHSMGMHSYDLGMNHLGDMGSCGACWAFSAVGALEAQLKLKTGKLVSLSAQNLVDCSTEKYGNKGCNGGFMTTAFQYIIDNKGIDSDASYPYKAMDQKCQYDSKYRAATCSKYTELPYGREDVLKEAVANKGPVSVGVDARHPSFFLYRSGVYYEPSCTQNVNHGVLVVGYGDLNGKEYWLVKNSWGHNFGEEGYIRMARNKGNHCGIASFPSYPEI

SEQ ID NO: 97 - protein, 189 aa, Mus musculus
MVTMLMFLATLAGLFTTAKGQNFHLGKCPSPPVQENFDVKKYLGRWYEIEKIPASFEKGNCIQANYSLMENGNIEVLNKELSPDGTMNQVKGEAKQSNVSEPAKLEVQFFPLMPPAPYWILATDYENYALVYSCTTFFWLFHVDFVWILGRNPYLPPETITYLKDILTSNGIDIEKMTTTDQANCPDFL

SEQ ID NO: 98 - protein, 189 aa, Mus musculus; identical to SEQ ID NO: 97

SEQ ID NO: 99 - protein, 189 aa, Mus musculus; identical to SEQ ID NO: 97

SEQ ID NO: 100 - protein, 189 aa, Homo sapiens
MVMLLLLLSALAGLFGAAEGQAFHLGKCPNPPVQENFDVNKYLGRWYEIEKIPTTFENGRCIQANYSLMENGKIKVLNQELRADGTVNQIEGEATPVNLTEPAKLEVKFSWFMPSAPYWILATDYENYALVYSCTCIIQLFHVDFAWILARNPNLPPETVDSLKNILTSNNIDVKKMTVTDQVNCPKLS

SEQ ID NO: 101 - protein, 301 aa, Mus musculus
MRAWIFFLLCLAGRALAAPQTEVAEEIVEEETVVEETGVPVGANPVQVEMGEFEDGAEETVEEVVADNPCQNHHCKHGKVCELDESNTPMCVCQDPTSCPAPIGEFEKVCSNDNKTFDSSCHFFATKCTLEGTKKGHKLHLDYIGPCKYIAPCLDSELTEFPLRMRDWLKNVLVTLYERDEGNNLLTEKQKLRVKKIHENEKRLEAGDHPVELLARDFEKNYNMYIFPVHWQFGQLDQHPIDGYLSHTELAPLRAPLIPMEHCTTRFFETCDLDNDKYIALEEWAGCFGIKEQDINKDLVI

SEQ ID NO: 102 - protein, 302 aa, Mus musculus
MRAWIFFLLCLAGRALAAPQQTEVAEEIVEEETVVEETGVPVGANPVQVEMGEFEDGAEETVEEVVADNPCQNHHCKHGKVCELDESNTPMCVCQDPTSCPAPIGEFEKVCSNDNKTFDSSCHFFATKCTLEGTKKGHKLHLDYIGPCKYIAPCLDSELTEFPLRMRDWLKNVLVTLYERDEGNNLLTEKQKLRVKKIHENEKRLEAGDHPVELLARDFEKNYNMYIFPVHWQFGQLDQHPIDGYLSHTELAPLRAPLIPMEHCTTRFFETCDLDNDKYIALEEWAGCFGIKEQDINKDLVI

SEQ ID NO: 103 - protein, 302 aa, Homo sapiens
MRAWIFFLLCLAGRALAAPQEALPDETEVVEETVAEVTEVSVGANPVQVEVGEFDDGAEETEEEVVAENPCQNHHCKHGKVCELDENNTPMCVCQDPTSCPAPIGEFEKVCSNDNKTFDSSCHFFATKCTLEGTKKGHKLHLDYIGPCKYIPPCLDSELTEFPLRMRDWLKNVLVTLYERDEDNNLLTEKQKLRVKKIHENEKRLEAGDHPVELLARDFEKNYNMYIFPVHWQFGQLDQHPIDGYLSHTELAPLRAPLIPMEHCTTRFFETCDLDNDKYIALDEWAGCFGIKQKDIDKDLVI

SEQ ID NO: 104 - protein, 341 aa, Homo sapiens
MRAWIFFLLCLAGRALAAPQQEALPDETEVVEETVAEVTEVSVGANPVQVEVGEFDDGAEETEEEVVAENPCQNHHCKHGKVCELDENNTPMCVCQDPTSCPAPIGEFEKVCSNDNKTFDSSCHFFATKCTLEGTKKGHKLHLDYIGPCKYIPPCLDSELTEFPLRMRDWLKNVLVTLYERDEDNNLLTEKQKLRVKKIHENEKRLEAGDHPVELLARDFEKNYNMYIFPVHWQFGQLDQHPIDGYLSHTELAPLRAPLIPMEHCTTRFFETCDLDNDKYIALDEWAGCFGIKQRYRQGSCDLNPLLPQYRILSLTLPFVFPPMFKMFGWFVVLPGDKVLT

SEQ ID NO: 105 - protein, 303 aa, Homo sapiens
MRAWIFFLLCLAGRALAAPQQEALPDETEVVEETVAEVTEVSVGANPVQVEVGEFDDGAEETEEEVVAENPCQNHHCKHGKVCELDENNTPMCVCQDPTSCPAPIGEFEKVCSNDNKTFDSSCHFFATKCTLEGTKKGHKLHLDYIGPCKYIPPCLDSELTEFPLRMRDWLKNVLVTLYERDEDNNLLTEKQKLRVKKIHENEKRLEAGDHPVELLARDFEKNYNMYIFPVHWQFGQLDQHPIDGYLSHTELAPLRAPLIPMEHCTTRFFETCDLDNDKYIALDEWAGCFGIKQKDIDKDLVI

SEQ ID NO: 106 - DNA, 2148 bp, Mus musculus
agatgcctcccagggagcccggaccccgacgcaggcagaccatgtgggtcctgatgagctggctggccttcgcggcagggctggtagccggaacacagtgtccagatgggcagttctgccctgttgcctgctgccttgaccagggaggagccaactacagctgctgtaaccctcttctggacacatggcctagaataacgagccatcatctagatggctcctgccagacccatggccactgtcctgctggctattcttgtcttctcactgtgtctgggacttccagctgctgcccgttctctaagggtgtgtcttgtggtgatggctaccactgctgcccccagggcttccactgtagtgcagatgggaaatcctgcttccagatgtcagataaccccttgggtgctgtccagtgtcctgggagccagtttgaatgtcctgactctgccacctgctgcattatggttgatggttcgtggggatgttgtcccatgccccaggcctcttgctgtgaagacagagtgcattgctgtccccatggggcctcctgtgacctggttcacacacgatgcgtttcacccacgggcacccacaccctactaaagaagttccctgcacaaaagaccaacagggcagtgtctttgcctttttctgtcgtgtgccctgatgctaagacccagtgtcccgatgattctacctgctgtgagctacccactgggaagtatggctgctgtccaatgcccaatgccatctgctgttccgaccacctgcactgctgcccccaggacactgtatgtgacctgatccagagtaagtgcctatccaagaactacaccacggatctcctgaccaagctgcctggatacccagtgaaggaggtgaagtgcgacatggaggtgagctgccctgaaggatatacctgctgccgcctcaacactggggcctggggctgctgtccatttgccaaggccgtgtgttgtgaggatcacattcattgctgcccggcagggtttcagtgtcacacagagaaaggaacctgcgaaatgggtatcctccaagtaccctggatgaagaaggtcatagcccccctccgcctgccagacccacagatcttgaagagtgatacaccttgtgatgacttcactaggtgtcctacaaacaatacctgctgcaaactcaattctggggactggggctgctgtcccatcccagaggctgtctgctgctcagacaaccagcattgctgccctcagggcttcacatgtctggctcaggggtactgtcagaagggagacacaatggtggctggcctggagaagatacctgcccgccagacaaccccgctccaaattggagatatcggttgtgaccagcataccagctgcccagtagggcaaacctgctgcccaagcctcaagggaagttgggcctgctgccagctgccccatgctgtgtgctgtgaggaccggcagcactgttgcccggccgggtacacctgcaatgtgaaggcgaggacctgtgagaaggatgtcgattttatccagcctcccgtgctcctgaccctcggccctaaggttgggaatgtggagtgtggagaagggcatttctgccatgataaccagacctgttgtaaagacagtgcaggagtctgggcctgctgtccctacctaaagggtgtctgctgtagagatggacgtcactgttgccccggtggcttccactgttcagccaggggaaccaagtgtttgcgaaagaagattcctcgctgggacatgtttttgagggatccggtcccaagaccgctactgtaaggaagggctacagacttaaggaactccacagtcctgggaaccctgttccgagggtacccactactcaggcctccctagcgcctcctcccctaacgtctccccggcctactcatcctgagtcaccctatcaccatgggaggtggagcctcaaactaaaaccttcttttatggaaagaaggctgtggccaaaagccccgtatcaaactgccatttcttccggtttctgtggaccttgtggccaggtgctcttcccgagccacaggtgttctgtgagcttgcttgtgtgtgtgtgcgcgtgtgcgtgtgttgctccaataaagtttgtacactttctgaa

SEQ ID NO: 107 - DNA, 2130 bp, Homo sapiens
gctgctgcccaaggaccgcggagtcggacgcaggcagaccatgtggaccctggtgagctgggtggccttaacagcagggctggtggctggaacgcggtgcccagatggtcagttctgccctgtggcctgctgcctggaccccggaggagccagctacagctgctgccgtccccttctggacaaatggcccacaacactgagcaggcatctgggtggcccctgccaggttgatgcccactgctctgccggccactcctgcatctttaccgtctcagggacttccagttgctgccccttcccagaggccgtggcatgcggggatggccatcactgctgcccacggggcttccactgcagtgcagacgggcgatcctgcttccaaagatcaggtaacaactccgtgggtgccatccagtgccctgatagtcagttcgaatgcccggacttctccacgtgctgtgttatggtcgatggctcctgggggtgctgccccatgccccaggcttcctgctgtgaagacagggtgcactgctgtccgcacggtgccttctgcgacctggttcacacccgctgcatcacacccacgggcacccaccccctggcaaagaagctccctgcccagaggactaacagggcagtggccttgtccagctcggtcatgtgtccggacgcacggtcccggtgccctgatggttctacctgctgtgagctgcccagtgggaagtatggctgctgcccaatgcccaacgccacctgctgctccgatcacctgcactgctgcccccaagacactgtgtgtgacctgatccagagtaagtgcctctccaaggagaacgctaccacggacctcctcactaagctgcctgcgcacacagtgggggatgtgaaatgtgacatggaggtgagctgcccagatggctatacctgctgccgtctacagtcgggggcctggggctgctgcccttttacccaggctgtgtgctgtgaggaccacatacactgctgtcccgcggggtttacgtgtgacacgcagaagggtacctgtgaacaggggccccaccaggtgccctggatggagaaggccccagctcacctcagcctgccagacccacaagccttgaagagagatgtcccctgtgataatgtcagcagctgtccctcctccgatacctgctgccaactcacgtctggggagtggggctgctgtccaatcccagaggctgtctgctgctcggaccaccagcactgctgcccccagggctacacgtgtgtagctgaggggcagtgtcagcgaggaagcgagatcgtggctggactggagaagatgcctgcccgccgggcttccttatcccaccccagagacatcggctgtgaccagcacaccagctgcccggtggggcagacctgctgcccgagcctgggtgggagctgggcctgctgccagttgccccatgctgtgtgctgcgaggatcgccagcactgctgcccggctggctacacctgcaacgtgaaggctcgatcctgcgagaaggaagtggtctctgcccagcctgccaccttcctggcccgtagccctcacgtgggtgtgaaggacgtggagtgtggggaaggacacttctgccatgataaccagacctgctgccgagacaaccgacagggctgggcctgctgtccctaccgccagggcgtctgttgtgctgatcggcgccactgctgtcctgctggcttccgctgcgcagccaggggtaccaagtgtttgcgcagggaggccccgcgctgggacgcccctttgagggacccagccttgagacagctgctgtgagggacagtactgaagactctgcagccctcgggaccccactcggagggtgccctctgctcaggcctccctagcacctccccctaaccaaattctccctggaccccattctgagctccccatcaccatgggaggtggggcctcaatctaaggccttccctgtcagaagggggttgtggcaaaagccacattacaagctgccatcccctccccgtttcagtggaccctgtggccaggtgcttttccctatccacaggggtgtttgtgtgtgtgcgcgtgtgcgtttcaataaagtttgtacactttcttaa

SEQ ID NO: 108 - DNA, 1934 bp, Mus musculus
gctctcttcgggccgccgcgaccatgaagactcccggcgtcttgctgctcattctcggcctcctggcttcgtcctccttcgcgattatcagaatccctctgcgcaagttcacatctatccgtcggactatgacggaggtgggcggctctgtggaagacctgatcctcaaaggccccatcaccaagtactccatgcagtcatcgcctaagaccacggagccagtgtcagagttactcaaaaactacctggatgcccagtactatggcgatatcggcatcggaaccccgccgcagtgtttcacagtcgtctttgatactggctcctctaacctgtgggtcccctccattcattgcaagatacttgacatagcctgctgggtccaccataagtacaacagtgacaagtccagcacctatgtgaagaacggcacgtcctttgacatccactacggctcaggaagcctctctgggtacctgagccaggacactgtatcggttccatgtaagtctgaccagtcaaaggcaagaggtatcaaggtggagaaacagatctttggagaagccaccaagcagcctggaatcgtatttgttgcagccaagtttgatggcatcttgggcatgggctaccctcatatctctgttaacaacgtgcttccggtctttgacaacctgatgcaacagaagctggtggacaagaacatcttctccttctacctgaacagggacccagaagggcaacccggaggagaactaatgcttggtggcactgactccaagtactaccacggggagctgtcctacctgaacgtcactcgaaaggcctactggcaggtgcacatggaccagttggaggtgggcaatgagctgaccctgtgcaagggaggctgtgaggctattgtggacacagggacatctcttctggtggggcctgtggaagaggtgaaggagctgcagaaggccatcggggcagtgcctcttatccagggtgagtatatgattccttgtgagaaggtgtccagcctgcccacggtctacctgaagctaggaggcaaaaactatgaactacacccagacaagtatatactcaaggtatcgcagggtggaaagacaatctgcctgagtggcttcatgggaatggacataccccctcccagtgggccgctctggatcctgggcgatgtcttcattggttcctactacactgtgtttgacagagacaacaatagggtcggctttgccaatgctgtcgtactctaacttgctccttctccactgtcagggaactggatcagagtccagtagaggaagccagccagccccatccctccacctgccccactcacacatagtcacactcgcttagtgttgctggacccttgggggagacctggctggagcttgtccagctgttctgttctgtggttcctcaccctgggttcagattgctgccctctgcctgtctgaaggaggccaaggcccacccagtacacgaggctgccttcaaaggcccctactggtttaatagctgctgagatggattgtcttgtcctgccgccctttgctgtgtgggcagtactctgaagcaggcaaatgggtcttaggatccctcccagaaacctgctctgacccagacccatcacccagcttggggatggcaccacgttctactgcccctccaactctggcctggcaaaggcctgaaggtgagcaggaaggagcaagaggacagaagcaaaactatgaacctggggggttacctagggcttgaccccgccctcctgggaaggcatgcctcagcctggggtagaggtaggatgactgactggttttggctggcctctgctgccctcatcctgggctaggcagctgggagccaaagttgaaatacaaataaagttgttttgggccttgatctctaaaaaaaaaaaaaaaaaa

SEQ ID NO: 109 - DNA, 2055 bp, Homo sapiens
aactgcggcgtcatcccggctataagcgcacggcctcggcgaccctctccgacccggccgccgccgccatgcagccctccagccttctgccgctcgccctctgcctgctggctgcacccgcctccgcgctcgtcaggatcccgctgcacaagttcacgtccatccgccggaccatgtcggaggttgggggctctgtggaggacctgattgccaaaggccccgtctcaaagtactcccaggcggtgccagccgtgaccgaggggcccattcccgaggtgctcaagaactacatggacgcccagtactacggggagattggcatcgggacgcccccccagtgcttcacagtcgtcttcgacacgggctcctccaacctgtgggtcccctccatccactgcaaactgctggacatcgcttgctggatccaccacaagtacaacagcgacaagtccagcacctacgtgaagaatggtacctcgtttgacatccactatggctcgggcagcctctccgggtacctgagccaggacactgtgtcggtgccctgccagtcagcgtcgtcagcctctgccctgggcggtgtcaaagtggagaggcaggtctttggggaggccaccaagcagccaggcatcaccttcatcgcagccaagttcgatggcatcctgggcatggcctacccccgcatctccgtcaacaacgtgctgcccgtcttcgacaacctgatgcagcagaagctggtggaccagaacatcttctccttctacctgagcagggacccagatgcgcagcctgggggtgagctgatgctgggtggcacagactccaagtattacaagggttctctgtcctacctgaatgtcacccgcaaggcctactggcaggtccacctggaccaggtggaggtggccagcgggctgaccctgtgcaaggagggctgtgaggccattgtggacacaggcacttccctcatggtgggcccggtggatgaggtgcgcgagctgcagaaggccatcggggccgtgccgctgattcagggcgagtacatgatcccctgtgagaaggtgtccaccctgcccgcgatcacactgaagctgggaggcaaaggctacaagctgtccccagaggactacacgctcaaggtgtcgcaggccgggaagaccctctgcctgagcggcttcatgggcatggacatcccgccacccagcgggccactctggatcctgggcgacgtcttcatcggccgctactacactgtgtttgaccgtgacaacaacagggtgggcttcgccgaggctgcccgcctctagttcccaaggcgtccgcgcgccagcacagaaacagaggagagtcccagagcaggaggcccctggcccagcggcccctcccacacacacccacacactcgcccgcccactgtcctgggcgccctggaagccggcggcccaagcccgacttgctgttttgttctgtggttttcccctccctgggttcagaaatgctgcctgcctgtctgtctctccatctgtttggtgggggtagagctgatccagagcacagatctgtttcgtgcattggaagaccccacccaagcttggcagccgagctcgtgtatcctggggctcccttcatctccagggagtcccctccccggccctaccagcgcccgctgggctgagcccctaccccacaccaggccgtcctcccgggccctcccttggaaacctgccctgcctgagggcccctctgcccagcttgggcccagctgggctctgccaccctacctgttcagtgtcccgggcccgttgaggatgaggccgctagaggcctgaggatgagctggaaggagtgagaggggacaaaacccaccttgttggagcctgcagggtggtgctgggactgagccagtcccaggggcatgtattggcctggaggtggggttgggattgggggctggtgccagccttcctctgcagctgacctctgttgtcctccccttgggcggctgagagccccagctgacatggaaatacagttgttggcctccggcctcccctc

SEQ ID NO: 110 - DNA, 1360 bp, Mus musculus
ttcctcattgtggatgcttcatgtgacaagctccgatttctttttagagtcatttcaagcagcctcctgctgccagggacatctttggagtgagcaccacacttcaggatgaccatgagggctcctggccacgctgccatcagaagatggctgttttggatgcccctggtgtgctctgtggcaatggagcaactgcagagagaccctaccctggactaccattgggatctctggaagaaaacccatgagaaagaatacaaggataagaatgaagaagaagtacggcgtctcatctgggaaaagaatctgaagtttataatgattcacaatctcgaatattctatgggaatgcatacctaccaagtgggcatgaacgatatgggagacatgaccaatgaagaaatcttgtgtcggatgggtgctctgagaattccccgacagtctccgaagactgtcactttcaggtcatactctaatcggacattgcctgacactgtggactggagagagaagggctgcgtcactgaggtgaaataccagggttcttgtggtgcctgctgggctttcagtgctgtgggggcccttgaagggcagctgaagctgaaaacggggaagctgatatccctcagtgctcagaacctggtggactgctcaaatgaagaaaagtatgggaataaaggctgtggaggcggctacatgaccgaagctttccagtacatcattgataatgggggcatagaggcagacgcttcctatccctacaaagccacggatgaaaagtgtcactataactcaaaaaatcgagctgccacgtgttcaaggtacattcagctcccgtttggtgacgaggatgccctgaaagaagcagtggccactaaagggcctgtctctgtgggcatcgacgccagccattcctccttcttcttctacaaaagcggtgtctatgacgacccctcctgtacgggcaatgtgaatcatggtgttcttgtggttggctatgggactcttgatggcaaagattactggcttgtgaaaaacagttggggccttaactttggtgatcaaggatacattcggatggcaagaaataataaaaatcactgcggaattgctagttattgctcttacccagaaatctaaaccatttcttctttttctaacaagtcacaaagatggaatatactctaacttaatttgcctgcaatatccagaggaaccaagtgtgtcgtgatcaatgtgtagttactgtactaactaggttatagctatttttacaccctgttgtctagtgttttctaataaccatttgtaacatgatagccccaaagtgcttaataaaatctgtcatttcaaatatcta

SEQ ID NO: 111 - DNA, 1357 bp, Mus musculus
ttcctcattgtggatgcttcatgtgacaagctccgatttctttttagagtcatttcaagcagcctcctgctgccagggacatctttggagtgagcaccacacttcaggatgaccatgagggctcctggccacgctgccataagatggctgttttggatgcccctggtgtgctctgtggcaatggagcaactgcagagagaccctaccctggactaccattgggatctctggaagaaaacccatgagaaagaatacaaggataagaatgaagaagaagtacggcgtctcatctgggaaaagaatctgaagtttataatgattcacaatctcgaatattctatgggaatgcatacctaccaagtgggcatgaacgatatgggagacatgaccaatgaagaaatcttgtgtcggatgggtgctctgagaattccccgacagtctccgaagactgtcactttcaggtcatactctaatcggacattgcctgacactgtggactggagagagaagggctgcgtcactgaggtgaaataccagggttcttgtggtgcctgctgggctttcagtgctgtgggggcccttgaagggcagctgaagctgaaaacggggaagctgatatccctcagtgctcagaacctggtggactgctcaaatgaagaaaagtatgggaataaaggctgtggaggcggctacatgaccgaagctttccagtacatcattgataatgggggcatagaggcagacgcttcctatccctacaaagccacggatgaaaagtgtcactataactcaaaaaatcgagctgccacgtgttcaaggtacattcagctcccgtttggtgacgaggatgccctgaaagaagcagtggccactaaagggcctgtctctgtgggcatcgacgccagccattcctccttcttcttctacaaaagcggtgtctatgacgacccctcctgtacgggcaatgtgaatcatggtgttcttgtggttggctatgggactcttgatggcaaagattactggcttgtgaaaaacagttggggccttaactttggtgatcaaggatacattcggatggcaagaaataataaaaatcactgcggaattgctagttattgctcttacccagaaatctaaaccatttcttctttttctaacaagtcacaaagatggaatatactctaacttaatttgcctgcaatatccagaggaaccaagtgtgtcgtgatcaatgtgtagttactgtactaactaggttatagctatttttacaccctgttgtctagtgttttctaataaccatttgtaacatgatagccccaaagtgcttaataaaatctgtcatttcaaatatcta

SEQ ID NO: 112 - DNA, 3936 bp, Homo sapiens
ctccttgttgctttgaaatcttagaagagagcccactaattcaaggactcttactgtgggagcaactgctggttctatcacaatgaaacggctggtttgtgtgctcttggtgtgctcctctgcagtggcacagttgcataaagatcctaccctggatcaccactggcatctctggaagaaaacctatggcaaacaatacaaggaaaagaatgaagaagcagtacgacgtctcatctgggaaaagaatctaaagtttgtgatgcttcacaacctggagcattcaatgggaatgcactcatacgatctgggcatgaaccacctgggagacatgaccagtgaagaagtgatgtctttgatgagttccctgagagttcccagccagtggcagagaaatatcacatataagtcaaaccctaatcggatattgcctgattctgtggactggagagagaaagggtgtgttactgaagtgaaatatcaaggttcttgtggtgcttgctgggctttcagtgctgtgggggccctggaagcacagctgaagctgaaaacaggaaagctggtgtctctcagtgcccagaacctggtggattgctcaactgaaaaatatggaaacaaaggctgcaatggtggcttcatgacaacggctttccagtacatcattgataacaagggcatcgactcagacgcttcctatccctacaaagccatggatcagaaatgtcaatatgactcaaaatatcgtgctgccacatgttcaaagtacactgaacttccttatggcagagaagatgtcctgaaagaagctgtggccaataaaggcccagtgtctgttggtgtagatgcgcgtcatccttctttcttcctctacagaagtggtgtctactatgaaccatcctgtactcagaatgtgaatcatggtgtacttgtggttggctatggtgatcttaatgggaaagaatactggcttgtgaaaaacagctggggccacaactttggtgaagaaggatatattcggatggcaagaaataaaggaaatcattgtgggattgctagctttccctcttacccagaaatctagaggatctctcctttttataacaaatcaagaaatatgaagcactttctcttaacttaatttttcctgctgtatccagaagaaataattgtgtcatgattaatgtgtatttactgtactaattagaaaatatagtttgaggccgggcacggtggctcacgcctgtaatcccagtacttgggaggccaaggcaggcatatcaacttgaggccaggagttaaagagcagcctggctaacatggtgaaaccccatctctactaaaaatacaaaaaattagccgagcacggtggtgcatgcctgtaatcccagctacttgggaggctgaggcacgagattccttgaacccaagaggttgaggctatgttgagctgagatcacaccactgtactccagcctggatgacagagtggagactctgtttcaaaaaaacagaaaagaaaatatagtttgattcttcatttttttaaatttgcaaatctcaggataaagtttgctaagtaaattagtaatgtactatagatataactgtacaaaaattgttcaacctaaaacaatctgtaattgcttattgttttattgtatactctttgtctttttaagacccctaatagccttttgtaacttgatggcttaaaaatacttaataaatctgccatttcaaatttctatcattgccacataccattcttattcctaggcaactattaataatctatcctgagaatattaattgtggtattctggtgatggggtttagcaactttgatggaagaaaatattaggctataaatgtcctaaggactcagattgtatctttgtacagaagaggattcaaaacgccacgtgtagtggctcatgcctgtaatcccaacactttgggaggctgaagtaggaggatcgtcttgagcccaggagttcaagaccagcctggacaacatagtgagaccttgtctccacaaaaataaaaaagaaactatccaggagtggtggtgtgtgcctgtggtccctgctatgcagatgtctaagacaggaggatcacaagagcccaggaggttgagaatgcagtgagcttgtaattgcaccactgcactccagcctgggtgacagagcaagaccctgtcttaaaaaaagaggattcaacacatatttttatattatgttaaagtaaagaaatgcataaaagacaagcactttggaagaattattttaatgatcaacaatttaatgtattagtccaaattatttttacgtagtcatcaacaatttgaccagggcctttatttggcaaataactgagccaaccagaataaaataaccaatactccactgctcatatttttatctaattcagatggatcttccttacaactgctctagattagtagatgcatctaagcaggcagcaggaactttaaattttttaagttcatgtctatgacatgaacaatgtgtgggataatgtcattaatatatcctaaattaacctaaacgtatttcactaactctggctccttctccataaagcacattttaaggaacaagaattgctaaatataaaaacataaataataccataatacatggctatcatcaaaagtgtatagaatattatagtttaaaagtatttagttgattacttttcagttttgttttgttttttgagacggagtctcactctgttgcccaggctggagtgcagtggcaccatctcagttcactgcaacttctgcctcccgagttcaagcgattctcctgcctcagcctcccgagtagctggaattataggcgtgcaccaccacgcccagctaatttttgtatttttagtaaagacagggttttgccacattagccaggctggtctcaaactcctgacctcaggtgatccacccaccccagcctcccaaagtgctaagattacaggcgtgagccactgagcccagcctacttttcagtttttaacataatttttgttttatccacaacttttcaagtattgaaagtagaataaaaacatgggttcttagtctttagctatctgttaaagcctatgaatgccttcttaaaatcatgtttttaaatgcataaaatatataggattacaaaggaatctaattatatcgaaatacagttattaaaatgttaaaagataagtttgttatatattaatatgcatgcttctttataaatgcattaaataagagttaatagctatcctaaatttgaaatagtgataagcataatgaaaatagatgcaaaaaactaatgtgatatgaaaatatctgggtttttcttttgatgatgaagtattgctaatattaccgtggtttatgaactatgttcagaattgaagaaaatcctaactttcagttagaggttagtgacggggttcaggacaccctacacaaaatacagcactttgacatattgaatattttaagctgaaggcatttgaggaaattgcagaagcaggaaggtgactctgaccttctgcctgctgttctccccagaagcagccataaaacctgggaaggattttctgaccttcccctgaagtagatcataagactgtcatgtaagaggtgctctcctggcacccagagaaaaggagcatccttacctccaaaagcacagggacacaaagaggaatctaaacaaacaggcctctcagtttcccccagtttattacatttagcttgttcacactttgccctatgacatttctacatcactggctgctcttcatcaaacctactataaaaaacattcaagttcaactgtttctttgggcctttatttccttatggagcccctcgtgtcgtgtaaaacttatattaaataaatgtgcatgcttttctcttgc

SEQ ID NO: 113 - DNA, 3786 bp, Homo sapiens
ctccttgttgctttgaaatcttagaagagagcccactaattcaaggactcttactgtgggagcaactgctggttctatcacaatgaaacggctggtttgtgtgctcttggtgtgctcctctgcagtggcacagttgcataaagatcctaccctggatcaccactggcatctctggaagaaaacctatggcaaacaatacaaggaaaagaatgaagaagcagtacgacgtctcatctgggaaaagaatctaaagtttgtgatgcttcacaacctggagcattcaatgggaatgcactcatacgatctgggcatgaaccacctgggagacatgggttcttgtggtgcttgctgggctttcagtgctgtgggggccctggaagcacagctgaagctgaaaacaggaaagctggtgtctctcagtgcccagaacctggtggattgctcaactgaaaaatatggaaacaaaggctgcaatggtggcttcatgacaacggctttccagtacatcattgataacaagggcatcgactcagacgcttcctatccctacaaagccatggatcagaaatgtcaatatgactcaaaatatcgtgctgccacatgttcaaagtacactgaacttccttatggcagagaagatgtcctgaaagaagctgtggccaataaaggcccagtgtctgttggtgtagatgcgcgtcatccttctttcttcctctacagaagtggtgtctactatgaaccatcctgtactcagaatgtgaatcatggtgtacttgtggttggctatggtgatcttaatgggaaagaatactggcttgtgaaaaacagctggggccacaactttggtgaagaaggatatattcggatggcaagaaataaaggaaatcattgtgggattgctagctttccctcttacccagaaatctagaggatctctcctttttataacaaatcaagaaatatgaagcactttctcttaacttaatttttcctgctgtatccagaagaaataattgtgtcatgattaatgtgtatttactgtactaattagaaaatatagtttgaggccgggcacggtggctcacgcctgtaatcccagtacttgggaggccaaggcaggcatatcaacttgaggccaggagttaaagagcagcctggctaacatggtgaaaccccatctctactaaaaatacaaaaaattagccgagcacggtggtgcatgcctgtaatcccagctacttgggaggctgaggcacgagattccttgaacccaagaggttgaggctatgttgagctgagatcacaccactgtactccagcctggatgacagagtggagactctgtttcaaaaaaacagaaaagaaaatatagtttgattcttcatttttttaaatttgcaaatctcaggataaagtttgctaagtaaattagtaatgtactatagatataactgtacaaaaattgttcaacctaaaacaatctgtaattgcttattgttttattgtatactctttgtctttttaagacccctaatagccttttgtaacttgatggcttaaaaatacttaataaatctgccatttcaaatttctatcattgccacataccattcttattcctaggcaactattaataatctatcctgagaatattaattgtggtattctggtgatggggtttagcaactttgatggaagaaaatattaggctataaatgtcctaaggactcagattgtatctttgtacagaagaggattcaaaacgccacgtgtagtggctcatgcctgtaatcccaacactttgggaggctgaagtaggaggatcgtcttgagcccaggagttcaagaccagcctggacaacatagtgagaccttgtctccacaaaaataaaaaagaaactatccaggagtggtggtgtgtgcctgtggtccctgctatgcagatgtctaagacaggaggatcacaagagcccaggaggttgagaatgcagtgagcttgtaattgcaccactgcactccagcctgggtgacagagcaagaccctgtcttaaaaaaagaggattcaacacatatttttatattatgttaaagtaaagaaatgcataaaagacaagcactttggaagaattattttaatgatcaacaatttaatgtattagtccaaattatttttacgtagtcatcaacaatttgaccagggcctttatttggcaaataactgagccaaccagaataaaataaccaatactccactgctcatatttttatctaattcagatggatcttccttacaactgctctagattagtagatgcatctaagcaggcagcaggaactttaaattttttaagttcatgtctatgacatgaacaatgtgtgggataatgtcattaatatatcctaaattaacctaaacgtatttcactaactctggctccttctccataaagcacattttaaggaacaagaattgctaaatataaaaacataaataataccataatacatggctatcatcaaaagtgtatagaatattatagtttaaaagtatttagttgattacttttcagttttgttttgttttttgagacggagtctcactctgttgcccaggctggagtgcagtggcaccatctcagttcactgcaacttctgcctcccgagttcaagcgattctcctgcctcagcctcccgagtagctggaattataggcgtgcaccaccacgcccagctaatttttgtatttttagtaaagacagggttttgccacattagccaggctggtctcaaactcctgacctcaggtgatccacccaccccagcctcccaaagtgctaagattacaggcgtgagccactgagcccagcctacttttcagtttttaacataatttttgttttatccacaacttttcaagtattgaaagtagaataaaaacatgggttcttagtctttagctatctgttaaagcctatgaatgccttcttaaaatcatgtttttaaatgcataaaatatataggattacaaaggaatctaattatatcgaaatacagttattaaaatgttaaaagataagtttgttatatattaatatgcatgcttctttataaatgcattaaataagagttaatagctatcctaaatttgaaatagtgataagcataatgaaaatagatgcaaaaaactaatgtgatatgaaaatatctgggtttttcttttgatgatgaagtattgctaatattaccgtggtttatgaactatgttcagaattgaagaaaatcctaactttcagttagaggttagtgacggggttcaggacaccctacacaaaatacagcactttgacatattgaatattttaagctgaaggcatttgaggaaattgcagaagcaggaaggtgactctgaccttctgcctgctgttctccccagaagcagccataaaacctgggaaggattttctgaccttcccctgaagtagatcataagactgtcatgtaagaggtgctctcctggcacccagagaaaaggagcatccttacctccaaaagcacagggacacaaagaggaatctaaacaaacaggcctctcagtttcccccagtttattacatttagcttgttcacactttgccctatgacatttctacatcactggctgctcttcatcaaacctactataaaaaacattcaagttcaactgtttctttgggcctttatttccttatggagcccctcgtgtcgtgtaaaacttatattaaataaatgtgcatgcttttctcttgc

SEQ ID NO: 114 - DNA, 2070 bp, Mus musculus
acaaacaatatctcattgtttcttcctcagggagcagctgtgaaggaaactaagtgaggggacagacacagcatcccatctttgtgccccacacagagctcagctttgaggccagtttcccccaagctgtggtgggtgtggcatgcctgactatcaaagggcaagggcctgatgggagcctataaagtgacttgggagaagccacacacctcacttggaggattctgggtggaaacttcagtcatctgatctgagagaaactgacagtgagcaccaactgaaggcttttacaggctccatctcattttcctcagacttctaaggcctctcctgcagccaccccaccccaagatggtgaccatgctgatgttcctggccacgctggcgggtctcttcaccacagccaaaggacaaaatttccatcttgggaaatgcccgtctcctcctgtgcaagagaattttgacgtgaaaaagtatcttggaagatggtacgaaattgagaagatcccagcgagctttgagaaaggaaactgcattcaagccaactactcgctgatggagaacggaaacatcgaagtgctaaacaaggagctgagtcctgatggaaccatgaaccaagtaaagggtgaagccaaacagagcaacgtctcagagccagccaagctggaagtccagttcttcccgttgatgccaccggcaccctactggatcctggccaccgattatgaaaactatgccctcgtgtactcctgcaccaccttcttctggctcttccatgtggattttgtttggattcttggaagaaatccttatctccctccagaaacaataacctacctaaaagatatccttacttctaatggcatcgacatcgaaaaaatgacaacaacagatcaagcgaactgcccggacttcctgtaaagggggcggggggggaaaaccacaccaggttatttctttgctttgcgttccctggctccaccccccacgcctcttaagtaccaagcaaccatggcaggcactagagggagagtaaggctatagaagccaatggagggaggggactcatggaaagttggcccaaacccaacctgaccccacactgtcaccttgctagcccaataataaacattttgctgatcagctgtgtttcctgtggattctgagctaggtttatagtgcaagagtcatggtcggcagatggttggaaaccctttggctgtagtttaaaggtagagaaagctgatggccaagttagatcctggtgactcggatccagggtccctctccacggcagatgctctggagggaattctgggacgtttttcacttctgtctggaggcttccttgaagcttttactttctcatcgggaagtcttcggaacagggccgaagcatgagcatcctgaaaatatctgggaaaagcagacagcctgtgaggaaaagacaaaggttgtttgtttggttggtttgttttgttttttcgacatagggtttctctgtatagccctggctgtcaggggactcactttgtagaccatgctggcctcgaactcagaaacccgtctgcctctgcctcccgagtgctgggattaaaggcgtgcgccaccatgcctggcttcaacggtgtttgtttgtttgtttgtttgtttgtttaatgatgcaaattttctctttcactcagaatttactgaggtccaattgcattccagtcagtgaaaaaaaaaatttagaatccctgaccaccgctctccttgcccccaagcgtcaactcagtccagtgatagaaataagacagagcaacatagagggcatcacgggaaatcagagaacatcccaccctcttcaagacacaggctcaagttatccagtatccagtctgtcttcaagccttggcactcccatgcctctgctccagtagcaagccagaaaccacctggtgttgttcttttctgatcttgtgacttttaaaaccaaaaacccagatttatcaccccacaagttcacttagttcctgttgtatagtctgttgtatgcttttcatttaattaaaaaaaaaaaaaaaactc

SEQ ID NO: 115 - DNA, 2004 bp, Mus musculus
acaaacaatatctcattgtttcttcctcagggagcagctgtgaaggaaactaagtgaggggacagacacagcatcccatctttgtgccccacacagagctcagctttgaggccagtttcccccaagctgtggtgggtgtggcatgcctgactatcaaagggcaagggcctgatgggagcctataaagtgacttgggagaagccacacacctcacttggaggattctgggtggaaacttcagtcatctgatctgagaggcctctcctgcagccaccccaccccaagatggtgaccatgctgatgttcctggccacgctggcgggtctcttcaccacagccaaaggacaaaatttccatcttgggaaatgcccgtctcctcctgtgcaagagaattttgacgtgaaaaagtatcttggaagatggtacgaaattgagaagatcccagcgagctttgagaaaggaaactgcattcaagccaactactcgctgatggagaacggaaacatcgaagtgctaaacaaggagctgagtcctgatggaaccatgaaccaagtaaagggtgaagccaaacagagcaacgtctcagagccagccaagctggaagtccagttcttcccgttgatgccaccggcaccctactggatcctggccaccgattatgaaaactatgccctcgtgtactcctgcaccaccttcttctggctcttccatgtggattttgtttggattcttggaagaaatccttatctccctccagaaacaataacctacctaaaagatatccttacttctaatggcatcgacatcgaaaaaatgacaacaacagatcaagcgaactgcccggacttcctgtaaagggggcggggggggaaaaccacaccaggttatttctttgctttgcgttccctggctccaccccccacgcctcttaagtaccaagcaaccatggcaggcactagagggagagtaaggctatagaagccaatggagggaggggactcatggaaagttggcccaaacccaacctgaccccacactgtcaccttgctagcccaataataaacattttgctgatcagctgtgtttcctgtggattctgagctaggtttatagtgcaagagtcatggtcggcagatggttggaaaccctttggctgtagtttaaaggtagagaaagctgatggccaagttagatcctggtgactcggatccagggtccctctccacggcagatgctctggagggaattctgggacgtttttcacttctgtctggaggcttccttgaagcttttactttctcatcgggaagtcttcggaacagggccgaagcatgagcatcctgaaaatatctgggaaaagcagacagcctgtgaggaaaagacaaaggttgtttgtttggttggtttgttttgttttttcgacatagggtttctctgtatagccctggctgtcaggggactcactttgtagaccatgctggcctcgaactcagaaacccgtctgcctctgcctcccgagtgctgggattaaaggcgtgcgccaccatgcctggcttcaacggtgtttgtttgtttgtttgtttgtttgtttaatgatgcaaattttctctttcactcagaatttactgaggtccaattgcattccagtcagtgaaaaaaaaaatttagaatccctgaccaccgctctccttgcccccaagcgtcaactcagtccagtgatagaaataagacagagcaacatagagggcatcacgggaaatcagagaacatcccaccctcttcaagacacaggctcaagttatccagtatccagtctgtcttcaagccttggcactcccatgcctctgctccagtagcaagccagaaaccacctggtgttgttcttttctgatcttgtgacttttaaaaccaaaaacccagatttatcaccccacaagttcacttagttcctgttgtatagtctgttgtatgcttttcatttaattaaaaaaaaaaaaaaaactc

SEQ ID NO: 116 - DNA, 2074 bp, Mus musculus
acaaacaatatctcattgtttcttcctcagggagcagctgtgaaggaaactaagtgaggggacagacacagcatcccatctttgtgccccacacagagctcagctttgaggccagtttcccccaagctgtggtgggtgtggcatgcctgactatcaaagggcaagggcctgatgggagcctataaagtgacttgggagaagccacacacctcacttggaggattctgggtggaaacttcagtcatctgatctgagagttagaaactgacagtgagcaccaactgaaggcttttacaggctccatctcattttcctcagacttctaaggcctctcctgcagccaccccaccccaagatggtgaccatgctgatgttcctggccacgctggcgggtctcttcaccacagccaaaggacaaaatttccatcttgggaaatgcccgtctcctcctgtgcaagagaattttgacgtgaaaaagtatcttggaagatggtacgaaattgagaagatcccagcgagctttgagaaaggaaactgcattcaagccaactactcgctgatggagaacggaaacatcgaagtgctaaacaaggagctgagtcctgatggaaccatgaaccaagtaaagggtgaagccaaacagagcaacgtctcagagccagccaagctggaagtccagttcttcccgttgatgccaccggcaccctactggatcctggccaccgattatgaaaactatgccctcgtgtactcctgcaccaccttcttctggctcttccatgtggattttgtttggattcttggaagaaatccttatctccctccagaaacaataacctacctaaaagatatccttacttctaatggcatcgacatcgaaaaaatgacaacaacagatcaagcgaactgcccggacttcctgtaaagggggcggggggggaaaaccacaccaggttatttctttgctttgcgttccctggctccaccccccacgcctcttaagtaccaagcaaccatggcaggcactagagggagagtaaggctatagaagccaatggagggaggggactcatggaaagttggcccaaacccaacctgaccccacactgtcaccttgctagcccaataataaacattttgctgatcagctgtgtttcctgtggattctgagctaggtttatagtgcaagagtcatggtcggcagatggttggaaaccctttggctgtagtttaaaggtagagaaagctgatggccaagttagatcctggtgactcggatccagggtccctctccacggcagatgctctggagggaattctgggacgtttttcacttctgtctggaggcttccttgaagcttttactttctcatcgggaagtcttcggaacagggccgaagcatgagcatcctgaaaatatctgggaaaagcagacagcctgtgaggaaaagacaaaggttgtttgtttggttggtttgttttgttttttcgacatagggtttctctgtatagccctggctgtcaggggactcactttgtagaccatgctggcctcgaactcagaaacccgtctgcctctgcctcccgagtgctgggattaaaggcgtgcgccaccatgcctggcttcaacggtgtttgtttgtttgtttgtttgtttgtttaatgatgcaaattttctctttcactcagaatttactgaggtccaattgcattccagtcagtgaaaaaaaaaatttagaatccctgaccaccgctctccttgcccccaagcgtcaactcagtccagtgatagaaataagacagagcaacatagagggcatcacgggaaatcagagaacatcccaccctcttcaagacacaggctcaagttatccagtatccagtctgtcttcaagccttggcactcccatgcctctgctccagtagcaagccagaaaccacctggtgttgttcttttctgatcttgtgacttttaaaaccaaaaacccagatttatcaccccacaagttcacttagttcctgttgtatagtctgttgtatgcttttcatttaattaaaaaaaaaaaaaaaactc

SEQ ID NO: 117 - DNA, 862 bp, Homo sapiens
aagacaggcatctcaaatcggctgattctgcatctggaaactgccttcatcttgaaagaaaagctccaggtcccttctccagccacccagccccaagatggtgatgctgctgctgctgctttccgcactggctggcctcttcggtgcggcagagggacaagcatttcatcttgggaagtgccccaatcctccggtgcaggagaattttgacgtgaataagtatctcggaagatggtacgaaattgagaagatcccaacaacctttgagaatggacgctgcatccaggccaactactcactaatggaaaacggaaagatcaaagtgttaaaccaggagttgagagctgatggaactgtgaatcaaatcgaaggtgaagccaccccagttaacctcacagagcctgccaagctggaagttaagttttcctggtttatgccatcggcaccgtactggatcctggccaccgactatgagaactatgccctcgtgtattcctgtacctgcatcatccaactttttcacgtggattttgcttggatcttggcaagaaaccctaatctccctccagaaacagtggactctctaaaaaatatcctgacttctaataacattgatgtcaagaaaatgacggtcacagaccaggtgaactgccccaagctctcgtaaccaggttctacagggaggctgcacccactccatgttacttctgcttcgctttcccctaccccccccccataaagacaaaccaatcaaccacgacaaaggaagttgacctgaacatgtaaccatgccctaccctgttaccttgctagctgcaaaataaacttgttgctgacctgctgtgctcgcagtagattccaa

SEQ ID NO: 118 - DNA, 2638 bp, Mus musculus
aggtggggccagggtgtctgggtagcacacagcctaccacaaggcaaggaagggagaaagaaaagacagctttggttctggggagaagggggaggcaggccaggggaaggaggagacagaggaggaggagggcctttgagtggaggcggagggtgagacagaccctgcccagagctccaagaggcttcctgctgctcgcctctaaacccctccacattcctgcagcccttcagaccgccagaactcttctgccgcctgcctgcctgcctgcctgcctgcctgcctgtgccgagagttcccagcatcatgagggcctggatcttctttctcctttgcctggccgggagggccctggcagcccctcagactgaagttgctgaggagatagtggaggaggaaaccgtggtggaggagacaggggtacctgtgggtgccaacccagtccaggtggaaatgggagaatttgaggacggtgcagaggaaacggtcgaggaggtggtggctgacaacccctgccagaaccatcattgcaaacatggcaaggtgtgtgagctggacgagagcaacacccccatgtgtgtgtgccaggaccccaccagctgccctgctcccattggcgagtttgagaaggtatgcagcaatgacaacaagaccttcgactcttcctgccacttctttgccaccaagtgcaccctggagggcaccaagaagggccacaagctccacctggactacatcggaccatgcaaatacatcgccccctgcctggattccgagctgactgaattccctctgcgcatgcgtgactggctcaaaaatgtcctggtcaccttgtacgagagagatgagggcaacaacctcctcactgagaagcagaagctgcgtgtgaagaagatccatgagaatgagaagcgcctggaggctggagaccaccccgtggagctgttggcccgagactttgagaagaactacaatatgtacatcttccctgtccactggcagtttggccagctggatcagcaccctattgatgggtacctgtcccacactgagctggccccactgcgcgctcccctcatccccatggaacattgcaccacacgtttctttgagacctgtgacctagacaacgacaagtacattgccctggaggaatgggccggctgctttggcatcaaggagcaggacatcaacaaggatctggtgatctaagttcacgcctcctgctgcagtcctgaactctctccctctgatgtgtcccccctcccattacccccttgtttaaaatgtttggatggttggctgttccgcctggggataaggtgctaacatagatttaactgaatacattaacggtgctaaaaaaaaaaaaaaaacaaagtaagaaagaaactagaacccaagtcacagcattttcccacataactctgaggccatggcccatccacagcctcctggtcccctgcactacccagtgtctcactggctgtgttggaaacggagttgcataagctcaccgtccacaagcacgaggagatatctctagctttcatttctgttttgcatttgactcttaacactcacccagactctgtgcttatttcattttgggggatgtgggctttttcccctggtggtttggagttaggcagagggaagttacagacacaggtacaaaatttgggtaaagatgctgtgagacctgaggacccaccagtcagaacccacatggcaagtcttagtagcctaggtcaaggaaagacagaataatccagagctgtggcacacatgacagactcccagcagcccgggaccttgctgtcttctcgactcttagggcgtttctttccatgtttggctgttggttttagttttggtgagccatgggtgggccagaacatcactcaactgcaattgggctttcaggttcttgccgggagctctaggcactgggaggctgtttcaggaaagtgagactcaagaggaagacagaaaaggttgtaacgtagaggaagtgagactggtgaattggtttgatttttttcacatctagatggctgtcataaagtttctagcatgttccccctcacctctccccaccccctgccacttgaaaccttctactaatcaagagaaacttccaagccaacggaatggtcagatctcacaggctgagaaattgttcccctccaagcatttcatgaaaaagctgcttctcattaaccatgcaaactctcacagcaatgtgaagagcttgacaagtctttcaaaataaaaagtaacaacttagaaacggctgtcctgtcccgggtgatggtatgtgtgtcttactctccggtgcttcgttttcaggtgtgcacaaacatggccatacttgtgcacagaagcaaacactccattgtgcttttatacacacacacatattcacacactcagacagggaagatatggctcctgtgagcactaatttaacacatgaagaagccagttcctgggctgggatgtagctcagttgataaagtgcttacccaatatgaacaaagcccaggttcgatcgtcagcgcaacctaagctggctgtggcagtgaatgtttgaaatcccagccccaaggaggtagaggcaggacagtcaaatgtc

SEQ ID NO: 119 - DNA, 2641 bp, Mus musculus
aggtggggccagggtgtctgggtagcacacagcctaccacaaggcaaggaagggagaaagaaaagacagctttggttctggggagaagggggaggcaggccaggggaaggaggagacagaggaggaggagggcctttgagtggaggcggagggtgagacagaccctgcccagagctccaagaggcttcctgctgctcgcctctaaacccctccacattcctgcagcccttcagaccgccagaactcttctgccgcctgcctgcctgcctgcctgcctgcctgcctgtgccgagagttcccagcatcatgagggcctggatcttctttctcctttgcctggccgggagggccctggcagcccctcagcagactgaagttgctgaggagatagtggaggaggaaaccgtggtggaggagacaggggtacctgtgggtgccaacccagtccaggtggaaatgggagaatttgaggacggtgcagaggaaacggtcgaggaggtggtggctgacaacccctgccagaaccatcattgcaaacatggcaaggtgtgtgagctggacgagagcaacacccccatgtgtgtgtgccaggaccccaccagctgccctgctcccattggcgagtttgagaaggtatgcagcaatgacaacaagaccttcgactcttcctgccacttctttgccaccaagtgcaccctggagggcaccaagaagggccacaagctccacctggactacatcggaccatgcaaatacatcgccccctgcctggattccgagctgactgaattccctctgcgcatgcgtgactggctcaaaaatgtcctggtcaccttgtacgagagagatgagggcaacaacctcctcactgagaagcagaagctgcgtgtgaagaagatccatgagaatgagaagcgcctggaggctggagaccaccccgtggagctgttggcccgagactttgagaagaactacaatatgtacatcttccctgtccactggcagtttggccagctggatcagcaccctattgatgggtacctgtcccacactgagctggccccactgcgcgctcccctcatccccatggaacattgcaccacacgtttctttgagacctgtgacctagacaacgacaagtacattgccctggaggaatgggccggctgctttggcatcaaggagcaggacatcaacaaggatctggtgatctaagttcacgcctcctgctgcagtcctgaactctctccctctgatgtgtcccccctcccattacccccttgtttaaaatgtttggatggttggctgttccgcctggggataaggtgctaacatagatttaactgaatacattaacggtgctaaaaaaaaaaaaaaaacaaagtaagaaagaaactagaacccaagtcacagcattttcccacataactctgaggccatggcccatccacagcctcctggtcccctgcactacccagtgtctcactggctgtgttggaaacggagttgcataagctcaccgtccacaagcacgaggagatatctctagctttcatttctgttttgcatttgactcttaacactcacccagactctgtgcttatttcattttgggggatgtgggctttttcccctggtggtttggagttaggcagagggaagttacagacacaggtacaaaatttgggtaaagatgctgtgagacctgaggacccaccagtcagaacccacatggcaagtcttagtagcctaggtcaaggaaagacagaataatccagagctgtggcacacatgacagactcccagcagcccgggaccttgctgtcttctcgactcttagggcgtttctttccatgtttggctgttggttttagttttggtgagccatgggtgggccagaacatcactcaactgcaattgggctttcaggttcttgccgggagctctaggcactgggaggctgtttcaggaaagtgagactcaagaggaagacagaaaaggttgtaacgtagaggaagtgagactggtgaattggtttgatttttttcacatctagatggctgtcataaagtttctagcatgttccccctcacctctccccaccccctgccacttgaaaccttctactaatcaagagaaacttccaagccaacggaatggtcagatctcacaggctgagaaattgttcccctccaagcatttcatgaaaaagctgcttctcattaaccatgcaaactctcacagcaatgtgaagagcttgacaagtctttcaaaataaaaagtaacaacttagaaacggctgtcctgtcccgggtgatggtatgtgtgtcttactctccggtgcttcgttttcaggtgtgcacaaacatggccatacttgtgcacagaagcaaacactccattgtgcttttatacacacacacatattcacacactcagacagggaagatatggctcctgtgagcactaatttaacacatgaagaagccagttcctgggctgggatgtagctcagttgataaagtgcttacccaatatgaacaaagcccaggttcgatcgtcagcgcaacctaagctggctgtggcagtgaatgtttgaaatcccagccccaaggaggtagaggcaggacagtcaaatgtc

SEQ ID NO: 120 - DNA, 3448 bp, Homo sapiens
agactgcccggagagcgcgctctgcctgccgcctgcctgcctgccactgagggttcccagcaccatgagggcctggatcttctttctcctttgcctggccgggagggccttggcagcccctcaagaagccctgcctgatgagacagaggtggtggaagaaactgtggcagaggtgactgaggtatctgtgggagctaatcctgtccaggtggaagtaggagaatttgatgatggtgcagaggaaaccgaagaggaggtggtggcggaaaatccctgccagaaccaccactgcaaacacggcaaggtgtgcgagctggatgagaacaacacccccatgtgcgtgtgccaggaccccaccagctgcccagcccccattggcgagtttgagaaggtgtgcagcaatgacaacaagaccttcgactcttcctgccacttctttgccacaaagtgcaccctggagggcaccaagaagggccacaagctccacctggactacatcgggccttgcaaatacatccccccttgcctggactctgagctgaccgaattccccctgcgcatgcgggactggctcaagaacgtcctggtcaccctgtatgagagggatgaggacaacaaccttctgactgagaagcagaagctgcgggtgaagaagatccatgagaatgagaagcgcctggaggcaggagaccaccccgtggagctgctggcccgggacttcgagaagaactataacatgtacatcttccctgtacactggcagttcggccagctggaccagcaccccattgacgggtacctctcccacaccgagctggctccactgcgtgctcccctcatccccatggagcattgcaccacccgctttttcgagacctgtgacctggacaatgacaagtacatcgccctggatgagtgggccggctgcttcggcatcaagcagaaggatatcgacaaggatcttgtgatctaaatccactccttccacagtaccggattctctctttaaccctccccttcgtgtttcccccaatgtttaaaatgtttggatggtttgttgttctgcctggagacaaggtgctaacatagatttaagtgaatacattaacggtgctaaaaatgaaaattctaacccaagacatgacattcttagctgtaacttaactattaaggccttttccacacgcattaatagtcccatttttctcttgccatttgtagctttgcccattgtcttattggcacatgggtggacacggatctgctgggctctgccttaaacacacattgcagcttcaacttttctctttagtgttctgtttgaaactaatacttaccgagtcagactttgtgttcatttcatttcagggtcttggctgcctgtgggcttccccaggtggcctggaggtgggcaaagggaagtaacagacacacgatgttgtcaaggatggttttgggactagaggctcagtggtgggagagatccctgcagaacccaccaaccagaacgtggtttgcctgaggctgtaactgagagaaagattctggggctgtgttatgaaaatatagacattctcacataagcccagttcatcaccatttcctcctttacctttcagtgcagtttcttttcacattaggctgttggttcaaacttttgggagcacggactgtcagttctctgggaagtggtcagcgcatcctgcagggcttctcctcctctgtcttttggagaaccagggctcttctcaggggctctagggactgccaggctgtttcagccaggaaggccaaaatcaagagtgagatgtagaaagttgtaaaatagaaaaagtggagttggtgaatcggttgttctttcctcacatttggatgattgtcataaggtttttagcatgttcctccttttcttcaccctccccttttttcttctattaatcaagagaaacttcaaagttaatgggatggtcggatctcacaggctgagaactcgttcacctccaagcatttcatgaaaaagctgcttcttattaatcatacaaactctcaccatgatgtgaagagtttcacaaatccttcaaaataaaaagtaatgacttagaaactgccttcctgggtgatttgcatgtgtcttagtcttagtcaccttattatcctgacacaaaaacacatgagcatacatgtctacacatgactacacaaatgcaaacctttgcaaacacattatgcttttgcacacacacacctgtacacacacaccggcatgtttatacacagggagtgtatggttcctgtaagcactaagttagctgttttcatttaatgacctgtggtttaacccttttgatcactaccaccattatcagcaccagactgagcagctatatccttttattaatcatggtcattcattcattcattcattcacaaaatatttatgatgtatttactctgcaccaggtcccatgccaagcactggggacacagttatggcaaagtagacaaagcatttgttcatttggagcttagagtccaggaggaatacattagataatgacacaatcaaatataaattgcaagatgtcacaggtgtgatgaagggagagtaggagagaccatgagtatgtgtaacaggaggacacagcattattctagtgctgtactgttccgtacggcagccactacccacatgtaactttttaagatttaaatttaaattagttaacattcaaaacgcagctccccaatcacactagcaacatttcaagtgcttgagagccatgcatgattagtggttaccctattgaataggtcagaagtagaatcttttcatcatcacagaaagttctattggacagtgctcttctagatcatcataagactacagagcacttttcaaagctcatgcatgttcatcatgttagtgtcgtattttgagctggggttttgagactccccttagagatagagaaacagacccaagaaatgtgctcaattgcaatgggccacatacctagatctccagatgtcatttcccctctcttattttaagttatgttaagattactaaaacaataaaagctcctaaaaaatcaaactgtattctggtgttctcttctacacagtgggagggcgagcagtaggagagattggcccatttggtgctggccatttgaggaatgcaagcccagcactagtctcataatctctaggaatctgtagagagaggaattgaagtaaatttcagcattggctcattcagtcattcggcgacattcatcaggtacctgcaatgtgttaggggatcttatgagtaggcagcgtgcgtgatccttgctcccctggagctttctaacattctagcaggcagaccacacataaatttgcaatactgtttctgataaaaacgtgctgtaaaggaaataaagcagagaactatcatggaaaa

SEQ ID NO: 121 - DNA, 3449 bp, Homo sapiens
agactgcccggagagcgcgctctgcctgccgcctgcctgcctgccactgagggttcccagcaccatgagggcctggatcttctttctcctttgcctggccgggagggccttggcagcccctcagcaagaagccctgcctgatgagacagaggtggtggaagaaactgtggcagaggtgactgaggtatctgtgggagctaatcctgtccaggtggaagtaggagaatttgatgatggtgcagaggaaaccgaagaggaggtggtggcggaaaatccctgccagaaccaccactgcaaacacggcaaggtgtgcgagctggatgagaacaacacccccatgtgcgtgtgccaggaccccaccagctgcccagcccccattggcgagtttgagaaggtgtgcagcaatgacaacaagaccttcgactcttcctgccacttctttgccacaaagtgcaccctggagggcaccaagaagggccacaagctccacctggactacatcgggccttgcaaatacatccccccttgcctggactctgagctgaccgaattccccctgcgcatgcgggactggctcaagaacgtcctggtcaccctgtatgagagggatgaggacaacaaccttctgactgagaagcagaagctgcgggtgaagaagatccatgagaatgagaagcgcctggaggcaggagaccaccccgtggagctgctggcccgggacttcgagaagaactataacatgtacatcttccctgtacactggcagttcggccagctggaccagcaccccattgacgggtacctctcccacaccgagctggctccactgcgtgctcccctcatccccatggagcattgcaccacccgctttttcgagacctgtgacctggacaatgacaagtacatcgccctggatgagtgggccggctgcttcggcatcaagcagagatatcgacaaggatcttgtgatctaaatccactccttccacagtaccggattctctctttaaccctccccttcgtgtttcccccaatgtttaaaatgtttggatggtttgttgttctgcctggagacaaggtgctaacatagatttaagtgaatacattaacggtgctaaaaatgaaaattctaacccaagacatgacattcttagctgtaacttaactattaaggccttttccacacgcattaatagtcccatttttctcttgccatttgtagctttgcccattgtcttattggcacatgggtggacacggatctgctgggctctgccttaaacacacattgcagcttcaacttttctctttagtgttctgtttgaaactaatacttaccgagtcagactttgtgttcatttcatttcagggtcttggctgcctgtgggcttccccaggtggcctggaggtgggcaaagggaagtaacagacacacgatgttgtcaaggatggttttgggactagaggctcagtggtgggagagatccctgcagaacccaccaaccagaacgtggtttgcctgaggctgtaactgagagaaagattctggggctgtgttatgaaaatatagacattctcacataagcccagttcatcaccatttcctcctttacctttcagtgcagtttcttttcacattaggctgttggttcaaacttttgggagcacggactgtcagttctctgggaagtggtcagcgcatcctgcagggcttctcctcctctgtcttttggagaaccagggctcttctcaggggctctagggactgccaggctgtttcagccaggaaggccaaaatcaagagtgagatgtagaaagttgtaaaatagaaaaagtggagttggtgaatcggttgttctttcctcacatttggatgattgtcataaggtttttagcatgttcctccttttcttcaccctccccttttttcttctattaatcaagagaaacttcaaagttaatgggatggtcggatctcacaggctgagaactcgttcacctccaagcatttcatgaaaaagctgcttcttattaatcatacaaactctcaccatgatgtgaagagtttcacaaatccttcaaaataaaaagtaatgacttagaaactgccttcctgggtgatttgcatgtgtcttagtcttagtcaccttattatcctgacacaaaaacacatgagcatacatgtctacacatgactacacaaatgcaaacctttgcaaacacattatgcttttgcacacacacacctgtacacacacaccggcatgtttatacacagggagtgtatggttcctgtaagcactaagttagctgttttcatttaatgacctgtggtttaacccttttgatcactaccaccattatcagcaccagactgagcagctatatccttttattaatcatggtcattcattcattcattcattcacaaaatatttatgatgtatttactctgcaccaggtcccatgccaagcactggggacacagttatggcaaagtagacaaagcatttgttcatttggagcttagagtccaggaggaatacattagataatgacacaatcaaatataaattgcaagatgtcacaggtgtgatgaagggagagtaggagagaccatgagtatgtgtaacaggaggacacagcattattctagtgctgtactgttccgtacggcagccactacccacatgtaactttttaagatttaaatttaaattagttaacattcaaaacgcagctccccaatcacactagcaacatttcaagtgcttgagagccatgcatgattagtggttaccctattgaataggtcagaagtagaatcttttcatcatcacagaaagttctattggacagtgctcttctagatcatcataagactacagagcacttttcaaagctcatgcatgttcatcatgttagtgtcgtattttgagctggggttttgagactccccttagagatagagaaacagacccaagaaatgtgctcaattgcaatgggccacatacctagatctccagatgtcatttcccctctcttattttaagttatgttaagattactaaaacaataaaagctcctaaaaaatcaaactgtattctggtgttctcttctacacagtgggagggcgagcagtaggagagattggcccatttggtgctggccatttgaggaatgcaagcccagcactagtctcataatctctaggaatctgtagagagaggaattgaagtaaatttcagcattggctcattcagtcattcggcgacattcatcaggtacctgcaatgtgttaggggatcttatgagtaggcagcgtgcgtgatccttgctcccctggagctttctaacattctagcaggcagaccacacataaatttgcaatactgtttctgataaaaacgtgctgtaaaggaaataaagcagagaactatcatggaaaa

SEQ ID NO: 122 - DNA, 3451 bp, Homo sapiens
agactgcccggagagcgcgctctgcctgccgcctgcctgcctgccactgagggttcccagcaccatgagggcctggatcttctttctcctttgcctggccgggagggccttggcagcccctcagcaagaagccctgcctgatgagacagaggtggtggaagaaactgtggcagaggtgactgaggtatctgtgggagctaatcctgtccaggtggaagtaggagaatttgatgatggtgcagaggaaaccgaagaggaggtggtggcggaaaatccctgccagaaccaccactgcaaacacggcaaggtgtgcgagctggatgagaacaacacccccatgtgcgtgtgccaggaccccaccagctgcccagcccccattggcgagtttgagaaggtgtgcagcaatgacaacaagaccttcgactcttcctgccacttctttgccacaaagtgcaccctggagggcaccaagaagggccacaagctccacctggactacatcgggccttgcaaatacatccccccttgcctggactctgagctgaccgaattccccctgcgcatgcgggactggctcaagaacgtcctggtcaccctgtatgagagggatgaggacaacaaccttctgactgagaagcagaagctgcgggtgaagaagatccatgagaatgagaagcgcctggaggcaggagaccaccccgtggagctgctggcccgggacttcgagaagaactataacatgtacatcttccctgtacactggcagttcggccagctggaccagcaccccattgacgggtacctctcccacaccgagctggctccactgcgtgctcccctcatccccatggagcattgcaccacccgctttttcgagacctgtgacctggacaatgacaagtacatcgccctggatgagtgggccggctgcttcggcatcaagcagaaggatatcgacaaggatcttgtgatctaaatccactccttccacagtaccggattctctctttaaccctccccttcgtgtttcccccaatgtttaaaatgtttggatggtttgttgttctgcctggagacaaggtgctaacatagatttaagtgaatacattaacggtgctaaaaatgaaaattctaacccaagacatgacattcttagctgtaacttaactattaaggccttttccacacgcattaatagtcccatttttctcttgccatttgtagctttgcccattgtcttattggcacatgggtggacacggatctgctgggctctgccttaaacacacattgcagcttcaacttttctctttagtgttctgtttgaaactaatacttaccgagtcagactttgtgttcatttcatttcagggtcttggctgcctgtgggcttccccaggtggcctggaggtgggcaaagggaagtaacagacacacgatgttgtcaaggatggttttgggactagaggctcagtggtgggagagatccctgcagaacccaccaaccagaacgtggtttgcctgaggctgtaactgagagaaagattctggggctgtgttatgaaaatatagacattctcacataagcccagttcatcaccatttcctcctttacctttcagtgcagtttcttttcacattaggctgttggttcaaacttttgggagcacggactgtcagttctctgggaagtggtcagcgcatcctgcagggcttctcctcctctgtcttttggagaaccagggctcttctcaggggctctagggactgccaggctgtttcagccaggaaggccaaaatcaagagtgagatgtagaaagttgtaaaatagaaaaagtggagttggtgaatcggttgttctttcctcacatttggatgattgtcataaggtttttagcatgttcctccttttcttcaccctccccttttttcttctattaatcaagagaaacttcaaagttaatgggatggtcggatctcacaggctgagaactcgttcacctccaagcatttcatgaaaaagctgcttcttattaatcatacaaactctcaccatgatgtgaagagtttcacaaatccttcaaaataaaaagtaatgacttagaaactgccttcctgggtgatttgcatgtgtcttagtcttagtcaccttattatcctgacacaaaaacacatgagcatacatgtctacacatgactacacaaatgcaaacctttgcaaacacattatgcttttgcacacacacacctgtacacacacaccggcatgtttatacacagggagtgtatggttcctgtaagcactaagttagctgttttcatttaatgacctgtggtttaacccttttgatcactaccaccattatcagcaccagactgagcagctatatccttttattaatcatggtcattcattcattcattcattcacaaaatatttatgatgtatttactctgcaccaggtcccatgccaagcactggggacacagttatggcaaagtagacaaagcatttgttcatttggagcttagagtccaggaggaatacattagataatgacacaatcaaatataaattgcaagatgtcacaggtgtgatgaagggagagtaggagagaccatgagtatgtgtaacaggaggacacagcattattctagtgctgtactgttccgtacggcagccactacccacatgtaactttttaagatttaaatttaaattagttaacattcaaaacgcagctccccaatcacactagcaacatttcaagtgcttgagagccatgcatgattagtggttaccctattgaataggtcagaagtagaatcttttcatcatcacagaaagttctattggacagtgctcttctagatcatcataagactacagagcacttttcaaagctcatgcatgttcatcatgttagtgtcgtattttgagctggggttttgagactccccttagagatagagaaacagacccaagaaatgtgctcaattgcaatgggccacatacctagatctccagatgtcatttcccctctcttattttaagttatgttaagattactaaaacaataaaagctcctaaaaaatcaaactgtattctggtgttctcttctacacagtgggagggcgagcagtaggagagattggcccatttggtgctggccatttgaggaatgcaagcccagcactagtctcataatctctaggaatctgtagagagaggaattgaagtaaatttcagcattggctcattcagtcattcggcgacattcatcaggtacctgcaatgtgttaggggatcttatgagtaggcagcgtgcgtgatccttgctcccctggagctttctaacattctagcaggcagaccacacataaatttgcaatactgtttctgataaaaacgtgctgtaaaggaaataaagcagagaactatcatggaaaa